European Patent Specification EP 3 157 555 B1, published May 15, 2024. Title: A DENGUE VIRUS CHIMERIC POLYEPITOPE COMPOSED OF FRAGMENTS OF NON-STRUCTURAL PROTEINS AND ITS USE IN AN IMMUNOGENIC COMPOSITION AGAINST DENGUE VIRUS INFECTION. Applicant: INSTITUT PASTEUR CENTRE NATIONAL DE LA RECHERCHE SCIENTIFIQUE. Application PCT/EPXXXXXX. The sequence listing filed with the application follows.

SEQUENCE LISTING (152 sequences)

SEQ ID NO: 1 - DNA, 1617 bp, Artificial Sequence
  Native nucleotide sequence of the polynucleotide encoding the chimeric polyepitope of DENV1
gcatcacaagaagggcccctaccagagattgaagatgaggtgtttaggaaaagaaacttaacaataatggacctacatccaggatcagggaaaacaagaagatatctcccagccatagtccgtgaggccataaaaaggaagctgcgcacactaattttggctcccacaagggttgtcgcttccgaaatggcagaggcgctcaagggaatgccaataaggtaccaaacaacagcagtgaagagtgaacacacaggaaaagagatagttgacctcatgtgccacgccactttcaccatgcgtctcctgtctcccgtgagagttcccaattacaacatgattattatggatgaagcacatttcaccgatccatccagtatagcagccagagggtacatctcaacccgagtgggcatgggtgaagcagctgcgatcttcatgacagccactcctccaggatcagtggaggcctttccacagagcaatgcagttatccaagatgaggaaagagacattcctgagagatcatggaactcaggatatgagtggatcactgacgaggaccatgctcattggacagaagcaaaaatgctccttgacaacataaacacaccagaaggaattatcccagctctctttgagccggagagagaaaagagtgcagcaatagacggggagtacagactgcggggagaagcaaggaaaacgttcgtggagctcatgagaagaggagatttaccagtttggctatcttacaaagttgcctcagaaggcttccaatactccgatagaaggtggtgctttgatggagaaaggaacaaccaggtgttggaggaaaacatggacgtggagatctggacaaaggagggagaaagaaagaaattacgaccccgctggttggacgccagaacatactctgatccactggccctgcgcgagttcaaagagttcgcagcaggagtggctgttgaaaatcaccaccatgccgcaatgctggacgtagacttacatccagcttcagcctggaccctctatgcagtggccacaacaattatcactcccatgatgaggcacacaatagaaaacacaacggcaaacatttccctgacagccattgcaaaccaggcggctatattgatgggacttgacaaaggatggccaatatcgaagatggacataggagttccacttctcgccttggggtgctattcccaggtgctggatatcattggccagaggatagagaacataaaacatgaacataagtcaacatggcattatgatgaggacaatccatataaaacatgggcctatcacggatcatatgaggtcaagccatcaggatcagcctcatccatggtcaatggcgtggtgaaactgctcaccaaaccatgggatgtcatccccatggtcacacaaatagccatgactgacaccacaccctttggacaacagagggtgttcaaagagaaagttgacacgcgcacaccaaaagcaaaacgaggcacagcacaaatcatggaggtgacagccaaatggttatggggttttctttctagaaacaaaaaaccaagaatttgtacaagagaggagttcacaagaaaagtcaggtcaaacgca

SEQ ID NO: 2 - DNA, 1617 bp, Artificial Sequence
  Optimised nucleotide sequence of the polynucleotide encoding the chimeric polyepitope of DENV1 (human codon optimised, measles optimised)
gcatcacaggagggaccactgcccgaaattgaggacgaagtgtttagaaagcgaaatctgactattatggacctgcaccccggatctggcaagacccggagatacctgccagccatcgtgagggaggctattaagcggaaactgagaacactgatcctggccccaactcgcgtggtcgcttccgaaatggctgaggccctgaaaggcatgcccatccggtatcagaccacagcagtgaagtctgaacataccggcaaggagattgtggacctgatgtgccacgccactttcaccatgcgactgctgagcccagtgcgggtccccaactacaatatgatcattatggacgaggcccactttactgatcccagctccatcgccgctagaggatatatttccaccagggtgggaatgggcgaggcagcagctatcttcatgacagcaactccccctggcagcgtggaggcatttcctcagtccaacgccgtcatccaggacgaggagcgggacattcctgagcggagctggaattctgggtacgaatggatcacagacgaggatcatgcacactggactgaagccaagatgctgctggacaacattaatactcctgagggaatcattccagctctgttcgagcccgaaagagagaagtctgcagccatcgacggcgagtatagactgaggggagaggcccggaagaccttcgtggaactgatgaggcgcggcgatctgcccgtgtggctgagttacaaggtcgcttcagagggattccagtatagtgaccgacggtggtgctttgatggcgaacgcaacaatcaggtgctggaggagaacatggatgtcgagatttggacaaaggaaggcgagcggaagaaactgcgcccacgatggctggacgctcggacttacagcgatcccctggcactgagagaattcaaagagtttgctgcaggggtggccgtcgagaatcaccatcacgccgctatgctggacgtggatctgcatcctgccagtgcttggaccctgtatgcagtggccactaccatcattaccccaatgatgcgccacacaatcgagaacacaactgccaatatctcactgacagctattgcaaaccaggcagccattctgatgggactggacaaaggctggcccatcagcaagatggatattggcgtgcctctgctggccctggggtgttacagtcaggtgctggacatcattggccagaggatcgagaacattaagcatgagcacaaatcaacctggcattacgacgaagataatccctataagacatgggcctaccacggaagctatgaggtgaaaccttcaggcagcgccagcagcatggtcaacggggtggtcaagctgctgaccaaaccttgggacgtgatcccaatggtcactcagattgccatgaccgataccaccccattcggccagcagcgggtgttcaaggagaaggtggacacccgcacacctaaggctaaacgagggactgcacagatcatggaggtgaccgccaagtggctgtggggattcctgtccaggaacaagaagccaagaatctgtaccagggaagagttcacaagaaaggtccggtcaaacgcc

SEQ ID NO: 3 - protein, 539 aa, Artificial Sequence
  Amino acid sequence of the chimeric polyepitope of DENV1
ASQEGPLPEIEDEVFRKRNLTIMDLHPGSGKTRRYLPAIVREAIKRKLRTLILAPTRVVASEMAEALKGMPIRYQTTAVKSEHTGKEIVDLMCHATFTMRLLSPVRVPNYNMIIMDEAHFTDPSSIAARGYISTRVGMGEAAAIFMTATPPGSVEAFPQSNAVIQDEERDIPERSWNSGYEWITDEDHAHWTEAKMLLDNINTPEGIIPALFEPEREKSAAIDGEYRLRGEARKTFVELMRRGDLPVWLSYKVASEGFQYSDRRWCFDGERNNQVLEENMDVEIWTKEGERKKLRPRWLDARTYSDPLALREFKEFAAGVAVENHHHAAMLDVDLHPASAWTLYAVATTIITPMMRHTIENTTANISLTAIANQAAILMGLDKGWPISKMDIGVPLLALGCYSQVLDIIGQRIENIKHEHKSTWHYDEDNPYKTWAYHGSYEVKPSGSASSMVNGVVKLLTKPWDVIPMVTQIAMTDTTPFGQQRVFKEKVDTRTPKAKRGTAQIMEVTAKWLWGFLSRNKKPRICTREEFTRKVRSNA

SEQ ID NO: 4 - DNA, 555 bp, Artificial Sequence
  Native nucleotide sequence of the polynucleotide encoding the first region of NS3 of DENV1
gcatcacaagaagggcccctaccagagattgaagatgaggtgtttaggaaaagaaacttaacaataatggacctacatccaggatcagggaaaacaagaagatatctcccagccatagtccgtgaggccataaaaaggaagctgcgcacactaattttggctcccacaagggttgtcgcttccgaaatggcagaggcgctcaagggaatgccaataaggtaccaaacaacagcagtgaagagtgaacacacaggaaaagagatagttgacctcatgtgccacgccactttcaccatgcgtctcctgtctcccgtgagagttcccaattacaacatgattattatggatgaagcacatttcaccgatccatccagtatagcagccagagggtacatctcaacccgagtgggcatgggtgaagcagctgcgatcttcatgacagccactcctccaggatcagtggaggcctttccacagagcaatgcagttatccaagatgaggaaagagacattcctgagagatcatggaactcaggatatgagtggatcactgac

SEQ ID NO: 5 - DNA, 555 bp, Artificial Sequence
  Optimised nucleotide sequence of the polynucleotide encoding the first region of NS3 of DENV1
gcatcacaggagggaccactgcccgaaattgaggacgaagtgtttagaaagcgaaatctgactattatggacctgcaccccggatctggcaagacccggagatacctgccagccatcgtgagggaggctattaagcggaaactgagaacactgatcctggccccaactcgcgtggtcgcttccgaaatggctgaggccctgaaaggcatgcccatccggtatcagaccacagcagtgaagtctgaacataccggcaaggagattgtggacctgatgtgccacgccactttcaccatgcgactgctgagcccagtgcgggtccccaactacaatatgatcattatggacgaggcccactttactgatcccagctccatcgccgctagaggatatatttccaccagggtgggaatgggcgaggcagcagctatcttcatgacagcaactccccctggcagcgtggaggcatttcctcagtccaacgccgtcatccaggacgaggagcgggacattcctgagcggagctggaattctgggtacgaatggatcacagac

SEQ ID NO: 6 - protein, 185 aa, Artificial Sequence
  Amino acid sequence of the first region of NS3 of DENV1
ASQEGPLPEIEDEVFRKRNLTIMDLHPGSGKTRRYLPAIVREAIKRKLRTLILAPTRVVASEMAEALKGMPIRYQTTAVKSEHTGKEIVDLMCHATFTMRLLSPVRVPNYNMIIMDEAHFTDPSSIAARGYISTRVGMGEAAAIFMTATPPGSVEAFPQSNAVIQDEERDIPERSWNSGYEWITD

SEQ ID NO: 7 - DNA, 402 bp, Artificial Sequence
  Native nucleotide sequence of the polynucleotide encoding the second region of NS3 of DENV1
gaggaccatgctcattggacagaagcaaaaatgctccttgacaacataaacacaccagaaggaattatcccagctctctttgagccggagagagaaaagagtgcagcaatagacggggagtacagactgcggggagaagcaaggaaaacgttcgtggagctcatgagaagaggagatttaccagtttggctatcttacaaagttgcctcagaaggcttccaatactccgatagaaggtggtgctttgatggagaaaggaacaaccaggtgttggaggaaaacatggacgtggagatctggacaaaggagggagaaagaaagaaattacgaccccgctggttggacgccagaacatactctgatccactggccctgcgcgagttcaaagagttcgcagcagga

SEQ ID NO: 8 - DNA, 402 bp, Artificial Sequence
  Optimised nucleotide sequence of the polynucleotide encoding the second region of NS3 of DENV1
gaggatcatgcacactggactgaagccaagatgctgctggacaacattaatactcctgagggaatcattccagctctgttcgagcccgaaagagagaagtctgcagccatcgacggcgagtatagactgaggggagaggcccggaagaccttcgtggaactgatgaggcgcggcgatctgcccgtgtggctgagttacaaggtcgcttcagagggattccagtatagtgaccgacggtggtgctttgatggcgaacgcaacaatcaggtgctggaggagaacatggatgtcgagatttggacaaaggaaggcgagcggaagaaactgcgcccacgatggctggacgctcggacttacagcgatcccctggcactgagagaattcaaagagtttgctgcaggg

SEQ ID NO: 9 - protein, 134 aa, Artificial Sequence
  Amino acid sequence of the second region of NS3 of DENV1
EDHAHWTEAKMLLDNINTPEGIIPALFEPEREKSAAIDGEYRLRGEARKTFVELMRRGDLPVWLSYKVASEGFQYSDRRWCFDGERNNQVLEENMDVEIWTKEGERKKLRPRWLDARTYSDPLALREFKEFAAG

SEQ ID NO: 10 - DNA, 258 bp, Artificial Sequence
  Native nucleotide sequence of the polynucleotide encoding the NS4b fragment of DENV1
gtggctgttgaaaatcaccaccatgccgcaatgctggacgtagacttacatccagcttcagcctggaccctctatgcagtggccacaacaattatcactcccatgatgaggcacacaatagaaaacacaacggcaaacatttccctgacagccattgcaaaccaggcggctatattgatgggacttgacaaaggatggccaatatcgaagatggacataggagttccacttctcgccttggggtgctattcccaggtg

SEQ ID NO: 11 - DNA, 258 bp, Artificial Sequence
  Optimised nucleotide sequence of the polynucleotide encoding the NS4b fragment of DENV1
gtggccgtcgagaatcaccatcacgccgctatgctggacgtggatctgcatcctgccagtgcttggaccctgtatgcagtggccactaccatcattaccccaatgatgcgccacacaatcgagaacacaactgccaatatctcactgacagctattgcaaaccaggcagccattctgatgggactggacaaaggctggcccatcagcaagatggatattggcgtgcctctgctggccctggggtgttacagtcaggtg

SEQ ID NO: 12 - protein, 86 aa, Artificial Sequence
  Amino acid sequence of the NS4b fragment of DENV1
VAVENHHHAAMLDVDLHPASAWTLYAVATTIITPMMRHTIENTTANISLTAIANQAAILMGLDKGWPISKMDIGVPLLALGCYSQV

SEQ ID NO: 13 - DNA, 402 bp, Artificial Sequence
  Native nucleotide sequence of the polynucleotide encoding the NS5 fragment of DENV1
ctggatatcattggccagaggatagagaacataaaacatgaacataagtcaacatggcattatgatgaggacaatccatataaaacatgggcctatcacggatcatatgaggtcaagccatcaggatcagcctcatccatggtcaatggcgtggtgaaactgctcaccaaaccatgggatgtcatccccatggtcacacaaatagccatgactgacaccacaccctttggacaacagagggtgttcaaagagaaagttgacacgcgcacaccaaaagcaaaacgaggcacagcacaaatcatggaggtgacagccaaatggttatggggttttctttctagaaacaaaaaaccaagaatttgtacaagagaggagttcacaagaaaagtcaggtcaaacgca

SEQ ID NO: 14 - DNA, 402 bp, Artificial Sequence
  Optimised nucleotide sequence of the polynucleotide encoding the NS5 fragment of DENV1
ctggacatcattggccagaggatcgagaacattaagcatgagcacaaatcaacctggcattacgacgaagataatccctataagacatgggcctaccacggaagctatgaggtgaaaccttcaggcagcgccagcagcatggtcaacggggtggtcaagctgctgaccaaaccttgggacgtgatcccaatggtcactcagattgccatgaccgataccaccccattcggccagcagcgggtgttcaaggagaaggtggacacccgcacacctaaggctaaacgagggactgcacagatcatggaggtgaccgccaagtggctgtggggattcctgtccaggaacaagaagccaagaatctgtaccagggaagagttcacaagaaaggtccggtcaaacgcc

SEQ ID NO: 15 - protein, 134 aa, Artificial Sequence
  Amino acid sequence of the NS5 fragment of DENV1
LDIIGQRIENIKHEHKSTWHYDEDNPYKTWAYHGSYEVKPSGSASSMVNGVVKLLTKPWDVIPMVTQIAMTDTTPFGQQRVFKEKVDTRTPKAKRGTAQIMEVTAKWLWGFLSRNKKPRICTREEFTRKVRSNA

SEQ ID NO: 16 - protein, 9 aa, Artificial Sequence
  Amino acid sequence of the P20 epitope
LPEIEDEVF

SEQ ID NO: 17 - protein, 10 aa, Artificial Sequence
  Amino acid sequence of the P19 epitope
HPGSGKTRRY

SEQ ID NO: 18 - protein, 11 aa, Artificial Sequence
  Amino acid sequence of the P30 epitope
RYLPAIVREAI

SEQ ID NO: 19 - protein, 9 aa, Artificial Sequence
  Amino acid sequence of the P451 epitope
YLPAIVREA

SEQ ID NO: 20 - protein, 9 aa, Artificial Sequence
  Amino acid sequence of the P11 epitope
LPAIVREAI

SEQ ID NO: 21 - protein, 10 aa, Artificial Sequence
  Amino acid sequence of the P36 epitope
APTRVVASEM

SEQ ID NO: 22 - protein, 15 aa, Artificial Sequence
  Amino acid sequence of the P48 EPITOPE
EMAEALKGMPIRYQT

SEQ ID NO: 23 - protein, 10 aa, Artificial Sequence
  Amino acid sequence of the P12 epitope
SPVRVPNYNM

SEQ ID NO: 24 - protein, 9 aa, Artificial Sequence
  Amino acid sequence of the P454 epitope
VPNYNMIIM

SEQ ID NO: 25 - protein, 10 aa, Artificial Sequence
  Amino acid sequence of the P18 epitope
DPSSIAARGY

SEQ ID NO: 26 - protein, 10 aa, Artificial Sequence
  Amino acid sequence of the P457 epitope
AVIQDEERDI

SEQ ID NO: 27 - protein, 9 aa, Artificial Sequence
  Amino acid sequence of the P453 epitope
RSWNSGYEW

SEQ ID NO: 28 - protein, 9 aa, Artificial Sequence
  Amino acid sequence of the P49 epitope
TPEGIIPAL

SEQ ID NO: 29 - protein, 9 aa, Artificial Sequence
  Amino acid sequence of the P28 epitope
KTFVELMRR

SEQ ID NO: 30 - protein, 10 aa, Artificial Sequence
  Amino acid sequence of the P2 epitope
ELMRRGDLPV

SEQ ID NO: 31 - protein, 10 aa, Artificial Sequence
  Amino acid sequence of the P450 epitope
DLMRRGDLPV

SEQ ID NO: 32 - protein, 10 aa, Artificial Sequence
  Amino acid sequence of the P50 epitope
LPVWLSYKVA

SEQ ID NO: 33 - protein, 9 aa, Artificial Sequence
  Amino acid sequence of the P32 epitope
QYSDRRWCF

SEQ ID NO: 34 - protein, 9 aa, Artificial Sequence
  Amino acid sequence of the P73 epitope
NYADRRWCF

SEQ ID NO: 35 - protein, 9 aa, Artificial Sequence
  Amino acid sequence of the P74 epitope
NYADRKWCF

SEQ ID NO: 36 - protein, 9 aa, Artificial Sequence
  Amino acid sequence of the P75 epitope
KYTDRKWCF

SEQ ID NO: 37 - protein, 9 aa, Artificial Sequence
  Amino acid sequence of the P76 epitope
SYKDREWCF

SEQ ID NO: 38 - protein, 9 aa, Artificial Sequence
  Amino acid sequence of the P35 epitope
RPRWLDART

SEQ ID NO: 39 - protein, 18 aa, Artificial Sequence
  Amino acid sequence of the P17 epitope
LDARTYSDPLALREFKEF

SEQ ID NO: 40 - protein, 10 aa, Artificial Sequence
  Amino acid sequence of the P29 epitope
RIYSDPLALK

SEQ ID NO: 41 - protein, 10 aa, Artificial Sequence
  Amino acid sequence of the P452 epitope
RTYSDPLALR

SEQ ID NO: 42 - protein, 9 aa, Artificial Sequence
  Amino acid sequence of the P21 epitope
HPASAWTLY

SEQ ID NO: 43 - protein, 8 aa, Artificial Sequence
  Amino acid sequence of the P16 epitope
PASAWTLY

SEQ ID NO: 44 - protein, 10 aa, Artificial Sequence
  Amino acid sequence of the P13 epitope
HPASAWTLYA

SEQ ID NO: 45 - protein, 9 aa, Artificial Sequence
  Amino acid sequence of the P51 epitope
TLYAVATTI

SEQ ID NO: 46 - protein, 9 aa, Artificial Sequence
  Amino acid sequence of the P52 epitope
VATTIITPM

SEQ ID NO: 47 - protein, 9 aa, Artificial Sequence
  Amino acid sequence of the P33 epitope
ITPMMRHTI

SEQ ID NO: 48 - protein, 10 aa, Artificial Sequence
  Amino acid sequence of the P14 epitope
TPMMRHTIEN

SEQ ID NO: 49 - protein, 9 aa, Artificial Sequence
  Amino acid sequence of the P22 epitope
IANQAAILM

SEQ ID NO: 50 - protein, 9 aa, Artificial Sequence
  Amino acid sequence of the P456 epitope
AAILMGLDK

SEQ ID NO: 51 - protein, 9 aa, Artificial Sequence
  Amino acid sequence of the P53 epitope
KMDIGVPLL

SEQ ID NO: 52 - protein, 9 aa, Artificial Sequence
  Amino acid sequence of the P54 epitope
VPLLALGCY

SEQ ID NO: 53 - protein, 10 aa, Artificial Sequence
  Amino acid sequence of the P55 epitope
DNPYKTWAYH

SEQ ID NO: 54 - protein, 9 aa, Artificial Sequence
  Amino acid sequence of the P24 epitope
WAYHGSYEV

SEQ ID NO: 55 - protein, 9 aa, Artificial Sequence
  Amino acid sequence of the P56 epitope
SMVNGVVKL

SEQ ID NO: 56 - protein, 15 aa, Artificial Sequence
  Amino acid sequence of the P5 epitope
LLTKPWDVIPMVTQI

SEQ ID NO: 57 - protein, 10 aa, Artificial Sequence
  Amino acid sequence of the P6 epitope
LLTKPWDVIP

SEQ ID NO: 58 - protein, 10 aa, Artificial Sequence
  Amino acid sequence of the P7 epitope
LTKPWDVIPM

SEQ ID NO: 59 - protein, 10 aa, Artificial Sequence
  Amino acid sequence of the P8 epitope
TKPWDVIPMV

SEQ ID NO: 60 - protein, 10 aa, Artificial Sequence
  Amino acid sequence of the P9 epitope
KPWDVIPMVT

SEQ ID NO: 61 - protein, 10 aa, Artificial Sequence
  Amino acid sequence of the P10 epitope
PWDVIPMVTQ

SEQ ID NO: 62 - protein, 10 aa, Artificial Sequence
  Amino acid sequence of the P27 epitope
WDVIPMVTQI

SEQ ID NO: 63 - protein, 9 aa, Artificial Sequence
  Amino acid sequence of the P455 epitope
IPMVTQIAM

SEQ ID NO: 64 - protein, 9 aa, Artificial Sequence
  Amino acid sequence of the P34 epitope
DTTPFGQQR

SEQ ID NO: 65 - protein, 9 aa, Artificial Sequence
  Amino acid sequence of the P23 epitope
TPFGQQRVF

SEQ ID NO: 66 - protein, 20 aa, Artificial Sequence
  Amino acid sequence of the P3 epitope
TAKWLWGFLSRNKKPRICTR

SEQ ID NO: 67 - protein, 9 aa, Artificial Sequence
  Amino acid sequence of the P4 epitope
WGFLSRNKK

SEQ ID NO: 68 - protein, 10 aa, Artificial Sequence
  Amino acid sequence of the P15 epitope
KPRICTREEF

SEQ ID NO: 69 - protein, 15 aa, Artificial Sequence
  Amino acid sequence of the peptide at position 8-22 of the first region of NS3
PELEEEMFKKRNLTI

SEQ ID NO: 70 - protein, 15 aa, Artificial Sequence
  Amino acid sequence of the peptide at position 18-32 of the first region of NS3
RKLTIMDLHPGSGKT

SEQ ID NO: 71 - protein, 15 aa, Artificial Sequence
  Amino acid sequence of the peptide at position 32-46 of the first region of NS3
TKRYLPAIVREAIKR

SEQ ID NO: 72 - protein, 10 aa, Artificial Sequence
  Amino acid sequence of the peptide at position 33-42 of the first region of NS3
RKYLPAIVRE

SEQ ID NO: 73 - protein, 15 aa, Artificial Sequence
  Amino acid sequence of the peptide at position 36-50 of the first region of NS3
LPAIVREAIKRRLRT

SEQ ID NO: 74 - protein, 15 aa, Artificial Sequence
  Amino acid sequence of the peptide at position 40-54 of the first region of NS3
VREAIKRRLRTLILA

SEQ ID NO: 75 - protein, 11 aa, Artificial Sequence
  Amino acid sequence of the peptide at position 56-66 of the first region of NS3
TRVVAAEMEEA

SEQ ID NO: 76 - protein, 15 aa, Artificial Sequence
  Amino acid sequence of the peptide at position 55-69 of the first region of NS3
PTRVVAAEMEEAMKG

SEQ ID NO: 77 - protein, 15 aa, Artificial Sequence
  Amino acid sequence of the peptide at position 66-80 of the first region of NS3
ALKGMPIRYQTTAVK

SEQ ID NO: 78 - protein, 15 aa, Artificial Sequence
  Amino acid sequence of the peptide at position 68-82 of the first region of NS3
KGLPIRYQTTATKSE

SEQ ID NO: 79 - protein, 15 aa, Artificial Sequence
  Amino acid sequence of the peptide at position 72-86 of the first region of NS3
IRYQTTATKSEHTGR

SEQ ID NO: 80 - protein, 15 aa, Artificial Sequence
  Amino acid sequence of the peptide at position 83-97 of the first region of NS3
HTGREIVDLMCHATE

SEQ ID NO: 81 - protein, 12 aa, Artificial Sequence
  Amino acid sequence of the peptide at position 86-97 of the first region of NS3
REIVDLMCHATF

SEQ ID NO: 82 - protein, 10 aa, Artificial Sequence
  Amino acid sequence of the peptide at position 87-96 of the first region of NS3
EIVDLMCHAT

SEQ ID NO: 83 - protein, 10 aa, Artificial Sequence
  Amino acid sequence of the peptide at position 89-98 of the first region of NS3
VDLMCHATFT

SEQ ID NO: 84 - protein, 15 aa, Artificial Sequence
  Amino acid sequence of the peptide at position 96-110 of the first region of NS3
TFTMRLLSPVRVPNY

SEQ ID NO: 85 - protein, 15 aa, Artificial Sequence
  Amino acid sequence of the peptide at position 108-122 of the first region of NS3
PNYNLIIMDEAHFTD

SEQ ID NO: 86 - protein, 15 aa, Artificial Sequence
  Amino acid sequence of the peptide at position 124-138 of the first region of NS3
ASIAARGYISTRVGM

SEQ ID NO: 87 - protein, 15 aa, Artificial Sequence
  Amino acid sequence of the peptide at position 139-154 of the first region of NS3
EAAAIFMTATPPGTA

SEQ ID NO: 88 - protein, 15 aa, Artificial Sequence
  Amino acid sequence of the peptide at position 287-301 of the second region of NS3
REGEKKKLRPRWLDR

SEQ ID NO: 89 - protein, 15 aa, Artificial Sequence
  Amino acid sequence of the peptide at position 307-319 of the second region of NS3
PLALKEFKDFAAGRK

SEQ ID NO: 90 - protein, 17 aa, Artificial Sequence
  Amino acid sequence of the peptide at position 417-433 of NS5
KEEHSSTWHYDDENPYK

SEQ ID NO: 91 - protein, 17 aa, Artificial Sequence
  Amino acid sequence of the peptide at position 423-439 of NS5
TWHYDDENPYKTWAYHG

SEQ ID NO: 92 - protein, 17 aa, Artificial Sequence
  Amino acid sequence of the peptide at position 427-444 of NS5
DENPYKTWAYHGSYEVK

SEQ ID NO: 93 - protein, 15 aa, Artificial Sequence
  Amino acid sequence of the peptide at position 433-447 of NS5
KTWAYHGSYETKQTG

SEQ ID NO: 94 - protein, 17 aa, Artificial Sequence
  Amino acid sequence of the peptide at position 451-473 of NS5
SMINGVVKLLTKPWDVV

SEQ ID NO: 95 - protein, 9 aa, Artificial Sequence
  Amino acid sequence of the peptide at position 462-471 of NS5
KPWDVLPMV

SEQ ID NO: 96 - protein, 17 aa, Artificial Sequence
  Amino acid sequence of the peptide at position 457-463 of NS5
VKLLTKPWDVVPMVTQM

SEQ ID NO: 97 - protein, 18 aa, Artificial Sequence
  Amino acid sequence of the peptide at position 469-485 of NS5
MVTQMAMTDTTPFGQQRV

SEQ ID NO: 98 - protein, 15 aa, Artificial Sequence
  Synthetic peptide
VKSEHTGKEIVDLMC

SEQ ID NO: 99 - protein, 15 aa, Artificial Sequence
  Synthetic peptide
HTGKEIVDLMCHATF

SEQ ID NO: 100 - protein, 15 aa, Artificial Sequence
  Synthetic peptide
EIVDLMCHATFTMRL

SEQ ID NO: 101 - protein, 15 aa, Artificial Sequence
  Synthetic peptide
LMCHATFTMRLLSPV

SEQ ID NO: 102 - protein, 15 aa, Artificial Sequence
  Synthetic peptide
ATFTMRLLSPVRVPN

SEQ ID NO: 103 - protein, 15 aa, Artificial Sequence
  Synthetic peptide
MRLLSPVRVPNYNMI

SEQ ID NO: 104 - protein, 15 aa, Artificial Sequence
  Synthetic peptide
EFKEFAAGVAVENHH

SEQ ID NO: 105 - protein, 15 aa, Artificial Sequence
  Synthetic peptide
FAAGVAVENHHHAAM

SEQ ID NO: 106 - protein, 15 aa, Artificial Sequence
  Synthetic peptide
VAVENHHHAAMLDVD

SEQ ID NO: 107 - protein, 15 aa, Artificial Sequence
  Synthetic peptide
NHHHAAMLDVDLHPA

SEQ ID NO: 108 - protein, 15 aa, Artificial Sequence
  Synthetic peptide
AAMLDVDLHPASAWT

SEQ ID NO: 109 - protein, 15 aa, Artificial Sequence
  Synthetic peptide
DVDLHPASAWTLYAV

SEQ ID NO: 110 - protein, 15 aa, Artificial Sequence
  Synthetic peptide
HPASAWTLYAVATTI

SEQ ID NO: 111 - protein, 15 aa, Artificial Sequence
  Synthetic peptide
AWTLYAVATTIITPM

SEQ ID NO: 112 - protein, 15 aa, Artificial Sequence
  Synthetic peptide
YAVATTIITPMMRHT

SEQ ID NO: 113 - protein, 15 aa, Artificial Sequence
  Synthetic peptide
TTIITPMMRHTIENT

SEQ ID NO: 114 - protein, 15 aa, Artificial Sequence
  Synthetic peptide
TPMMRHTIENTTANI

SEQ ID NO: 115 - protein, 15 aa, Artificial Sequence
  Synthetic peptide
RHTIENTTANISLTA

SEQ ID NO: 116 - protein, 15 aa, Artificial Sequence
  Synthetic peptide
ENTTANISLTAIANQ

SEQ ID NO: 117 - protein, 15 aa, Artificial Sequence
  Synthetic peptide
ANISLTAIANQAAIL

SEQ ID NO: 118 - protein, 15 aa, Artificial Sequence
  Synthetic peptide
GWPISKMDIGVPLLA

SEQ ID NO: 119 - protein, 15 aa, Artificial Sequence
  Synthetic peptide
SKMDIGVPLLALGCY

SEQ ID NO: 120 - protein, 15 aa, Artificial Sequence
  Synthetic peptide
IGVPLLALGCYSQVL

SEQ ID NO: 121 - protein, 15 aa, Artificial Sequence
  Synthetic peptide
DEDNPYKTWAYHGSY

SEQ ID NO: 122 - protein, 15 aa, Artificial Sequence
  Synthetic peptide
PYKTWAYHGSYEVKP

SEQ ID NO: 123 - protein, 15 aa, Artificial Sequence
  Synthetic peptide
WAYHGSYEVKPSGSA

SEQ ID NO: 124 - protein, 15 aa, Artificial Sequence
  Synthetic peptide
GSYEVKPSGSASSMV

SEQ ID NO: 125 - protein, 15 aa, Artificial Sequence
  Synthetic peptide
VKPSGSASSMVNGVV

SEQ ID NO: 126 - protein, 15 aa, Artificial Sequence
  Synthetic peptide
GSASSMVNGVVKLLT

SEQ ID NO: 127 - protein, 15 aa, Artificial Sequence
  Synthetic peptide
SMVNGVVKLLTKPWD

SEQ ID NO: 128 - protein, 15 aa, Artificial Sequence
  Synthetic peptide
GVVKLLTKPWDVIPM

SEQ ID NO: 129 - protein, 15 aa, Artificial Sequence
  Synthetic peptide
LLTKPWDVIPMVTQI

SEQ ID NO: 130 - protein, 15 aa, Artificial Sequence
  Synthetic peptide
PWDVIPMVTQIAMTD

SEQ ID NO: 131 - protein, 15 aa, Artificial Sequence
  Synthetic peptide
IPMVTQIAMTDTTPF

SEQ ID NO: 132 - protein, 15 aa, Artificial Sequence
  Synthetic peptide
TQIAMTDTTPFGQQR

SEQ ID NO: 133 - protein, 15 aa, Artificial Sequence
  Synthetic peptide
MTDTTPFGQQRVFKE

SEQ ID NO: 134 - protein, 9 aa, Artificial Sequence
  Synthetic peptide
FTMRLLSPV

SEQ ID NO: 135 - protein, 11 aa, Artificial Sequence
  Synthetic peptide
VAVENHHHAAM

SEQ ID NO: 136 - protein, 9 aa, Artificial Sequence
  Synthetic peptide
LYAVATTII

SEQ ID NO: 137 - protein, 9 aa, Artificial Sequence
  Synthetic peptide
TAIANQAAI

SEQ ID NO: 138 - protein, 10 aa, Artificial Sequence
  Synthetic peptide
SSMVNGVVKL

SEQ ID NO: 139 - DNA, 22363 bp, Artificial Sequence
  Complete optimised nucleotide sequence of the polynucleotide encoding pTM-MVDVax6
  misc_feature (1)..(8): NotI
  misc_feature (9)..(28): T7 promoter
  misc_feature (29)..(82): Hammerhead ribozyme
  misc_feature (83)..(189): MV Leader and N promoter
  misc_feature (190)..(1767): MV N ORF
  misc_feature (1768)..(1888): MV N-P intergenic
  misc_feature (1889)..(3412): MV P ORF
  misc_feature (3413)..(3531): MV ATU2
  misc_feature (3532)..(5085): DENV tetra EDIII + ectoM
  misc_feature (5086)..(5181): MV P-M intergenic
  misc_feature (5182)..(6189): MV M ORF
  misc_feature (6190)..(7192): MV M-F intergenic
  misc_feature (7193)..(8854): MV F ORF
  misc_feature (8855)..(9014): MV-F-H intergenic
  misc_feature (9015)..(10868): MV H ORF
  misc_feature (10869)..(10995): MV ATU3
  misc_feature (10996)..(12618): DENV1 NS polyepitope
  misc_feature (12619)..(12712): MV H-L intergenic
  misc_feature (12713)..(19263): MV L ORF
  misc_feature (19264)..(19372): MV Trailer
  misc_feature (19373)..(19456): HDV ribozyme
  misc_feature (19457)..(19598): T7 terminator
  misc_feature (19599)..(19606): Not I
  misc_feature (19607)..(22363): pTM plasmid
gcggccgctaatacgactcactatagggccaactttgtttggtctgatgagtccgtgaggacgaaacccggagtcccgggtcaccaaacaaagttgggtaaggatagttcaatcaatgatcatcttctagtgcacttaggattcaagatcctattatcagggacaagagcaggattagggatatccgagatggccacacttttaaggagcttagcattgttcaaaagaaacaaggacaaaccacccattacatcaggatccggtggagccatcagaggaatcaaacacattattatagtaccaatccctggagattcctcaattaccactcgatccagacttctggaccggttggtgaggttaattggaaacccggatgtgagcgggcccaaactaacaggggcactaataggtatattatccttatttgtggagtctccaggtcaattgattcagaggatcaccgatgaccctgacgttagcataaggctgttagaggttgtccagagtgaccagtcacaatctggccttaccttcgcatcaagaggtaccaacatggaggatgaggcggaccaatacttttcacatgatgatccaattagtagtgatcaatccaggttcggatggttcgggaacaaggaaatctcagatattgaagtgcaagaccctgagggattcaacatgattctgggtaccatcctagcccaaatttgggtcttgctcgcaaaggcggttacggccccagacacggcagctgattcggagctaagaaggtggataaagtacacccaacaaagaagggtagttggtgaatttagattggagagaaaatggttggatgtggtgaggaacaggattgccgaggacctctccttacgccgattcatggtcgctctaatcctggatatcaagagaacacccggaaacaaacccaggattgctgaaatgatatgtgacattgatacatatatcgtagaggcaggattagccagttttatcctgactattaagtttgggatagaaactatgtatcctgctcttggactgcatgaatttgctggtgagttatccacacttgagtccttgatgaacctttaccagcaaatgggggaaactgcaccctacatggtaatcctggagaactcaattcagaacaagttcagtgcaggatcataccctctgctctggagctatgccatgggagtaggagtggaacttgaaaactccatgggaggtttgaactttggccgatcttactttgatccagcatattttagattagggcaagagatggtaaggaggtcagctggaaaggtcagttccacattggcatctgaactcggtatcactgccgaggatgcaaggcttgtttcagagattgcaatgcatactactgaggacaagatcagtagagcggttggacccagacaagcccaagtatcatttctacacggtgatcaaagtgagaatgagctaccgagattggggggcaaggaagataggagggtcaaacagagtcgaggagaagccagggagagctacagagaaaccgggcccagcagagcaagtgatgcgagagctgcccatcttccaaccggcacacccctagacattgacactgcaacggagtccagccaagatccgcaggacagtcgaaggtcagctgacgccctgcttaggctgcaagccatggcaggaatctcggaagaacaaggctcagacacggacacccctatagtgtacaatgacagaaatcttctagactaggtgcgagaggccgagggccagaacaacatccgcctaccatccatcattgttataaaaaacttaggaaccaggtccacacagccgccagcccatcaaccatccactcccacgattggagccaatggcagaagagcaggcacgccatgtcaaaaacggactggaatgcatccgggctctcaaggccgagcccatcggctcactggccatcgaggaagctatggcagcatggtcagaaatatcagacaacccaggacaggagcgagccacctgcagggaagagaaggcaggcagttcgggtctcagcaaaccatgcctctcagcaattggatcaactgaaggcggtgcacctcgcatccgcggtcagggacctggagagagcgatgacgacgctgaaactttgggaatccccccaagaaatctccaggcatcaagcactgggttacagtgttattacgtttatgatcacagcggtgaagcggttaagggaatccaagatgctgactctatcatggttcaatcaggccttgatggtgatagcaccctctcaggaggagacaatgaatctgaaaacagcgatgtggatattggcgaacctgataccgagggatatgctatcactgaccggggatctgctcccatctctatggggttcagggcttctgatgttgaaactgcagaaggaggggagatccacgagctcctgagactccaatccagaggcaacaactttccgaagcttgggaaaactctcaatgttcctccgcccccggaccccggtagggccagcacttccgggacacccattaaaaagggcacagacgcgagattagcctcatttggaacggagatcgcgtctttattgacaggtggtgcaacccaatgtgctcgaaagtcaccctcggaaccatcagggccaggtgcacctgcggggaatgtccccgagtgtgtgagcaatgccgcactgatacaggagtggacacccgaatctggtaccacaatctccccgagatcccagaataatgaagaagggggagactattatgatgatgagctgttctctgatgtccaagatattaaaacagccttggccaaaatacacgaggataatcagaagataatctccaagctagaatcactgctgttattgaagggagaagttgagtcaattaagaagcagatcaacaggcaaaatatcagcatatccaccctggaaggacacctctcaagcatcatgatcgccattcctggacttgggaaggatcccaacgaccccactgcagatgtcgaaatcaatcccgacttgaaacccatcataggcagagattcaggccgagcactggccgaagttctcaagaaacccgttgccagccgacaactccaaggaatgacaaatggacggaccagttccagaggacagctgctgaaggaatttcagctaaagccgatcgggaaaaagatgagctcagccgtcgggtttgttcctgacaccggccctgcatcacgcagtgtaatccgctccattataaaatccagccggctagaggaggatcggaagcgttacctgatgactctccttgatgatatcaaaggagccaatgatcttgccaagttccaccagatgctgatgaagataataatgaagtagctacagctcaacttacctgccaaccccatgccagtcgacccaactagcctaccctccatcattgttataaaaaacttaggaaccaggtccacacagccgccagcccatcaacgcgtacgatgggcatcatattcattcttcttatgctggttacaccgtctatggcggagaaacttcgaatcaaaggtatgagctatacgatgtgcagcggcaagttcaagatcgagaaggaaatggctgaaacccagcacggtacaactgtggtcaaagtcaaatatgagggggctggcgctccctgtaaagtacccattgagattagggacgtcaataaagagaaggtggtaggtcgcatcatctccagtacacctttggccgagaacacgaactccgtcacaaacatagagttggaacccccgttcggagactcatacattgtgatcggggtgggcaactctgcactcacactgcattggttcaagaagggaagcagtatcggccgcagggataagagagacaaactgaaattgaaaggtatgtcctatgccatgtgcacgaatactttcgttctcaagaaagaagtatctgagactcagcacggaaccatcctgatcaaagtcgagtacaaaggagaagacgtgccctgtaagatcccattcagtaccgaggatggacagggcaaggcccataacggcaggctgataaccgccaaccctgtggttacaaagaaggaagagccagtcaatatcgaagctgagccaccgttcggggagagcaacatagtaattggcataggggataatgctttgaagatcaactggtacaagaaaggaagctccattggccgaagagataagcgcgacaaactccagctgaaaggaatgagctactccatgtgtactgggaagttcaagattgtcaaggaaatcgccgaaactcagcatggcactattgtgatccgcgtgcagtatgaaggcgatggtagcccctgcaagataccatttgaaatcaccgatttggagaaacggcacgtcctgggtcggctcattaccgtgaacccaatcgtgaccgagaaggacagtccagttaatatcgaggccgagcctcctttcggcgacagttacatcattgtaggggtggaaccagggcaactgaagctgaactggttcaagaaaggcagcagtataggacggcgggataaacgggacaaactcacactgaaaggcatgtcatacgttatgtgcaccggctcattcaaactggagaaggaagttgcagagacacagcatgggaccgtgctcgtgcaggtcaaatacgagggcaccgacgctccttgcaagattccgttcagtacacaggacgagaaaggcgtgactcagaacggcagattgattacagcgaaccctatcgtgactgacaaggagaagccagttaacatcgagactgagccgcctttcggagaatcatacattatcgtgggagccggcgagaaggcactgaaactcagctggttcaagaagggcagctcaatcggtcggagagacaagcggtctgtcgccctcgcaccgcacgtgggcctgggtctggaaacgaggaccgagacgtggatgagttccgaaggcgcatggaagcaaatccagaaagtggagacgtgggccctcaggcatccgtaatgagcgcgcagcgcttagacgtctcgcgatcgatactagtacaacctaaatccattataaaaaacttaggagcaaagtgattgcctcccaaggtccacaatgacagagacctacgacttcgacaagtcggcatgggacatcaaagggtcgatcgctccgatacaacccaccacctacagtgatggcaggctggtgccccaggtcagagtcatagatcctggtctaggcgacaggaaggatgaatgctttatgtacatgtttctgctgggggttgttgaggacagcgattccctagggcctccaatcgggcgagcatttgggttcctgcccttaggtgttggcagatccacagcaaagcccgaaaaactcctcaaagaggccactgagcttgacatagttgttagacgtacagcagggctcaatgaaaaactggtgttctacaacaacaccccactaactctcctcacaccttggagaaaggtcctaacaacagggagtgtcttcaacgcaaaccaagtgtgcaatgcggttaatctgataccgctcgataccccgcagaggttccgtgttgtttatatgagcatcacccgtctttcggataacgggtattacaccgttcctagaagaatgctggaattcagatcggtcaatgcagtggccttcaacctgctggtgacccttaggattgacaaggcgataggccctgggaagatcatcgacaatacagagcaacttcctgaggcaacatttatggtccacatcgggaacttcaggagaaagaagagtgaagtctactctgccgattattgcaaaatgaaaatcgaaaagatgggcctggtttttgcacttggtgggatagggggcaccagtcttcacattagaagcacaggcaaaatgagcaagactctccatgcacaactcgggttcaagaagaccttatgttacccgctgatggatatcaatgaagaccttaatcgattactctggaggagcagatgcaagatagtaagaatccaggcagttttgcagccatcagttcctcaagaattccgcatttacgacgacgtgatcataaatgatgaccaaggactattcaaagttctgtagaccgtagtgcccagcaatgcccgaaaacgacccccctcacaatgacagccagaaggcccggacaaaaaagccccctccgaaagactccacggaccaagcgagaggccagccagcagccgacggcaagcgcgaacaccaggcggccccagcacagaacagccctgacacaaggccaccaccagccaccccaatctgcatcctcctcgtgggacccccgaggaccaacccccaaggctgcccccgatccaaaccaccaaccgcatccccaccacccccgggaaagaaacccccagcaattggaaggcccctccccctcttcctcaacacaagaactccacaaccgaaccgcacaagcgaccgaggtgacccaaccgcaggcatccgactccctagacagatcctctctccccggcaaactaaacaaaacttagggccaaggaacatacacacccaacagaacccagaccccggcccacggcgccgcgcccccaacccccgacaaccagagggagcccccaaccaatcccgccggctcccccggtgcccacaggcagggacaccaacccccgaacagacccagcacccaaccatcgacaatccaagacgggggggcccccccaaaaaaaggcccccaggggccgacagccagcaccgcgaggaagcccacccaccccacacacgaccacggcaaccaaaccagaacccagaccaccctgggccaccagctcccagactcggccatcaccccgcagaaaggaaaggccacaacccgcgcaccccagccccgatccggcggggagccacccaacccgaaccagcacccaagagcgatccccgaaggacccccgaaccgcaaaggacatcagtatcccacagcctctccaagtcccccggtctcctcctcttctcgaagggaccaaaagatcaatccaccacacccgacgacactcaactccccacccctaaaggagacaccgggaatcccagaatcaagactcatccaatgtccatcatgggtctcaaggtgaacgtctctgccatattcatggcagtactgttaactctccaaacacccaccggtcaaatccattggggcaatctctctaagataggggtggtaggaataggaagtgcaagctacaaagttatgactcgttccagccatcaatcattagtcataaaattaatgcccaatataactctcctcaataactgcacgagggtagagattgcagaatacaggagactactgagaacagttttggaaccaattagagatgcacttaatgcaatgacccagaatataagaccggttcagagtgtagcttcaagtaggagacacaagagatttgcgggagtagtcctggcaggtgcggccctaggcgttgccacagctgctcagataacagccggcattgcacttcaccagtccatgctgaactctcaagccatcgacaatctgagagcgagcctggaaactactaatcaggcaattgagacaatcagacaagcagggcaggagatgatattggctgttcagggtgtccaagactacatcaataatgagctgataccgtctatgaaccaactatcttgtgatttaatcggccagaagctcgggctcaaattgctcagatactatacagaaatcctgtcattatttggccccagtttacgggaccccatatctgcggagatatctatccaggctttgagctatgcgcttggaggagacatcaataaggtgttagaaaagctcggatacagtggaggtgatttactgggcatcttagagagcggaggaataaaggcccggataactcacgtcgacacagagtcctacttcattgtcctcagtatagcctatccgacgctgtccgagattaagggggtgattgtccaccggctagagggggtctcgtacaacataggctctcaagagtggtataccactgtgcccaagtatgttgcaacccaagggtaccttatctcgaattttgatgagtcatcgtgtactttcatgccagaggggactgtgtgcagccaaaatgccttgtacccgatgagtcctctgctccaagaatgcctccgggggtacaccaagtcctgtgctcgtacactcgtatccgggtcttttgggaaccggttcattttatcacaagggaacctaatagccaattgtgcatcaatcctttgcaagtgttacacaacaggaacgatcattaatcaagaccctgacaagatcctaacatacattgctgccgatcactgcccggtagtcgaggtgaacggcgtgaccatccaagtcgggagcaggaggtatccagacgctgtgtacttgcacagaattgacctcggtcctcccatatcattggagaggttggacgtagggacaaatctggggaatgcaattgctaagttggaggatgccaaggaattgttggagtcatcggaccagatattgaggagtatgaaaggtttatcgagcactagcatagtctacatcctgattgcagtgtgtcttggagggttgatagggatccccgctttaatatgttgctgcagggggcgttgtaacaaaaagggagaacaagttggtatgtcaagaccaggcctaaagcctgatcttacgggaacatcaaaatcctatgtaaggtcgctctgatcctctacaactcttgaaacacaaatgtcccacaagtctcctcttcgtcatcaagcaaccaccgcacccagcatcaagcccacctgaaattatctccggcttccctctggccgaacaatatcggtagttaatcaaaacttagggtgcaagatcatccacaatgtcaccacaacgagaccggataaatgccttctacaaagataacccccatcccaagggaagtaggatagtcattaacagagaacatcttatgattgatagaccttatgttttgctggctgttctgtttgtcatgtttctgagcttgatcgggttgctagccattgcaggcattagacttcatcgggcagccatctacaccgcagagatccataaaagcctcagcaccaatctagatgtaactaactcaatcgagcatcaggtcaaggacgtgctgacaccactcttcaaaatcatcggtgatgaagtgggcctgaggacacctcagagattcactgacctagtgaaattaatctctgacaagattaaattccttaatccggatagggagtacgacttcagagatctcacttggtgtatcaacccgccagagagaatcaaattggattatgatcaatactgtgcagatgtggctgctgaagagctcatgaatgcattggtgaactcaactctactggagaccagaacaaccaatcagttcctagctgtctcaaagggaaactgctcagggcccactacaatcagaggtcaattctcaaacatgtcgctgtccctgttagacttgtatttaggtcgaggttacaatgtgtcatctatagtcactatgacatcccagggaatgtatgggggaacttacctagtggaaaagcctaatctgagcagcaaaaggtcagagttgtcacaactgagcatgtaccgagtgtttgaagtaggtgttatcagaaatccgggtttgggggctccggtgttccatatgacaaactatcttgagcaaccagtcagtaatgatctcagcaactgtatggtggctttgggggagctcaaactcgcagccctttgtcacggggaagattctatcacaattccctatcagggatcagggaaaggtgtcagcttccagctcgtcaagctaggtgtctggaaatccccaaccgacatgcaatcctgggtccccttatcaacggatgatccagtgatagacaggctttacctctcatctcacagaggtgttatcgctgacaatcaagcaaaatgggctgtcccgacaacacgaacagatgacaagttgcgaatggagacatgcttccaacaggcgtgtaagggtaaaatccaagcactctgcgagaatcccgagtgggcaccattgaaggataacaggattccttcatacggggtcttgtctgttgatctgagtctgacagttgagcttaaaatcaaaattgcttcgggattcgggccattgatcacacacggttcagggatggacctatacaaatccaaccacaacaatgtgtattggctgactatcccgccaatgaagaacctagccttaggtgtaatcaacacattggagtggataccgagattcaaggttagtccctacctcttcactgtcccaattaaggaagcaggcgaagactgccatgccccaacatacctacctgcggaggtggatggtgatgtcaaactcagttccaatctggtgattctacctggtcaagatctccaatatgttttggcaacctacgatacttccagggttgaacatgctgtggtttattacgtttacagcccaagccgctcattttcttacttttatccttttaggttgcctataaagggggtccccatcgaattacaagtggaatgcttcacatgggaccaaaaactctggtgccgtcacttctgtgtgcttgcggactcagaatctggtggacatatcactcactctgggatggtgggcatgggagtcagctgcacagtcacccgggaagatggaaccaatcgcagatagggctgctagtgaaccaatcacatgatgtcacccagacatcaggcatacccactagtctaccctccatcattgttataaaaaacttaggaaccaggtccacacagccgccagcccatcaacgcgtacgatggcatcacaggagggaccactgcccgaaattgaggacgaagtgtttagaaagcgaaatctgactattatggacctgcaccccggatctggcaagacccggagatacctgccagccatcgtgagggaggctattaagcggaaactgagaacactgatcctggccccaactcgcgtggtcgcttccgaaatggctgaggccctgaaaggcatgcccatccggtatcagaccacagcagtgaagtctgaacataccggcaaggagattgtggacctgatgtgccacgccactttcaccatgcgactgctgagcccagtgcgggtccccaactacaatatgatcattatggacgaggcccactttactgatcccagctccatcgccgctagaggatatatttccaccagggtgggaatgggcgaggcagcagctatcttcatgacagcaactccccctggcagcgtggaggcatttcctcagtccaacgccgtcatccaggacgaggagcgggacattcctgagcggagctggaattctgggtacgaatggatcacagacgaggatcatgcacactggactgaagccaagatgctgctggacaacattaatactcctgagggaatcattccagctctgttcgagcccgaaagagagaagtctgcagccatcgacggcgagtatagactgaggggagaggcccggaagaccttcgtggaactgatgaggcgcggcgatctgcccgtgtggctgagttacaaggtcgcttcagagggattccagtatagtgaccgacggtggtgctttgatggcgaacgcaacaatcaggtgctggaggagaacatggatgtcgagatttggacaaaggaaggcgagcggaagaaactgcgcccacgatggctggacgctcggacttacagcgatcccctggcactgagagaattcaaagagtttgctgcaggggtggccgtcgagaatcaccatcacgccgctatgctggacgtggatctgcatcctgccagtgcttggaccctgtatgcagtggccactaccatcattaccccaatgatgcgccacacaatcgagaacacaactgccaatatctcactgacagctattgcaaaccaggcagccattctgatgggactggacaaaggctggcccatcagcaagatggatattggcgtgcctctgctggccctggggtgttacagtcaggtgctggacatcattggccagaggatcgagaacattaagcatgagcacaaatcaacctggcattacgacgaagataatccctataagacatgggcctaccacggaagctatgaggtgaaaccttcaggcagcgccagcagcatggtcaacggggtggtcaagctgctgaccaaaccttgggacgtgatcccaatggtcactcagattgccatgaccgataccaccccattcggccagcagcgggtgttcaaggagaaggtggacacccgcacacctaaggctaaacgagggactgcacagatcatggaggtgaccgccaagtggctgtggggattcctgtccaggaacaagaagccaagaatctgtaccagggaagagttcacaagaaaggtccggtcaaacgcctaatgagcgcgcagcgcttagacgtctcgcgatcgatgctagtgtgaaatagacatcagaattaagaaaaacgtagggtccaagtggttccccgttatggactcgctatctgtcaaccagatcttataccctgaagttcacctagatagcccgatagttaccaataagatagtagccatcctggagtatgctcgagtccctcacgcttacagcctggaggaccctacactgtgtcagaacatcaagcaccgcctaaaaaacggattttccaaccaaatgattataaacaatgtggaagttgggaatgtcatcaagtccaagcttaggagttatccggcccactctcatattccatatccaaattgtaatcaggatttatttaacatagaagacaaagagtcaacgaggaagatccgtgaactcctcaaaaaggggaattcgctgtactccaaagtcagtgataaggttttccaatgcttaagggacactaactcacggcttggcctaggctccgaattgagggaggacatcaaggagaaagttattaacttgggagtttacatgcacagctcccagtggtttgagccctttctgttttggtttacagtcaagactgagatgaggtcagtgattaaatcacaaacccatacttgccataggaggagacacacacctgtattcttcactggtagttcagttgagttgctaatctctcgtgaccttgttgctataatcagtaaagagtctcaacatgtatattacctgacatttgaactggttttgatgtattgtgatgtcatagaggggaggttaatgacagagaccgctatgactattgatgctaggtatacagagcttctaggaagagtcagatacatgtggaaactgatagatggtttcttccctgcactcgggaatccaacttatcaaattgtagccatgctggagcctctttcacttgcttacctgcagctgagggatataacagtagaactcagaggtgctttccttaaccactgctttactgaaatacatgatgttcttgaccaaaacgggttttctgatgaaggtacttatcatgagttaactgaagctctagattacattttcataactgatgacatacatctgacaggggagattttctcatttttcagaagtttcggccaccccagacttgaagcagtaacggctgctgaaaatgttaggaaatacatgaatcagcctaaagtcattgtgtatgagactctgatgaaaggtcatgccatattttgtggaatcataatcaacggctatcgtgacaggcacggaggcagttggccaccgctgaccctccccctgcatgctgcagacacaatccggaatgctcaagcttcaggtgaagggttaacacatgagcagtgcgttgataactggaaatcttttgctggagtgaaatttggctgctttatgcctcttagcctggatagtgatctgacaatgtacctaaaggacaaggcacttgctgctctccaaagggaatgggattcagtttacccgaaagagttcctgcgttacgaccctcccaagggaaccgggtcacggaggcttgtagatgttttccttaatgattcgagctttgacccatatgatgtgataatgtatgttgtaagtggagcttacctccatgaccctgagttcaacctgtcttacagcctgaaagaaaaggagatcaaggaaacaggtagactttttgctaaaatgacttacaaaatgagggcatgccaagtgattgctgaaaatctaatctcaaacgggattggcaaatattttaaggacaatgggatggccaaggatgagcacgatttgactaaggcactccacactctagctgtctcaggagtccccaaagatctcaaagaaagtcacaggggggggccagtcttaaaaacctactcccgaagcccagtccacacaagtaccaggaacgtgagagcagcaaaagggtttatagggttccctcaagtaattcggcaggaccaagacactgatcatccggagaatatggaagcttacgagacagtcagtgcatttatcacgactgatctcaagaagtactgccttaattggagatatgagaccatcagcttgtttgcacagaggctaaatgagatttacggattgccctcatttttccagtggctgcataagaggcttgagacctctgtcctgtatgtaagtgaccctcattgcccccccgaccttgacgcccatatcccgttatataaagtccccaatgatcaaatcttcattaagtaccctatgggaggtatagaagggtattgtcagaagctgtggaccatcagcaccattccctatctatacctggctgcttatgagagcggagtaaggattgcttcgttagtgcaaggggacaatcagaccatagccgtaacaaaaagggtacccagcacatggccctacaaccttaagaaacgggaagctgctagagtaactagagattactttgtaattcttaggcaaaggctacatgatattggccatcacctcaaggcaaatgagacaattgtttcatcacatttttttgtctattcaaaaggaatatattatgatgggctacttgtgtcccaatcactcaagagcatcgcaagatgtgtattctggtcagagactatagttgatgaaacaagggcagcatgcagtaatattgctacaacaatggctaaaagcatcgagagaggttatgaccgttaccttgcatattccctgaacgtcctaaaagtgatacagcaaattctgatctctcttggcttcacaatcaattcaaccatgacccgggatgtagtcatacccctcctcacaaacaacgacctcttaataaggatggcactgttgcccgctcctattggggggatgaattatctgaatatgagcaggctgtttgtcagaaacatcggtgatccagtaacatcatcaattgctgatctcaagagaatgattctcgcctcactaatgcctgaagagaccctccatcaagtaatgacacaacaaccgggggactcttcattcctagactgggctagcgacccttactcagcaaatcttgtatgtgtccagagcatcactagactcctcaagaacataactgcaaggtttgtcctgatccatagtccaaacccaatgttaaaaggattattccatgatgacagtaaagaagaggacgagggactggcggcattcctcatggacaggcatattatagtacctagggcagctcatgaaatcctggatcatagtgtcacaggggcaagagagtctattgcaggcatgctggataccacaaaaggcttgattcgagccagcatgaggaagggggggttaacctctcgagtgataaccagattgtccaattatgactatgaacaattcagagcagggatggtgctattgacaggaagaaagagaaatgtcctcattgacaaagagtcatgttcagtgcagctggcgagagctctaagaagccatatgtgggcgaggctagctcgaggacggcctatttacggccttgaggtccctgatgtactagaatctatgcgaggccaccttattcggcgtcatgagacatgtgtcatctgcgagtgtggatcagtcaactacggatggttttttgtcccctcgggttgccaactggatgatattgacaaggaaacatcatccttgagagtcccatatattggttctaccactgatgagagaacagacatgaagcttgccttcgtaagagccccaagtcgatccttgcgatctgctgttagaatagcaacagtgtactcatgggcttacggtgatgatgatagctcttggaacgaagcctggttgttggctaggcaaagggccaatgtgagcctggaggagctaagggtgatcactcccatctcaacttcgactaatttagcgcataggttgagggatcgtagcactcaagtgaaatactcaggtacatcccttgtccgagtggcgaggtataccacaatctccaacgacaatctctcatttgtcatatcagataagaaggttgatactaactttatataccaacaaggaatgcttctagggttgggtgttttagaaacattgtttcgactcgagaaagataccggatcatctaacacggtattacatcttcacgtcgaaacagattgttgcgtgatcccgatgatagatcatcccaggatacccagctcccgcaagctagagctgagggcagagctatgtaccaacccattgatatatgataatgcacctttaattgacagagatgcaacaaggctatacacccagagccataggaggcaccttgtggaatttgttacatggtccacaccccaactatatcacattttagctaagtccacagcactatctatgattgacctggtaacaaaatttgagaaggaccatatgaatgaaatttcagctctcataggggatgacgatatcaatagtttcataactgagtttctgctcatagagccaagattattcactatctacttgggccagtgtgcggccatcaattgggcatttgatgtacattatcatagaccatcagggaaatatcagatgggtgagctgttgtcatcgttcctttctagaatgagcaaaggagtgtttaaggtgcttgtcaatgctctaagccacccaaagatctacaagaaattctggcattgtggtattatagagcctatccatggtccttcacttgatgctcaaaacttgcacacaactgtgtgcaacatggtttacacatgctatatgacctacctcgacctgttgttgaatgaagagttagaagagttcacatttctcttgtgtgaaagcgacgaggatgtagtaccggacagattcgacaacatccaggcaaaacacttatgtgttctggcagatttgtactgtcaaccagggacctgcccaccaattcgaggtctaagaccggtagagaaatgtgcagttctaaccgaccatatcaaggcagaggctatgttatctccagcaggatcttcgtggaacataaatccaattattgtagaccattactcatgctctctgacttatctccggcgaggatcgatcaaacagataagattgagagttgatccaggattcattttcgacgccctcgctgaggtaaatgtcagtcagccaaagatcggcagcaacaacatctcaaatatgagcatcaaggctttcagacccccacacgatgatgttgcaaaattgctcaaagatatcaacacaagcaagcacaatcttcccatttcagggggcaatctcgccaattatgaaatccatgctttccgcagaatcgggttgaactcatctgcttgctacaaagctgttgagatatcaacattaattaggagatgccttgagccaggggaggacggcttgttcttgggtgagggatcgggttctatgttgatcacttataaagagatacttaaactaaacaagtgcttctataatagtggggtttccgccaattctagatctggtcaaagggaattagcaccctatccctccgaagttggccttgtcgaacacagaatgggagtaggtaatattgtcaaagtgctctttaacgggaggcccgaagtcacgtgggtaggcagtgtagattgcttcaatttcatagttagtaatatccctacctctagtgtggggtttatccattcagatatagagaccttgcctgacaaagatactatagagaagctagaggaattggcagccatcttatcgatggctctgctcctgggcaaaataggatcaatactggtgattaagcttatgcctttcagcggggattttgttcagggatttataagttatgtagggtctcattatagagaagtgaaccttgtataccctagatacagcaacttcatctctactgaatcttatttggttatgacagatctcaaggctaaccggctaatgaatcctgaaaagattaagcagcagataattgaatcatctgtgaggacttcacctggacttataggtcacatcctatccattaagcaactaagctgcatacaagcaattgtgggagacgcagttagtagaggtgatatcaatcctactctgaaaaaacttacacctatagagcaggtgctgatcaattgcgggttggcaattaacggacctaagctgtgcaaagaattgatccaccatgatgttgcctcagggcaagatggattgcttaattctatactcatcctctacagggagttggcaagattcaaagacaaccaaagaagtcaacaagggatgttccacgcttaccccgtattggtaagtagcaggcaacgagaacttatatctaggatcacccgcaaattctgggggcacattcttctttactccgggaacaaaaagttgataaataagtttatccagaatctcaagtccggctatctgatactagacttacaccagaatatcttcgttaagaatctatccaagtcagagaaacagattattatgacggggggtttgaaacgtgagtgggtttttaaggtaacagtcaaggagaccaaagaatggtataagttagtcggatacagtgccctgattaaggactaattggttgaactccggaaccctaatcctgccctaggtggttaggcattatttgcaatatattaaagaaaactttgaaaatacgaagtttctattcccagctttgtctggtggccggcatggtcccagcctcctcgctggcgccggctgggcaacattccgaggggaccgtcccctcggtaatggcgaatgggacgcggccgatccggctgctaacaaagcccgaaaggaagctgagttggctgctgccaccgctgagcaataactagcataaccccttggggcctctaaacgggtcttgaggggttttttgctgaaaggaggaactatatccggatgcggccgcgggccctatggtacccagcttttgttccctttagtgagggttaattccgagcttggcgtaatcatggtcatagctgtttcctgtgtgaaattgttatccgctcacaattccacacaacataggagccggaagcataaagtgtaaagcctggggtgcctaatgagtgaggtaactcacattaattgcgttgcgctcactgcccgctttccagtcgggaaacctgtcgtgccagctgcattaatgaatcggccaacgcgcggggagaggcggtttgcgtattgggcgctcttccgcttcctcgctcactgactcgctgcgctcggtcgttcggctgcggcgagcggtatcagctcactcaaaggcggtaatacggttatccacagaatcaggggataacgcaggaaagaacatgtgagcaaaaggccagcaaaaggccaggaaccgtaaaaaggccgcgttgctggcgtttttccataggctcggcccccctgacgagcatcacaaaaatcgacgctcaagtcagaggtggcgaaacccgacaggactataaagataccaggcgttcccccctggaagctccctcgtgcgctctcctgttccgaccctgccgcttaccggatacctgtccgcctttctcccttcgggaagcgtggcgctttctcaatgctcacgctgtaggtatctcagttcggtgtaggtcgttcgctccaagctgggctgtgtgcacgaaccccccgttcagcccgaccgctgcgccttatccggtaactatcgtcttgagtccaacccggtaagacacgacttatcgccactggcagcagccactggtaacaggattagcagagcgaggtatgtaggcggtgctacagagttcttgaagtggtggcctaactacggctacactagaaggacagtatttggtatctgcgctctgctgaagccagttaccttcggaaaaagagttggtagctcttgatccggcaaacaaaccaccgctggtagcggtggtttttttgtttgcaagcagcagattacgcgcagaaaaaaaggatctcaagaagatcctttgatcttttctacggggtctgacgctcagtggaacgaaaactcacgttaagggattttggtcatgagattatcaaaaaggatcttcacctagatccttttaaattaaaaatgaagttttaaatcaatctaaagtatatatgagtaaacttggtctgacagttaccaatgcttaatcagtgaggcacctatctcagcgatctgtctatttcgttcatccatagttgcctgactgcccgtcgtgtagataactacgatacgggagggcttaccatctggccccagtgctgcaatgataccgcgagacccacgctcaccggctccagatttatcagcaataaaccagccagccggaagggccgagcgcagaagtggtcctgcaactttatccgcctccatccagtctattaattgttgccgggaagctagagtaagtagttcgccagttaatagtttgcgcaacgttgttgccattgctacaggcatcgtggtgtcacgctcgtcgtttggtatggcttcattcagctccggttcccaacgatcaaggcgagttacatgatcccccatgttgtgaaaaaaagcggttagctccttcggtcctccgatcgttgtcagaagtaagttggccgcagtgttatcactcatgcttatggcagcactgcataattctcttactgtcatgccatccgtaagatgcttttctgtgactggtgagtactcaaccaagtcattctgagaatagtgtatgcggcgaccgagttgctcttgcccggcgtcaatacgggataataccgcgccacatagcagaactttaaaagtgctcatcattggaaaacgttcttcggggcgaaaactctcaaggatcttaccgctgttgagatccagttcgatgtaacccactcgtgcacccaactgatcttcagcatcttttactttcaccagcgtttctgggtgagcaaaaacaggaaggcaaaatgccgcaaaaaagggaataagggcgacacggaaatgttgaatactcatactcttcctttttcaatattattgaagcatttatcagggttattgtctcatgagcggatacatatttgaatgtatttagaaaaataaacaaataggggttccgcgcacatttccccgaaaagtgccacctgaaattgtaaacgttaatattttgttaaaattcgcgttaaatttttgttaaatcagctcattttttaaccaataggccgaaatcggcaaaatcccttataaatcaaaagaatagaccgagatagggttgagtgttgttccagtttggaacaagagtccactattaaagaacgtggactccaacgtcaaagggcgaaaaaccgtctatcagggcgatggcccactacgtgaaccatcaccctaatcaagttttttggggtcgaggtgccgtaaagcactaaatcggaaccctaaagggagcccccgatttagagcttgacggggaaagccggcgaacgtggcgagaaaggaagggaagaaagcgaaaggagcgggcgctagggcgctggcaagtgtagcggtcacgctgcgcgtaaccaccacacccgccgcgcttaatgcgccgctacagggcgcgtcccattcgccattcaggctgcgcaactgttgggaagggcgatcggtgcgggcctcttcgctattacgccagccaccgcggtg

SEQ ID NO: 140 - DNA, 20701 bp, Artificial Sequence
  Complete optimised nucleotide sequence of the polynucleotide encoding pTM-MVDVax7
  misc_feature (1)..(8): NotI
  misc_feature (9)..(28): T7 promoter
  misc_feature (29)..(82): Hammerhead ribozyme
  misc_feature (83)..(189): MV Leader and N promoter
  misc_feature (190)..(1767): MV N ORF
  misc_feature (1768)..(1888): MV N-P intergenic
  misc_feature (1889)..(3412): MV P ORF
  misc_feature (3413)..(3531): MV ATU2
  misc_feature (3532)..(5154): DENV1 NS polyepitope
  misc_feature (5155)..(5253): MV P-M intergenic
  misc_feature (5254)..(6261): MV M ORF
  misc_feature (6262)..(7264): MV M-F intergenic
  misc_feature (7265)..(8926): MV F ORF
  misc_feature (8927)..(9086): MV-F-H intergenic
  misc_feature (9087)..(10940): MV H ORF
  misc_feature (10941)..(11049): MV H-L intergenic
  misc_feature (11050)..(17601): MV L ORF
  misc_feature (17602)..(17710): MV Trailer
  misc_feature (17711)..(17794): HDV ribozyme
  misc_feature (17795)..(17936): T7 terminator
  misc_feature (17937)..(17944): Not I
  misc_feature (17945)..(20701): pTM plasmid
gcggccgctaatacgactcactatagggccaactttgtttggtctgatgagtccgtgaggacgaaacccggagtcccgggtcaccaaacaaagttgggtaaggatagttcaatcaatgatcatcttctagtgcacttaggattcaagatcctattatcagggacaagagcaggattagggatatccgagatggccacacttttaaggagcttagcattgttcaaaagaaacaaggacaaaccacccattacatcaggatccggtggagccatcagaggaatcaaacacattattatagtaccaatccctggagattcctcaattaccactcgatccagacttctggaccggttggtgaggttaattggaaacccggatgtgagcgggcccaaactaacaggggcactaataggtatattatccttatttgtggagtctccaggtcaattgattcagaggatcaccgatgaccctgacgttagcataaggctgttagaggttgtccagagtgaccagtcacaatctggccttaccttcgcatcaagaggtaccaacatggaggatgaggcggaccaatacttttcacatgatgatccaattagtagtgatcaatccaggttcggatggttcgggaacaaggaaatctcagatattgaagtgcaagaccctgagggattcaacatgattctgggtaccatcctagcccaaatttgggtcttgctcgcaaaggcggttacggccccagacacggcagctgattcggagctaagaaggtggataaagtacacccaacaaagaagggtagttggtgaatttagattggagagaaaatggttggatgtggtgaggaacaggattgccgaggacctctccttacgccgattcatggtcgctctaatcctggatatcaagagaacacccggaaacaaacccaggattgctgaaatgatatgtgacattgatacatatatcgtagaggcaggattagccagttttatcctgactattaagtttgggatagaaactatgtatcctgctcttggactgcatgaatttgctggtgagttatccacacttgagtccttgatgaacctttaccagcaaatgggggaaactgcaccctacatggtaatcctggagaactcaattcagaacaagttcagtgcaggatcataccctctgctctggagctatgccatgggagtaggagtggaacttgaaaactccatgggaggtttgaactttggccgatcttactttgatccagcatattttagattagggcaagagatggtaaggaggtcagctggaaaggtcagttccacattggcatctgaactcggtatcactgccgaggatgcaaggcttgtttcagagattgcaatgcatactactgaggacaagatcagtagagcggttggacccagacaagcccaagtatcatttctacacggtgatcaaagtgagaatgagctaccgagattggggggcaaggaagataggagggtcaaacagagtcgaggagaagccagggagagctacagagaaaccgggcccagcagagcaagtgatgcgagagctgcccatcttccaaccggcacacccctagacattgacactgcaacggagtccagccaagatccgcaggacagtcgaaggtcagctgacgccctgcttaggctgcaagccatggcaggaatctcggaagaacaaggctcagacacggacacccctatagtgtacaatgacagaaatcttctagactaggtgcgagaggccgagggccagaacaacatccgcctaccatccatcattgttataaaaaacttaggaaccaggtccacacagccgccagcccatcaaccatccactcccacgattggagccaatggcagaagagcaggcacgccatgtcaaaaacggactggaatgcatccgggctctcaaggccgagcccatcggctcactggccatcgaggaagctatggcagcatggtcagaaatatcagacaacccaggacaggagcgagccacctgcagggaagagaaggcaggcagttcgggtctcagcaaaccatgcctctcagcaattggatcaactgaaggcggtgcacctcgcatccgcggtcagggacctggagagagcgatgacgacgctgaaactttgggaatccccccaagaaatctccaggcatcaagcactgggttacagtgttattacgtttatgatcacagcggtgaagcggttaagggaatccaagatgctgactctatcatggttcaatcaggccttgatggtgatagcaccctctcaggaggagacaatgaatctgaaaacagcgatgtggatattggcgaacctgataccgagggatatgctatcactgaccggggatctgctcccatctctatggggttcagggcttctgatgttgaaactgcagaaggaggggagatccacgagctcctgagactccaatccagaggcaacaactttccgaagcttgggaaaactctcaatgttcctccgcccccggaccccggtagggccagcacttccgggacacccattaaaaagggcacagacgcgagattagcctcatttggaacggagatcgcgtctttattgacaggtggtgcaacccaatgtgctcgaaagtcaccctcggaaccatcagggccaggtgcacctgcggggaatgtccccgagtgtgtgagcaatgccgcactgatacaggagtggacacccgaatctggtaccacaatctccccgagatcccagaataatgaagaagggggagactattatgatgatgagctgttctctgatgtccaagatattaaaacagccttggccaaaatacacgaggataatcagaagataatctccaagctagaatcactgctgttattgaagggagaagttgagtcaattaagaagcagatcaacaggcaaaatatcagcatatccaccctggaaggacacctctcaagcatcatgatcgccattcctggacttgggaaggatcccaacgaccccactgcagatgtcgaaatcaatcccgacttgaaacccatcataggcagagattcaggccgagcactggccgaagttctcaagaaacccgttgccagccgacaactccaaggaatgacaaatggacggaccagttccagaggacagctgctgaaggaatttcagctaaagccgatcgggaaaaagatgagctcagccgtcgggtttgttcctgacaccggccctgcatcacgcagtgtaatccgctccattataaaatccagccggctagaggaggatcggaagcgttacctgatgactctccttgatgatatcaaaggagccaatgatcttgccaagttccaccagatgctgatgaagataataatgaagtagctacagctcaacttacctgccaaccccatgccagtcgacccaactagcctaccctccatcattgttataaaaaacttaggaaccaggtccacacagccgccagcccatcaacgcgtacgatggcatcacaggagggaccactgcccgaaattgaggacgaagtgtttagaaagcgaaatctgactattatggacctgcaccccggatctggcaagacccggagatacctgccagccatcgtgagggaggctattaagcggaaactgagaacactgatcctggccccaactcgcgtggtcgcttccgaaatggctgaggccctgaaaggcatgcccatccggtatcagaccacagcagtgaagtctgaacataccggcaaggagattgtggacctgatgtgccacgccactttcaccatgcgactgctgagcccagtgcgggtccccaactacaatatgatcattatggacgaggcccactttactgatcccagctccatcgccgctagaggatatatttccaccagggtgggaatgggcgaggcagcagctatcttcatgacagcaactccccctggcagcgtggaggcatttcctcagtccaacgccgtcatccaggacgaggagcgggacattcctgagcggagctggaattctgggtacgaatggatcacagacgaggatcatgcacactggactgaagccaagatgctgctggacaacattaatactcctgagggaatcattccagctctgttcgagcccgaaagagagaagtctgcagccatcgacggcgagtatagactgaggggagaggcccggaagaccttcgtggaactgatgaggcgcggcgatctgcccgtgtggctgagttacaaggtcgcttcagagggattccagtatagtgaccgacggtggtgctttgatggcgaacgcaacaatcaggtgctggaggagaacatggatgtcgagatttggacaaaggaaggcgagcggaagaaactgcgcccacgatggctggacgctcggacttacagcgatcccctggcactgagagaattcaaagagtttgctgcaggggtggccgtcgagaatcaccatcacgccgctatgctggacgtggatctgcatcctgccagtgcttggaccctgtatgcagtggccactaccatcattaccccaatgatgcgccacacaatcgagaacacaactgccaatatctcactgacagctattgcaaaccaggcagccattctgatgggactggacaaaggctggcccatcagcaagatggatattggcgtgcctctgctggccctggggtgttacagtcaggtgctggacatcattggccagaggatcgagaacattaagcatgagcacaaatcaacctggcattacgacgaagataatccctataagacatgggcctaccacggaagctatgaggtgaaaccttcaggcagcgccagcagcatggtcaacggggtggtcaagctgctgaccaaaccttgggacgtgatcccaatggtcactcagattgccatgaccgataccaccccattcggccagcagcgggtgttcaaggagaaggtggacacccgcacacctaaggctaaacgagggactgcacagatcatggaggtgaccgccaagtggctgtggggattcctgtccaggaacaagaagccaagaatctgtaccagggaagagttcacaagaaaggtccggtcaaacgcctaatgagcgcgcagcgcttagacgtctcgcgatcgatactagtacaacctaaatccattataaaaaacttaggagcaaagtgattgcctcccaaggtccacaatgacagagacctacgacttcgacaagtcggcatgggacatcaaagggtcgatcgctccgatacaacccaccacctacagtgatggcaggctggtgccccaggtcagagtcatagatcctggtctaggcgacaggaaggatgaatgctttatgtacatgtttctgctgggggttgttgaggacagcgattccctagggcctccaatcgggcgagcatttgggttcctgcccttaggtgttggcagatccacagcaaagcccgaaaaactcctcaaagaggccactgagcttgacatagttgttagacgtacagcagggctcaatgaaaaactggtgttctacaacaacaccccactaactctcctcacaccttggagaaaggtcctaacaacagggagtgtcttcaacgcaaaccaagtgtgcaatgcggttaatctgataccgctcgataccccgcagaggttccgtgttgtttatatgagcatcacccgtctttcggataacgggtattacaccgttcctagaagaatgctggaattcagatcggtcaatgcagtggccttcaacctgctggtgacccttaggattgacaaggcgataggccctgggaagatcatcgacaatacagagcaacttcctgaggcaacatttatggtccacatcgggaacttcaggagaaagaagagtgaagtctactctgccgattattgcaaaatgaaaatcgaaaagatgggcctggtttttgcacttggtgggatagggggcaccagtcttcacattagaagcacaggcaaaatgagcaagactctccatgcacaactcgggttcaagaagaccttatgttacccgctgatggatatcaatgaagaccttaatcgattactctggaggagcagatgcaagatagtaagaatccaggcagttttgcagccatcagttcctcaagaattccgcatttacgacgacgtgatcataaatgatgaccaaggactattcaaagttctgtagaccgtagtgcccagcaatgcccgaaaacgacccccctcacaatgacagccagaaggcccggacaaaaaagccccctccgaaagactccacggaccaagcgagaggccagccagcagccgacggcaagcgcgaacaccaggcggccccagcacagaacagccctgacacaaggccaccaccagccaccccaatctgcatcctcctcgtgggacccccgaggaccaacccccaaggctgcccccgatccaaaccaccaaccgcatccccaccacccccgggaaagaaacccccagcaattggaaggcccctccccctcttcctcaacacaagaactccacaaccgaaccgcacaagcgaccgaggtgacccaaccgcaggcatccgactccctagacagatcctctctccccggcaaactaaacaaaacttagggccaaggaacatacacacccaacagaacccagaccccggcccacggcgccgcgcccccaacccccgacaaccagagggagcccccaaccaatcccgccggctcccccggtgcccacaggcagggacaccaacccccgaacagacccagcacccaaccatcgacaatccaagacgggggggcccccccaaaaaaaggcccccaggggccgacagccagcaccgcgaggaagcccacccaccccacacacgaccacggcaaccaaaccagaacccagaccaccctgggccaccagctcccagactcggccatcaccccgcagaaaggaaaggccacaacccgcgcaccccagccccgatccggcggggagccacccaacccgaaccagcacccaagagcgatccccgaaggacccccgaaccgcaaaggacatcagtatcccacagcctctccaagtcccccggtctcctcctcttctcgaagggaccaaaagatcaatccaccacacccgacgacactcaactccccacccctaaaggagacaccgggaatcccagaatcaagactcatccaatgtccatcatgggtctcaaggtgaacgtctctgccatattcatggcagtactgttaactctccaaacacccaccggtcaaatccattggggcaatctctctaagataggggtggtaggaataggaagtgcaagctacaaagttatgactcgttccagccatcaatcattagtcataaaattaatgcccaatataactctcctcaataactgcacgagggtagagattgcagaatacaggagactactgagaacagttttggaaccaattagagatgcacttaatgcaatgacccagaatataagaccggttcagagtgtagcttcaagtaggagacacaagagatttgcgggagtagtcctggcaggtgcggccctaggcgttgccacagctgctcagataacagccggcattgcacttcaccagtccatgctgaactctcaagccatcgacaatctgagagcgagcctggaaactactaatcaggcaattgagacaatcagacaagcagggcaggagatgatattggctgttcagggtgtccaagactacatcaataatgagctgataccgtctatgaaccaactatcttgtgatttaatcggccagaagctcgggctcaaattgctcagatactatacagaaatcctgtcattatttggccccagtttacgggaccccatatctgcggagatatctatccaggctttgagctatgcgcttggaggagacatcaataaggtgttagaaaagctcggatacagtggaggtgatttactgggcatcttagagagcggaggaataaaggcccggataactcacgtcgacacagagtcctacttcattgtcctcagtatagcctatccgacgctgtccgagattaagggggtgattgtccaccggctagagggggtctcgtacaacataggctctcaagagtggtataccactgtgcccaagtatgttgcaacccaagggtaccttatctcgaattttgatgagtcatcgtgtactttcatgccagaggggactgtgtgcagccaaaatgccttgtacccgatgagtcctctgctccaagaatgcctccgggggtacaccaagtcctgtgctcgtacactcgtatccgggtcttttgggaaccggttcattttatcacaagggaacctaatagccaattgtgcatcaatcctttgcaagtgttacacaacaggaacgatcattaatcaagaccctgacaagatcctaacatacattgctgccgatcactgcccggtagtcgaggtgaacggcgtgaccatccaagtcgggagcaggaggtatccagacgctgtgtacttgcacagaattgacctcggtcctcccatatcattggagaggttggacgtagggacaaatctggggaatgcaattgctaagttggaggatgccaaggaattgttggagtcatcggaccagatattgaggagtatgaaaggtttatcgagcactagcatagtctacatcctgattgcagtgtgtcttggagggttgatagggatccccgctttaatatgttgctgcagggggcgttgtaacaaaaagggagaacaagttggtatgtcaagaccaggcctaaagcctgatcttacgggaacatcaaaatcctatgtaaggtcgctctgatcctctacaactcttgaaacacaaatgtcccacaagtctcctcttcgtcatcaagcaaccaccgcacccagcatcaagcccacctgaaattatctccggcttccctctggccgaacaatatcggtagttaatcaaaacttagggtgcaagatcatccacaatgtcaccacaacgagaccggataaatgccttctacaaagataacccccatcccaagggaagtaggatagtcattaacagagaacatcttatgattgatagaccttatgttttgctggctgttctgtttgtcatgtttctgagcttgatcgggttgctagccattgcaggcattagacttcatcgggcagccatctacaccgcagagatccataaaagcctcagcaccaatctagatgtaactaactcaatcgagcatcaggtcaaggacgtgctgacaccactcttcaaaatcatcggtgatgaagtgggcctgaggacacctcagagattcactgacctagtgaaattaatctctgacaagattaaattccttaatccggatagggagtacgacttcagagatctcacttggtgtatcaacccgccagagagaatcaaattggattatgatcaatactgtgcagatgtggctgctgaagagctcatgaatgcattggtgaactcaactctactggagaccagaacaaccaatcagttcctagctgtctcaaagggaaactgctcagggcccactacaatcagaggtcaattctcaaacatgtcgctgtccctgttagacttgtatttaggtcgaggttacaatgtgtcatctatagtcactatgacatcccagggaatgtatgggggaacttacctagtggaaaagcctaatctgagcagcaaaaggtcagagttgtcacaactgagcatgtaccgagtgtttgaagtaggtgttatcagaaatccgggtttgggggctccggtgttccatatgacaaactatcttgagcaaccagtcagtaatgatctcagcaactgtatggtggctttgggggagctcaaactcgcagccctttgtcacggggaagattctatcacaattccctatcagggatcagggaaaggtgtcagcttccagctcgtcaagctaggtgtctggaaatccccaaccgacatgcaatcctgggtccccttatcaacggatgatccagtgatagacaggctttacctctcatctcacagaggtgttatcgctgacaatcaagcaaaatgggctgtcccgacaacacgaacagatgacaagttgcgaatggagacatgcttccaacaggcgtgtaagggtaaaatccaagcactctgcgagaatcccgagtgggcaccattgaaggataacaggattccttcatacggggtcttgtctgttgatctgagtctgacagttgagcttaaaatcaaaattgcttcgggattcgggccattgatcacacacggttcagggatggacctatacaaatccaaccacaacaatgtgtattggctgactatcccgccaatgaagaacctagccttaggtgtaatcaacacattggagtggataccgagattcaaggttagtccctacctcttcactgtcccaattaaggaagcaggcgaagactgccatgccccaacatacctacctgcggaggtggatggtgatgtcaaactcagttccaatctggtgattctacctggtcaagatctccaatatgttttggcaacctacgatacttccagggttgaacatgctgtggtttattacgtttacagcccaagccgctcattttcttacttttatccttttaggttgcctataaagggggtccccatcgaattacaagtggaatgcttcacatgggaccaaaaactctggtgccgtcacttctgtgtgcttgcggactcagaatctggtggacatatcactcactctgggatggtgggcatgggagtcagctgcacagtcacccgggaagatggaaccaatcgcagatagggctgctagtgaaccaatcacatgatgtcacccagacatcaggcatacccactagtgtgaaatagacatcagaattaagaaaaacgtagggtccaagtggttccccgttatggactcgctatctgtcaaccagatcttataccctgaagttcacctagatagcccgatagttaccaataagatagtagccatcctggagtatgctcgagtccctcacgcttacagcctggaggaccctacactgtgtcagaacatcaagcaccgcctaaaaaacggattttccaaccaaatgattataaacaatgtggaagttgggaatgtcatcaagtccaagcttaggagttatccggcccactctcatattccatatccaaattgtaatcaggatttatttaacatagaagacaaagagtcaacgaggaagatccgtgaactcctcaaaaaggggaattcgctgtactccaaagtcagtgataaggttttccaatgcttaagggacactaactcacggcttggcctaggctccgaattgagggaggacatcaaggagaaagttattaacttgggagtttacatgcacagctcccagtggtttgagccctttctgttttggtttacagtcaagactgagatgaggtcagtgattaaatcacaaacccatacttgccataggaggagacacacacctgtattcttcactggtagttcagttgagttgctaatctctcgtgaccttgttgctataatcagtaaagagtctcaacatgtatattacctgacatttgaactggttttgatgtattgtgatgtcatagaggggaggttaatgacagagaccgctatgactattgatgctaggtatacagagcttctaggaagagtcagatacatgtggaaactgatagatggtttcttccctgcactcgggaatccaacttatcaaattgtagccatgctggagcctctttcacttgcttacctgcagctgagggatataacagtagaactcagaggtgctttccttaaccactgctttactgaaatacatgatgttcttgaccaaaacgggttttctgatgaaggtacttatcatgagttaactgaagctctagattacattttcataactgatgacatacatctgacaggggagattttctcatttttcagaagtttcggccaccccagacttgaagcagtaacggctgctgaaaatgttaggaaatacatgaatcagcctaaagtcattgtgtatgagactctgatgaaaggtcatgccatattttgtggaatcataatcaacggctatcgtgacaggcacggaggcagttggccaccgctgaccctccccctgcatgctgcagacacaatccggaatgctcaagcttcaggtgaagggttaacacatgagcagtgcgttgataactggaaatcttttgctggagtgaaatttggctgctttatgcctcttagcctggatagtgatctgacaatgtacctaaaggacaaggcacttgctgctctccaaagggaatgggattcagtttacccgaaagagttcctgcgttacgaccctcccaagggaaccgggtcacggaggcttgtagatgttttccttaatgattcgagctttgacccatatgatgtgataatgtatgttgtaagtggagcttacctccatgaccctgagttcaacctgtcttacagcctgaaagaaaaggagatcaaggaaacaggtagactttttgctaaaatgacttacaaaatgagggcatgccaagtgattgctgaaaatctaatctcaaacgggattggcaaatattttaaggacaatgggatggccaaggatgagcacgatttgactaaggcactccacactctagctgtctcaggagtccccaaagatctcaaagaaagtcacaggggggggccagtcttaaaaacctactcccgaagcccagtccacacaagtaccaggaacgtgagagcagcaaaagggtttatagggttccctcaagtaattcggcaggaccaagacactgatcatccggagaatatggaagcttacgagacagtcagtgcatttatcacgactgatctcaagaagtactgccttaattggagatatgagaccatcagcttgtttgcacagaggctaaatgagatttacggattgccctcatttttccagtggctgcataagaggcttgagacctctgtcctgtatgtaagtgaccctcattgcccccccgaccttgacgcccatatcccgttatataaagtccccaatgatcaaatcttcattaagtaccctatgggaggtatagaagggtattgtcagaagctgtggaccatcagcaccattccctatctatacctggctgcttatgagagcggagtaaggattgcttcgttagtgcaaggggacaatcagaccatagccgtaacaaaaagggtacccagcacatggccctacaaccttaagaaacgggaagctgctagagtaactagagattactttgtaattcttaggcaaaggctacatgatattggccatcacctcaaggcaaatgagacaattgtttcatcacatttttttgtctattcaaaaggaatatattatgatgggctacttgtgtcccaatcactcaagagcatcgcaagatgtgtattctggtcagagactatagttgatgaaacaagggcagcatgcagtaatattgctacaacaatggctaaaagcatcgagagaggttatgaccgttaccttgcatattccctgaacgtcctaaaagtgatacagcaaattctgatctctcttggcttcacaatcaattcaaccatgacccgggatgtagtcatacccctcctcacaaacaacgacctcttaataaggatggcactgttgcccgctcctattggggggatgaattatctgaatatgagcaggctgtttgtcagaaacatcggtgatccagtaacatcatcaattgctgatctcaagagaatgattctcgcctcactaatgcctgaagagaccctccatcaagtaatgacacaacaaccgggggactcttcattcctagactgggctagcgacccttactcagcaaatcttgtatgtgtccagagcatcactagactcctcaagaacataactgcaaggtttgtcctgatccatagtccaaacccaatgttaaaaggattattccatgatgacagtaaagaagaggacgagggactggcggcattcctcatggacaggcatattatagtacctagggcagctcatgaaatcctggatcatagtgtcacaggggcaagagagtctattgcaggcatgctggataccacaaaaggcttgattcgagccagcatgaggaagggggggttaacctctcgagtgataaccagattgtccaattatgactatgaacaattcagagcagggatggtgctattgacaggaagaaagagaaatgtcctcattgacaaagagtcatgttcagtgcagctggcgagagctctaagaagccatatgtgggcgaggctagctcgaggacggcctatttacggccttgaggtccctgatgtactagaatctatgcgaggccaccttattcggcgtcatgagacatgtgtcatctgcgagtgtggatcagtcaactacggatggttttttgtcccctcgggttgccaactggatgatattgacaaggaaacatcatccttgagagtcccatatattggttctaccactgatgagagaacagacatgaagcttgccttcgtaagagccccaagtcgatccttgcgatctgctgttagaatagcaacagtgtactcatgggcttacggtgatgatgatagctcttggaacgaagcctggttgttggctaggcaaagggccaatgtgagcctggaggagctaagggtgatcactcccatctcaacttcgactaatttagcgcataggttgagggatcgtagcactcaagtgaaatactcaggtacatcccttgtccgagtggcgaggtataccacaatctccaacgacaatctctcatttgtcatatcagataagaaggttgatactaactttatataccaacaaggaatgcttctagggttgggtgttttagaaacattgtttcgactcgagaaagataccggatcatctaacacggtattacatcttcacgtcgaaacagattgttgcgtgatcccgatgatagatcatcccaggatacccagctcccgcaagctagagctgagggcagagctatgtaccaacccattgatatatgataatgcacctttaattgacagagatgcaacaaggctatacacccagagccataggaggcaccttgtggaatttgttacatggtccacaccccaactatatcacattttagctaagtccacagcactatctatgattgacctggtaacaaaatttgagaaggaccatatgaatgaaatttcagctctcataggggatgacgatatcaatagtttcataactgagtttctgctcatagagccaagattattcactatctacttgggccagtgtgcggccatcaattgggcatttgatgtacattatcatagaccatcagggaaatatcagatgggtgagctgttgtcatcgttcctttctagaatgagcaaaggagtgtttaaggtgcttgtcaatgctctaagccacccaaagatctacaagaaattctggcattgtggtattatagagcctatccatggtccttcacttgatgctcaaaacttgcacacaactgtgtgcaacatggtttacacatgctatatgacctacctcgacctgttgttgaatgaagagttagaagagttcacatttctcttgtgtgaaagcgacgaggatgtagtaccggacagattcgacaacatccaggcaaaacacttatgtgttctggcagatttgtactgtcaaccagggacctgcccaccaattcgaggtctaagaccggtagagaaatgtgcagttctaaccgaccatatcaaggcagaggctatgttatctccagcaggatcttcgtggaacataaatccaattattgtagaccattactcatgctctctgacttatctccggcgaggatcgatcaaacagataagattgagagttgatccaggattcattttcgacgccctcgctgaggtaaatgtcagtcagccaaagatcggcagcaacaacatctcaaatatgagcatcaaggctttcagacccccacacgatgatgttgcaaaattgctcaaagatatcaacacaagcaagcacaatcttcccatttcagggggcaatctcgccaattatgaaatccatgctttccgcagaatcgggttgaactcatctgcttgctacaaagctgttgagatatcaacattaattaggagatgccttgagccaggggaggacggcttgttcttgggtgagggatcgggttctatgttgatcacttataaagagatacttaaactaaacaagtgcttctataatagtggggtttccgccaattctagatctggtcaaagggaattagcaccctatccctccgaagttggccttgtcgaacacagaatgggagtaggtaatattgtcaaagtgctctttaacgggaggcccgaagtcacgtgggtaggcagtgtagattgcttcaatttcatagttagtaatatccctacctctagtgtggggtttatccattcagatatagagaccttgcctgacaaagatactatagagaagctagaggaattggcagccatcttatcgatggctctgctcctgggcaaaataggatcaatactggtgattaagcttatgcctttcagcggggattttgttcagggatttataagttatgtagggtctcattatagagaagtgaaccttgtataccctagatacagcaacttcatctctactgaatcttatttggttatgacagatctcaaggctaaccggctaatgaatcctgaaaagattaagcagcagataattgaatcatctgtgaggacttcacctggacttataggtcacatcctatccattaagcaactaagctgcatacaagcaattgtgggagacgcagttagtagaggtgatatcaatcctactctgaaaaaacttacacctatagagcaggtgctgatcaattgcgggttggcaattaacggacctaagctgtgcaaagaattgatccaccatgatgttgcctcagggcaagatggattgcttaattctatactcatcctctacagggagttggcaagattcaaagacaaccaaagaagtcaacaagggatgttccacgcttaccccgtattggtaagtagcaggcaacgagaacttatatctaggatcacccgcaaattctgggggcacattcttctttactccgggaacaaaaagttgataaataagtttatccagaatctcaagtccggctatctgatactagacttacaccagaatatcttcgttaagaatctatccaagtcagagaaacagattattatgacggggggtttgaaacgtgagtgggtttttaaggtaacagtcaaggagaccaaagaatggtataagttagtcggatacagtgccctgattaaggactaattggttgaactccggaaccctaatcctgccctaggtggttaggcattatttgcaatatattaaagaaaactttgaaaatacgaagtttctattcccagctttgtctggtggccggcatggtcccagcctcctcgctggcgccggctgggcaacattccgaggggaccgtcccctcggtaatggcgaatgggacgcggccgatccggctgctaacaaagcccgaaaggaagctgagttggctgctgccaccgctgagcaataactagcataaccccttggggcctctaaacgggtcttgaggggttttttgctgaaaggaggaactatatccggatgcggccgcgggccctatggtacccagcttttgttccctttagtgagggttaattccgagcttggcgtaatcatggtcatagctgtttcctgtgtgaaattgttatccgctcacaattccacacaacataggagccggaagcataaagtgtaaagcctggggtgcctaatgagtgaggtaactcacattaattgcgttgcgctcactgcccgctttccagtcgggaaacctgtcgtgccagctgcattaatgaatcggccaacgcgcggggagaggcggtttgcgtattgggcgctcttccgcttcctcgctcactgactcgctgcgctcggtcgttcggctgcggcgagcggtatcagctcactcaaaggcggtaatacggttatccacagaatcaggggataacgcaggaaagaacatgtgagcaaaaggccagcaaaaggccaggaaccgtaaaaaggccgcgttgctggcgtttttccataggctcggcccccctgacgagcatcacaaaaatcgacgctcaagtcagaggtggcgaaacccgacaggactataaagataccaggcgttcccccctggaagctccctcgtgcgctctcctgttccgaccctgccgcttaccggatacctgtccgcctttctcccttcgggaagcgtggcgctttctcaatgctcacgctgtaggtatctcagttcggtgtaggtcgttcgctccaagctgggctgtgtgcacgaaccccccgttcagcccgaccgctgcgccttatccggtaactatcgtcttgagtccaacccggtaagacacgacttatcgccactggcagcagccactggtaacaggattagcagagcgaggtatgtaggcggtgctacagagttcttgaagtggtggcctaactacggctacactagaaggacagtatttggtatctgcgctctgctgaagccagttaccttcggaaaaagagttggtagctcttgatccggcaaacaaaccaccgctggtagcggtggtttttttgtttgcaagcagcagattacgcgcagaaaaaaaggatctcaagaagatcctttgatcttttctacggggtctgacgctcagtggaacgaaaactcacgttaagggattttggtcatgagattatcaaaaaggatcttcacctagatccttttaaattaaaaatgaagttttaaatcaatctaaagtatatatgagtaaacttggtctgacagttaccaatgcttaatcagtgaggcacctatctcagcgatctgtctatttcgttcatccatagttgcctgactgcccgtcgtgtagataactacgatacgggagggcttaccatctggccccagtgctgcaatgataccgcgagacccacgctcaccggctccagatttatcagcaataaaccagccagccggaagggccgagcgcagaagtggtcctgcaactttatccgcctccatccagtctattaattgttgccgggaagctagagtaagtagttcgccagttaatagtttgcgcaacgttgttgccattgctacaggcatcgtggtgtcacgctcgtcgtttggtatggcttcattcagctccggttcccaacgatcaaggcgagttacatgatcccccatgttgtgaaaaaaagcggttagctccttcggtcctccgatcgttgtcagaagtaagttggccgcagtgttatcactcatgcttatggcagcactgcataattctcttactgtcatgccatccgtaagatgcttttctgtgactggtgagtactcaaccaagtcattctgagaatagtgtatgcggcgaccgagttgctcttgcccggcgtcaatacgggataataccgcgccacatagcagaactttaaaagtgctcatcattggaaaacgttcttcggggcgaaaactctcaaggatcttaccgctgttgagatccagttcgatgtaacccactcgtgcacccaactgatcttcagcatcttttactttcaccagcgtttctgggtgagcaaaaacaggaaggcaaaatgccgcaaaaaagggaataagggcgacacggaaatgttgaatactcatactcttcctttttcaatattattgaagcatttatcagggttattgtctcatgagcggatacatatttgaatgtatttagaaaaataaacaaataggggttccgcgcacatttccccgaaaagtgccacctgaaattgtaaacgttaatattttgttaaaattcgcgttaaatttttgttaaatcagctcattttttaaccaataggccgaaatcggcaaaatcccttataaatcaaaagaatagaccgagatagggttgagtgttgttccagtttggaacaagagtccactattaaagaacgtggactccaacgtcaaagggcgaaaaaccgtctatcagggcgatggcccactacgtgaaccatcaccctaatcaagttttttggggtcgaggtgccgtaaagcactaaatcggaaccctaaagggagcccccgatttagagcttgacggggaaagccggcgaacgtggcgagaaaggaagggaagaaagcgaaaggagcgggcgctagggcgctggcaagtgtagcggtcacgctgcgcgtaaccaccacacccgccgcgcttaatgcgccgctacagggcgcgtcccattcgccattcaggctgcgcaactgttgggaagggcgatcggtgcgggcctcttcgctattacgccagccaccgcggtg

SEQ ID NO: 141 - DNA, 20701 bp, Artificial Sequence
  Complete optimised nucleotide sequence of the polynucleotide encoding pTM-MVDVax8
  misc_feature (1)..(8): NotI
  misc_feature (9)..(28): T7 promoter
  misc_feature (29)..(82): Hammerhead ribozyme
  misc_feature (83)..(189): MV Leader and N promoter
  misc_feature (190)..(1767): MV N ORF
  misc_feature (1768)..(1888): MV N-P intergenic
  misc_feature (1889)..(3412): MV P ORF
  misc_feature (3413)..(3519): MV P-M intergenic
  misc_feature (3520)..(4527): MV M ORF
  misc_feature (4528)..(5530): MV M-F intergenic
  misc_feature (5531)..(7192): MV F ORF
  misc_feature (7193)..(7352): MV-F-H intergenic
  misc_feature (7353)..(9206): MV H ORF
  misc_feature (9207)..(9333): MV ATU3
  misc_feature (9334)..(10956): DENV1 NS polyepitope
  misc_feature (10957)..(11049): MV H-L intergenic
  misc_feature (11050)..(17601): MV L ORF
  misc_feature (17602)..(17710): MV Trailer
  misc_feature (17711)..(17794): HDV ribozyme
  misc_feature (17795)..(17936): T7 terminator
  misc_feature (17937)..(17944): Not I
  misc_feature (17945)..(20701): pTM plasmid
gcggccgctaatacgactcactatagggccaactttgtttggtctgatgagtccgtgaggacgaaacccggagtcccgggtcaccaaacaaagttgggtaaggatagttcaatcaatgatcatcttctagtgcacttaggattcaagatcctattatcagggacaagagcaggattagggatatccgagatggccacacttttaaggagcttagcattgttcaaaagaaacaaggacaaaccacccattacatcaggatccggtggagccatcagaggaatcaaacacattattatagtaccaatccctggagattcctcaattaccactcgatccagacttctggaccggttggtgaggttaattggaaacccggatgtgagcgggcccaaactaacaggggcactaataggtatattatccttatttgtggagtctccaggtcaattgattcagaggatcaccgatgaccctgacgttagcataaggctgttagaggttgtccagagtgaccagtcacaatctggccttaccttcgcatcaagaggtaccaacatggaggatgaggcggaccaatacttttcacatgatgatccaattagtagtgatcaatccaggttcggatggttcgggaacaaggaaatctcagatattgaagtgcaagaccctgagggattcaacatgattctgggtaccatcctagcccaaatttgggtcttgctcgcaaaggcggttacggccccagacacggcagctgattcggagctaagaaggtggataaagtacacccaacaaagaagggtagttggtgaatttagattggagagaaaatggttggatgtggtgaggaacaggattgccgaggacctctccttacgccgattcatggtcgctctaatcctggatatcaagagaacacccggaaacaaacccaggattgctgaaatgatatgtgacattgatacatatatcgtagaggcaggattagccagttttatcctgactattaagtttgggatagaaactatgtatcctgctcttggactgcatgaatttgctggtgagttatccacacttgagtccttgatgaacctttaccagcaaatgggggaaactgcaccctacatggtaatcctggagaactcaattcagaacaagttcagtgcaggatcataccctctgctctggagctatgccatgggagtaggagtggaacttgaaaactccatgggaggtttgaactttggccgatcttactttgatccagcatattttagattagggcaagagatggtaaggaggtcagctggaaaggtcagttccacattggcatctgaactcggtatcactgccgaggatgcaaggcttgtttcagagattgcaatgcatactactgaggacaagatcagtagagcggttggacccagacaagcccaagtatcatttctacacggtgatcaaagtgagaatgagctaccgagattggggggcaaggaagataggagggtcaaacagagtcgaggagaagccagggagagctacagagaaaccgggcccagcagagcaagtgatgcgagagctgcccatcttccaaccggcacacccctagacattgacactgcaacggagtccagccaagatccgcaggacagtcgaaggtcagctgacgccctgcttaggctgcaagccatggcaggaatctcggaagaacaaggctcagacacggacacccctatagtgtacaatgacagaaatcttctagactaggtgcgagaggccgagggccagaacaacatccgcctaccatccatcattgttataaaaaacttaggaaccaggtccacacagccgccagcccatcaaccatccactcccacgattggagccaatggcagaagagcaggcacgccatgtcaaaaacggactggaatgcatccgggctctcaaggccgagcccatcggctcactggccatcgaggaagctatggcagcatggtcagaaatatcagacaacccaggacaggagcgagccacctgcagggaagagaaggcaggcagttcgggtctcagcaaaccatgcctctcagcaattggatcaactgaaggcggtgcacctcgcatccgcggtcagggacctggagagagcgatgacgacgctgaaactttgggaatccccccaagaaatctccaggcatcaagcactgggttacagtgttattacgtttatgatcacagcggtgaagcggttaagggaatccaagatgctgactctatcatggttcaatcaggccttgatggtgatagcaccctctcaggaggagacaatgaatctgaaaacagcgatgtggatattggcgaacctgataccgagggatatgctatcactgaccggggatctgctcccatctctatggggttcagggcttctgatgttgaaactgcagaaggaggggagatccacgagctcctgagactccaatccagaggcaacaactttccgaagcttgggaaaactctcaatgttcctccgcccccggaccccggtagggccagcacttccgggacacccattaaaaagggcacagacgcgagattagcctcatttggaacggagatcgcgtctttattgacaggtggtgcaacccaatgtgctcgaaagtcaccctcggaaccatcagggccaggtgcacctgcggggaatgtccccgagtgtgtgagcaatgccgcactgatacaggagtggacacccgaatctggtaccacaatctccccgagatcccagaataatgaagaagggggagactattatgatgatgagctgttctctgatgtccaagatattaaaacagccttggccaaaatacacgaggataatcagaagataatctccaagctagaatcactgctgttattgaagggagaagttgagtcaattaagaagcagatcaacaggcaaaatatcagcatatccaccctggaaggacacctctcaagcatcatgatcgccattcctggacttgggaaggatcccaacgaccccactgcagatgtcgaaatcaatcccgacttgaaacccatcataggcagagattcaggccgagcactggccgaagttctcaagaaacccgttgccagccgacaactccaaggaatgacaaatggacggaccagttccagaggacagctgctgaaggaatttcagctaaagccgatcgggaaaaagatgagctcagccgtcgggtttgttcctgacaccggccctgcatcacgcagtgtaatccgctccattataaaatccagccggctagaggaggatcggaagcgttacctgatgactctccttgatgatatcaaaggagccaatgatcttgccaagttccaccagatgctgatgaagataataatgaagtagctacagctcaacttacctgccaaccccatgccagtcgacccaactagtacaacctaaatccattataaaaaacttaggagcaaagtgattgcctcccaaggtccacaatgacagagacctacgacttcgacaagtcggcatgggacatcaaagggtcgatcgctccgatacaacccaccacctacagtgatggcaggctggtgccccaggtcagagtcatagatcctggtctaggcgacaggaaggatgaatgctttatgtacatgtttctgctgggggttgttgaggacagcgattccctagggcctccaatcgggcgagcatttgggttcctgcccttaggtgttggcagatccacagcaaagcccgaaaaactcctcaaagaggccactgagcttgacatagttgttagacgtacagcagggctcaatgaaaaactggtgttctacaacaacaccccactaactctcctcacaccttggagaaaggtcctaacaacagggagtgtcttcaacgcaaaccaagtgtgcaatgcggttaatctgataccgctcgataccccgcagaggttccgtgttgtttatatgagcatcacccgtctttcggataacgggtattacaccgttcctagaagaatgctggaattcagatcggtcaatgcagtggccttcaacctgctggtgacccttaggattgacaaggcgataggccctgggaagatcatcgacaatacagagcaacttcctgaggcaacatttatggtccacatcgggaacttcaggagaaagaagagtgaagtctactctgccgattattgcaaaatgaaaatcgaaaagatgggcctggtttttgcacttggtgggatagggggcaccagtcttcacattagaagcacaggcaaaatgagcaagactctccatgcacaactcgggttcaagaagaccttatgttacccgctgatggatatcaatgaagaccttaatcgattactctggaggagcagatgcaagatagtaagaatccaggcagttttgcagccatcagttcctcaagaattccgcatttacgacgacgtgatcataaatgatgaccaaggactattcaaagttctgtagaccgtagtgcccagcaatgcccgaaaacgacccccctcacaatgacagccagaaggcccggacaaaaaagccccctccgaaagactccacggaccaagcgagaggccagccagcagccgacggcaagcgcgaacaccaggcggccccagcacagaacagccctgacacaaggccaccaccagccaccccaatctgcatcctcctcgtgggacccccgaggaccaacccccaaggctgcccccgatccaaaccaccaaccgcatccccaccacccccgggaaagaaacccccagcaattggaaggcccctccccctcttcctcaacacaagaactccacaaccgaaccgcacaagcgaccgaggtgacccaaccgcaggcatccgactccctagacagatcctctctccccggcaaactaaacaaaacttagggccaaggaacatacacacccaacagaacccagaccccggcccacggcgccgcgcccccaacccccgacaaccagagggagcccccaaccaatcccgccggctcccccggtgcccacaggcagggacaccaacccccgaacagacccagcacccaaccatcgacaatccaagacgggggggcccccccaaaaaaaggcccccaggggccgacagccagcaccgcgaggaagcccacccaccccacacacgaccacggcaaccaaaccagaacccagaccaccctgggccaccagctcccagactcggccatcaccccgcagaaaggaaaggccacaacccgcgcaccccagccccgatccggcggggagccacccaacccgaaccagcacccaagagcgatccccgaaggacccccgaaccgcaaaggacatcagtatcccacagcctctccaagtcccccggtctcctcctcttctcgaagggaccaaaagatcaatccaccacacccgacgacactcaactccccacccctaaaggagacaccgggaatcccagaatcaagactcatccaatgtccatcatgggtctcaaggtgaacgtctctgccatattcatggcagtactgttaactctccaaacacccaccggtcaaatccattggggcaatctctctaagataggggtggtaggaataggaagtgcaagctacaaagttatgactcgttccagccatcaatcattagtcataaaattaatgcccaatataactctcctcaataactgcacgagggtagagattgcagaatacaggagactactgagaacagttttggaaccaattagagatgcacttaatgcaatgacccagaatataagaccggttcagagtgtagcttcaagtaggagacacaagagatttgcgggagtagtcctggcaggtgcggccctaggcgttgccacagctgctcagataacagccggcattgcacttcaccagtccatgctgaactctcaagccatcgacaatctgagagcgagcctggaaactactaatcaggcaattgagacaatcagacaagcagggcaggagatgatattggctgttcagggtgtccaagactacatcaataatgagctgataccgtctatgaaccaactatcttgtgatttaatcggccagaagctcgggctcaaattgctcagatactatacagaaatcctgtcattatttggccccagtttacgggaccccatatctgcggagatatctatccaggctttgagctatgcgcttggaggagacatcaataaggtgttagaaaagctcggatacagtggaggtgatttactgggcatcttagagagcggaggaataaaggcccggataactcacgtcgacacagagtcctacttcattgtcctcagtatagcctatccgacgctgtccgagattaagggggtgattgtccaccggctagagggggtctcgtacaacataggctctcaagagtggtataccactgtgcccaagtatgttgcaacccaagggtaccttatctcgaattttgatgagtcatcgtgtactttcatgccagaggggactgtgtgcagccaaaatgccttgtacccgatgagtcctctgctccaagaatgcctccgggggtacaccaagtcctgtgctcgtacactcgtatccgggtcttttgggaaccggttcattttatcacaagggaacctaatagccaattgtgcatcaatcctttgcaagtgttacacaacaggaacgatcattaatcaagaccctgacaagatcctaacatacattgctgccgatcactgcccggtagtcgaggtgaacggcgtgaccatccaagtcgggagcaggaggtatccagacgctgtgtacttgcacagaattgacctcggtcctcccatatcattggagaggttggacgtagggacaaatctggggaatgcaattgctaagttggaggatgccaaggaattgttggagtcatcggaccagatattgaggagtatgaaaggtttatcgagcactagcatagtctacatcctgattgcagtgtgtcttggagggttgatagggatccccgctttaatatgttgctgcagggggcgttgtaacaaaaagggagaacaagttggtatgtcaagaccaggcctaaagcctgatcttacgggaacatcaaaatcctatgtaaggtcgctctgatcctctacaactcttgaaacacaaatgtcccacaagtctcctcttcgtcatcaagcaaccaccgcacccagcatcaagcccacctgaaattatctccggcttccctctggccgaacaatatcggtagttaatcaaaacttagggtgcaagatcatccacaatgtcaccacaacgagaccggataaatgccttctacaaagataacccccatcccaagggaagtaggatagtcattaacagagaacatcttatgattgatagaccttatgttttgctggctgttctgtttgtcatgtttctgagcttgatcgggttgctagccattgcaggcattagacttcatcgggcagccatctacaccgcagagatccataaaagcctcagcaccaatctagatgtaactaactcaatcgagcatcaggtcaaggacgtgctgacaccactcttcaaaatcatcggtgatgaagtgggcctgaggacacctcagagattcactgacctagtgaaattaatctctgacaagattaaattccttaatccggatagggagtacgacttcagagatctcacttggtgtatcaacccgccagagagaatcaaattggattatgatcaatactgtgcagatgtggctgctgaagagctcatgaatgcattggtgaactcaactctactggagaccagaacaaccaatcagttcctagctgtctcaaagggaaactgctcagggcccactacaatcagaggtcaattctcaaacatgtcgctgtccctgttagacttgtatttaggtcgaggttacaatgtgtcatctatagtcactatgacatcccagggaatgtatgggggaacttacctagtggaaaagcctaatctgagcagcaaaaggtcagagttgtcacaactgagcatgtaccgagtgtttgaagtaggtgttatcagaaatccgggtttgggggctccggtgttccatatgacaaactatcttgagcaaccagtcagtaatgatctcagcaactgtatggtggctttgggggagctcaaactcgcagccctttgtcacggggaagattctatcacaattccctatcagggatcagggaaaggtgtcagcttccagctcgtcaagctaggtgtctggaaatccccaaccgacatgcaatcctgggtccccttatcaacggatgatccagtgatagacaggctttacctctcatctcacagaggtgttatcgctgacaatcaagcaaaatgggctgtcccgacaacacgaacagatgacaagttgcgaatggagacatgcttccaacaggcgtgtaagggtaaaatccaagcactctgcgagaatcccgagtgggcaccattgaaggataacaggattccttcatacggggtcttgtctgttgatctgagtctgacagttgagcttaaaatcaaaattgcttcgggattcgggccattgatcacacacggttcagggatggacctatacaaatccaaccacaacaatgtgtattggctgactatcccgccaatgaagaacctagccttaggtgtaatcaacacattggagtggataccgagattcaaggttagtccctacctcttcactgtcccaattaaggaagcaggcgaagactgccatgccccaacatacctacctgcggaggtggatggtgatgtcaaactcagttccaatctggtgattctacctggtcaagatctccaatatgttttggcaacctacgatacttccagggttgaacatgctgtggtttattacgtttacagcccaagccgctcattttcttacttttatccttttaggttgcctataaagggggtccccatcgaattacaagtggaatgcttcacatgggaccaaaaactctggtgccgtcacttctgtgtgcttgcggactcagaatctggtggacatatcactcactctgggatggtgggcatgggagtcagctgcacagtcacccgggaagatggaaccaatcgcagatagggctgctagtgaaccaatcacatgatgtcacccagacatcaggcatacccactagtctaccctccatcattgttataaaaaacttaggaaccaggtccacacagccgccagcccatcaacgcgtacgatggcatcacaggagggaccactgcccgaaattgaggacgaagtgtttagaaagcgaaatctgactattatggacctgcaccccggatctggcaagacccggagatacctgccagccatcgtgagggaggctattaagcggaaactgagaacactgatcctggccccaactcgcgtggtcgcttccgaaatggctgaggccctgaaaggcatgcccatccggtatcagaccacagcagtgaagtctgaacataccggcaaggagattgtggacctgatgtgccacgccactttcaccatgcgactgctgagcccagtgcgggtccccaactacaatatgatcattatggacgaggcccactttactgatcccagctccatcgccgctagaggatatatttccaccagggtgggaatgggcgaggcagcagctatcttcatgacagcaactccccctggcagcgtggaggcatttcctcagtccaacgccgtcatccaggacgaggagcgggacattcctgagcggagctggaattctgggtacgaatggatcacagacgaggatcatgcacactggactgaagccaagatgctgctggacaacattaatactcctgagggaatcattccagctctgttcgagcccgaaagagagaagtctgcagccatcgacggcgagtatagactgaggggagaggcccggaagaccttcgtggaactgatgaggcgcggcgatctgcccgtgtggctgagttacaaggtcgcttcagagggattccagtatagtgaccgacggtggtgctttgatggcgaacgcaacaatcaggtgctggaggagaacatggatgtcgagatttggacaaaggaaggcgagcggaagaaactgcgcccacgatggctggacgctcggacttacagcgatcccctggcactgagagaattcaaagagtttgctgcaggggtggccgtcgagaatcaccatcacgccgctatgctggacgtggatctgcatcctgccagtgcttggaccctgtatgcagtggccactaccatcattaccccaatgatgcgccacacaatcgagaacacaactgccaatatctcactgacagctattgcaaaccaggcagccattctgatgggactggacaaaggctggcccatcagcaagatggatattggcgtgcctctgctggccctggggtgttacagtcaggtgctggacatcattggccagaggatcgagaacattaagcatgagcacaaatcaacctggcattacgacgaagataatccctataagacatgggcctaccacggaagctatgaggtgaaaccttcaggcagcgccagcagcatggtcaacggggtggtcaagctgctgaccaaaccttgggacgtgatcccaatggtcactcagattgccatgaccgataccaccccattcggccagcagcgggtgttcaaggagaaggtggacacccgcacacctaaggctaaacgagggactgcacagatcatggaggtgaccgccaagtggctgtggggattcctgtccaggaacaagaagccaagaatctgtaccagggaagagttcacaagaaaggtccggtcaaacgcctaatgagcgcgcagcgcttagacgtctcgcgatcgatgctagtgtgaaatagacatcagaattaagaaaaacgtagggtccaagtggttccccgttatggactcgctatctgtcaaccagatcttataccctgaagttcacctagatagcccgatagttaccaataagatagtagccatcctggagtatgctcgagtccctcacgcttacagcctggaggaccctacactgtgtcagaacatcaagcaccgcctaaaaaacggattttccaaccaaatgattataaacaatgtggaagttgggaatgtcatcaagtccaagcttaggagttatccggcccactctcatattccatatccaaattgtaatcaggatttatttaacatagaagacaaagagtcaacgaggaagatccgtgaactcctcaaaaaggggaattcgctgtactccaaagtcagtgataaggttttccaatgcttaagggacactaactcacggcttggcctaggctccgaattgagggaggacatcaaggagaaagttattaacttgggagtttacatgcacagctcccagtggtttgagccctttctgttttggtttacagtcaagactgagatgaggtcagtgattaaatcacaaacccatacttgccataggaggagacacacacctgtattcttcactggtagttcagttgagttgctaatctctcgtgaccttgttgctataatcagtaaagagtctcaacatgtatattacctgacatttgaactggttttgatgtattgtgatgtcatagaggggaggttaatgacagagaccgctatgactattgatgctaggtatacagagcttctaggaagagtcagatacatgtggaaactgatagatggtttcttccctgcactcgggaatccaacttatcaaattgtagccatgctggagcctctttcacttgcttacctgcagctgagggatataacagtagaactcagaggtgctttccttaaccactgctttactgaaatacatgatgttcttgaccaaaacgggttttctgatgaaggtacttatcatgagttaactgaagctctagattacattttcataactgatgacatacatctgacaggggagattttctcatttttcagaagtttcggccaccccagacttgaagcagtaacggctgctgaaaatgttaggaaatacatgaatcagcctaaagtcattgtgtatgagactctgatgaaaggtcatgccatattttgtggaatcataatcaacggctatcgtgacaggcacggaggcagttggccaccgctgaccctccccctgcatgctgcagacacaatccggaatgctcaagcttcaggtgaagggttaacacatgagcagtgcgttgataactggaaatcttttgctggagtgaaatttggctgctttatgcctcttagcctggatagtgatctgacaatgtacctaaaggacaaggcacttgctgctctccaaagggaatgggattcagtttacccgaaagagttcctgcgttacgaccctcccaagggaaccgggtcacggaggcttgtagatgttttccttaatgattcgagctttgacccatatgatgtgataatgtatgttgtaagtggagcttacctccatgaccctgagttcaacctgtcttacagcctgaaagaaaaggagatcaaggaaacaggtagactttttgctaaaatgacttacaaaatgagggcatgccaagtgattgctgaaaatctaatctcaaacgggattggcaaatattttaaggacaatgggatggccaaggatgagcacgatttgactaaggcactccacactctagctgtctcaggagtccccaaagatctcaaagaaagtcacaggggggggccagtcttaaaaacctactcccgaagcccagtccacacaagtaccaggaacgtgagagcagcaaaagggtttatagggttccctcaagtaattcggcaggaccaagacactgatcatccggagaatatggaagcttacgagacagtcagtgcatttatcacgactgatctcaagaagtactgccttaattggagatatgagaccatcagcttgtttgcacagaggctaaatgagatttacggattgccctcatttttccagtggctgcataagaggcttgagacctctgtcctgtatgtaagtgaccctcattgcccccccgaccttgacgcccatatcccgttatataaagtccccaatgatcaaatcttcattaagtaccctatgggaggtatagaagggtattgtcagaagctgtggaccatcagcaccattccctatctatacctggctgcttatgagagcggagtaaggattgcttcgttagtgcaaggggacaatcagaccatagccgtaacaaaaagggtacccagcacatggccctacaaccttaagaaacgggaagctgctagagtaactagagattactttgtaattcttaggcaaaggctacatgatattggccatcacctcaaggcaaatgagacaattgtttcatcacatttttttgtctattcaaaaggaatatattatgatgggctacttgtgtcccaatcactcaagagcatcgcaagatgtgtattctggtcagagactatagttgatgaaacaagggcagcatgcagtaatattgctacaacaatggctaaaagcatcgagagaggttatgaccgttaccttgcatattccctgaacgtcctaaaagtgatacagcaaattctgatctctcttggcttcacaatcaattcaaccatgacccgggatgtagtcatacccctcctcacaaacaacgacctcttaataaggatggcactgttgcccgctcctattggggggatgaattatctgaatatgagcaggctgtttgtcagaaacatcggtgatccagtaacatcatcaattgctgatctcaagagaatgattctcgcctcactaatgcctgaagagaccctccatcaagtaatgacacaacaaccgggggactcttcattcctagactgggctagcgacccttactcagcaaatcttgtatgtgtccagagcatcactagactcctcaagaacataactgcaaggtttgtcctgatccatagtccaaacccaatgttaaaaggattattccatgatgacagtaaagaagaggacgagggactggcggcattcctcatggacaggcatattatagtacctagggcagctcatgaaatcctggatcatagtgtcacaggggcaagagagtctattgcaggcatgctggataccacaaaaggcttgattcgagccagcatgaggaagggggggttaacctctcgagtgataaccagattgtccaattatgactatgaacaattcagagcagggatggtgctattgacaggaagaaagagaaatgtcctcattgacaaagagtcatgttcagtgcagctggcgagagctctaagaagccatatgtgggcgaggctagctcgaggacggcctatttacggccttgaggtccctgatgtactagaatctatgcgaggccaccttattcggcgtcatgagacatgtgtcatctgcgagtgtggatcagtcaactacggatggttttttgtcccctcgggttgccaactggatgatattgacaaggaaacatcatccttgagagtcccatatattggttctaccactgatgagagaacagacatgaagcttgccttcgtaagagccccaagtcgatccttgcgatctgctgttagaatagcaacagtgtactcatgggcttacggtgatgatgatagctcttggaacgaagcctggttgttggctaggcaaagggccaatgtgagcctggaggagctaagggtgatcactcccatctcaacttcgactaatttagcgcataggttgagggatcgtagcactcaagtgaaatactcaggtacatcccttgtccgagtggcgaggtataccacaatctccaacgacaatctctcatttgtcatatcagataagaaggttgatactaactttatataccaacaaggaatgcttctagggttgggtgttttagaaacattgtttcgactcgagaaagataccggatcatctaacacggtattacatcttcacgtcgaaacagattgttgcgtgatcccgatgatagatcatcccaggatacccagctcccgcaagctagagctgagggcagagctatgtaccaacccattgatatatgataatgcacctttaattgacagagatgcaacaaggctatacacccagagccataggaggcaccttgtggaatttgttacatggtccacaccccaactatatcacattttagctaagtccacagcactatctatgattgacctggtaacaaaatttgagaaggaccatatgaatgaaatttcagctctcataggggatgacgatatcaatagtttcataactgagtttctgctcatagagccaagattattcactatctacttgggccagtgtgcggccatcaattgggcatttgatgtacattatcatagaccatcagggaaatatcagatgggtgagctgttgtcatcgttcctttctagaatgagcaaaggagtgtttaaggtgcttgtcaatgctctaagccacccaaagatctacaagaaattctggcattgtggtattatagagcctatccatggtccttcacttgatgctcaaaacttgcacacaactgtgtgcaacatggtttacacatgctatatgacctacctcgacctgttgttgaatgaagagttagaagagttcacatttctcttgtgtgaaagcgacgaggatgtagtaccggacagattcgacaacatccaggcaaaacacttatgtgttctggcagatttgtactgtcaaccagggacctgcccaccaattcgaggtctaagaccggtagagaaatgtgcagttctaaccgaccatatcaaggcagaggctatgttatctccagcaggatcttcgtggaacataaatccaattattgtagaccattactcatgctctctgacttatctccggcgaggatcgatcaaacagataagattgagagttgatccaggattcattttcgacgccctcgctgaggtaaatgtcagtcagccaaagatcggcagcaacaacatctcaaatatgagcatcaaggctttcagacccccacacgatgatgttgcaaaattgctcaaagatatcaacacaagcaagcacaatcttcccatttcagggggcaatctcgccaattatgaaatccatgctttccgcagaatcgggttgaactcatctgcttgctacaaagctgttgagatatcaacattaattaggagatgccttgagccaggggaggacggcttgttcttgggtgagggatcgggttctatgttgatcacttataaagagatacttaaactaaacaagtgcttctataatagtggggtttccgccaattctagatctggtcaaagggaattagcaccctatccctccgaagttggccttgtcgaacacagaatgggagtaggtaatattgtcaaagtgctctttaacgggaggcccgaagtcacgtgggtaggcagtgtagattgcttcaatttcatagttagtaatatccctacctctagtgtggggtttatccattcagatatagagaccttgcctgacaaagatactatagagaagctagaggaattggcagccatcttatcgatggctctgctcctgggcaaaataggatcaatactggtgattaagcttatgcctttcagcggggattttgttcagggatttataagttatgtagggtctcattatagagaagtgaaccttgtataccctagatacagcaacttcatctctactgaatcttatttggttatgacagatctcaaggctaaccggctaatgaatcctgaaaagattaagcagcagataattgaatcatctgtgaggacttcacctggacttataggtcacatcctatccattaagcaactaagctgcatacaagcaattgtgggagacgcagttagtagaggtgatatcaatcctactctgaaaaaacttacacctatagagcaggtgctgatcaattgcgggttggcaattaacggacctaagctgtgcaaagaattgatccaccatgatgttgcctcagggcaagatggattgcttaattctatactcatcctctacagggagttggcaagattcaaagacaaccaaagaagtcaacaagggatgttccacgcttaccccgtattggtaagtagcaggcaacgagaacttatatctaggatcacccgcaaattctgggggcacattcttctttactccgggaacaaaaagttgataaataagtttatccagaatctcaagtccggctatctgatactagacttacaccagaatatcttcgttaagaatctatccaagtcagagaaacagattattatgacggggggtttgaaacgtgagtgggtttttaaggtaacagtcaaggagaccaaagaatggtataagttagtcggatacagtgccctgattaaggactaattggttgaactccggaaccctaatcctgccctaggtggttaggcattatttgcaatatattaaagaaaactttgaaaatacgaagtttctattcccagctttgtctggtggccggcatggtcccagcctcctcgctggcgccggctgggcaacattccgaggggaccgtcccctcggtaatggcgaatgggacgcggccgatccggctgctaacaaagcccgaaaggaagctgagttggctgctgccaccgctgagcaataactagcataaccccttggggcctctaaacgggtcttgaggggttttttgctgaaaggaggaactatatccggatgcggccgcgggccctatggtacccagcttttgttccctttagtgagggttaattccgagcttggcgtaatcatggtcatagctgtttcctgtgtgaaattgttatccgctcacaattccacacaacataggagccggaagcataaagtgtaaagcctggggtgcctaatgagtgaggtaactcacattaattgcgttgcgctcactgcccgctttccagtcgggaaacctgtcgtgccagctgcattaatgaatcggccaacgcgcggggagaggcggtttgcgtattgggcgctcttccgcttcctcgctcactgactcgctgcgctcggtcgttcggctgcggcgagcggtatcagctcactcaaaggcggtaatacggttatccacagaatcaggggataacgcaggaaagaacatgtgagcaaaaggccagcaaaaggccaggaaccgtaaaaaggccgcgttgctggcgtttttccataggctcggcccccctgacgagcatcacaaaaatcgacgctcaagtcagaggtggcgaaacccgacaggactataaagataccaggcgttcccccctggaagctccctcgtgcgctctcctgttccgaccctgccgcttaccggatacctgtccgcctttctcccttcgggaagcgtggcgctttctcaatgctcacgctgtaggtatctcagttcggtgtaggtcgttcgctccaagctgggctgtgtgcacgaaccccccgttcagcccgaccgctgcgccttatccggtaactatcgtcttgagtccaacccggtaagacacgacttatcgccactggcagcagccactggtaacaggattagcagagcgaggtatgtaggcggtgctacagagttcttgaagtggtggcctaactacggctacactagaaggacagtatttggtatctgcgctctgctgaagccagttaccttcggaaaaagagttggtagctcttgatccggcaaacaaaccaccgctggtagcggtggtttttttgtttgcaagcagcagattacgcgcagaaaaaaaggatctcaagaagatcctttgatcttttctacggggtctgacgctcagtggaacgaaaactcacgttaagggattttggtcatgagattatcaaaaaggatcttcacctagatccttttaaattaaaaatgaagttttaaatcaatctaaagtatatatgagtaaacttggtctgacagttaccaatgcttaatcagtgaggcacctatctcagcgatctgtctatttcgttcatccatagttgcctgactgcccgtcgtgtagataactacgatacgggagggcttaccatctggccccagtgctgcaatgataccgcgagacccacgctcaccggctccagatttatcagcaataaaccagccagccggaagggccgagcgcagaagtggtcctgcaactttatccgcctccatccagtctattaattgttgccgggaagctagagtaagtagttcgccagttaatagtttgcgcaacgttgttgccattgctacaggcatcgtggtgtcacgctcgtcgtttggtatggcttcattcagctccggttcccaacgatcaaggcgagttacatgatcccccatgttgtgaaaaaaagcggttagctccttcggtcctccgatcgttgtcagaagtaagttggccgcagtgttatcactcatgcttatggcagcactgcataattctcttactgtcatgccatccgtaagatgcttttctgtgactggtgagtactcaaccaagtcattctgagaatagtgtatgcggcgaccgagttgctcttgcccggcgtcaatacgggataataccgcgccacatagcagaactttaaaagtgctcatcattggaaaacgttcttcggggcgaaaactctcaaggatcttaccgctgttgagatccagttcgatgtaacccactcgtgcacccaactgatcttcagcatcttttactttcaccagcgtttctgggtgagcaaaaacaggaaggcaaaatgccgcaaaaaagggaataagggcgacacggaaatgttgaatactcatactcttcctttttcaatattattgaagcatttatcagggttattgtctcatgagcggatacatatttgaatgtatttagaaaaataaacaaataggggttccgcgcacatttccccgaaaagtgccacctgaaattgtaaacgttaatattttgttaaaattcgcgttaaatttttgttaaatcagctcattttttaaccaataggccgaaatcggcaaaatcccttataaatcaaaagaatagaccgagatagggttgagtgttgttccagtttggaacaagagtccactattaaagaacgtggactccaacgtcaaagggcgaaaaaccgtctatcagggcgatggcccactacgtgaaccatcaccctaatcaagttttttggggtcgaggtgccgtaaagcactaaatcggaaccctaaagggagcccccgatttagagcttgacggggaaagccggcgaacgtggcgagaaaggaagggaagaaagcgaaaggagcgggcgctagggcgctggcaagtgtagcggtcacgctgcgcgtaaccaccacacccgccgcgcttaatgcgccgctacagggcgcgtcccattcgccattcaggctgcgcaactgttgggaagggcgatcggtgcgggcctcttcgctattacgccagccaccgcggtg

SEQ ID NO: 142 - DNA, 22261 bp, Artificial Sequence
  Complete optimised nucleotide sequence of the polynucleotide encoding pTM-MVDVax9
  misc_feature (1 )..(8): NotI
  misc_feature (9)..(28): T7 promoter
  misc_feature (29)..(82): Hammerhead ribozyme
  misc_feature (83)..(189): MV Leader and N promoter
  misc_feature (190)..(1767): MV N ORF
  misc_feature (1768)..(1888): MV N-P intergenic
  misc_feature (1889)..(3412): MV P ORF
  misc_feature (3413)..(3531): MV ATU2
  misc_feature (3532)..(6717): DENV tetra EDIII/ectoM/DENV1 NS polyepitope
  misc_feature (6718)..(6813): MV P-M intergenic
  misc_feature (6814)..(7821): MV M ORF
  misc_feature (7822)..(8824): MV M-F intergenic
  misc_feature (8825)..(10486): MV F ORF
  misc_feature (10487)..(10646): MV-F-H intergenic
  misc_feature (10647)..(12500): MV H ORF
  misc_feature (12501)..(12609): MV H-L intergenic
  misc_feature (12610)..(19161): MV L ORF
  misc_feature (19162)..(19270): MV Trailer
  misc_feature (19271)..(19354): HDV ribozyme
  misc_feature (19355)..(19496): T7 terminator
  misc_feature (19497)..(19504): Not I
  misc_feature (19506)..(22261): pTM plasmid
gcggccgctaatacgactcactatagggccaactttgtttggtctgatgagtccgtgaggacgaaacccggagtcccgggtcaccaaacaaagttgggtaaggatagttcaatcaatgatcatcttctagtgcacttaggattcaagatcctattatcagggacaagagcaggattagggatatccgagatggccacacttttaaggagcttagcattgttcaaaagaaacaaggacaaaccacccattacatcaggatccggtggagccatcagaggaatcaaacacattattatagtaccaatccctggagattcctcaattaccactcgatccagacttctggaccggttggtgaggttaattggaaacccggatgtgagcgggcccaaactaacaggggcactaataggtatattatccttatttgtggagtctccaggtcaattgattcagaggatcaccgatgaccctgacgttagcataaggctgttagaggttgtccagagtgaccagtcacaatctggccttaccttcgcatcaagaggtaccaacatggaggatgaggcggaccaatacttttcacatgatgatccaattagtagtgatcaatccaggttcggatggttcgggaacaaggaaatctcagatattgaagtgcaagaccctgagggattcaacatgattctgggtaccatcctagcccaaatttgggtcttgctcgcaaaggcggttacggccccagacacggcagctgattcggagctaagaaggtggataaagtacacccaacaaagaagggtagttggtgaatttagattggagagaaaatggttggatgtggtgaggaacaggattgccgaggacctctccttacgccgattcatggtcgctctaatcctggatatcaagagaacacccggaaacaaacccaggattgctgaaatgatatgtgacattgatacatatatcgtagaggcaggattagccagttttatcctgactattaagtttgggatagaaactatgtatcctgctcttggactgcatgaatttgctggtgagttatccacacttgagtccttgatgaacctttaccagcaaatgggggaaactgcaccctacatggtaatcctggagaactcaattcagaacaagttcagtgcaggatcataccctctgctctggagctatgccatgggagtaggagtggaacttgaaaactccatgggaggtttgaactttggccgatcttactttgatccagcatattttagattagggcaagagatggtaaggaggtcagctggaaaggtcagttccacattggcatctgaactcggtatcactgccgaggatgcaaggcttgtttcagagattgcaatgcatactactgaggacaagatcagtagagcggttggacccagacaagcccaagtatcatttctacacggtgatcaaagtgagaatgagctaccgagattggggggcaaggaagataggagggtcaaacagagtcgaggagaagccagggagagctacagagaaaccgggcccagcagagcaagtgatgcgagagctgcccatcttccaaccggcacacccctagacattgacactgcaacggagtccagccaagatccgcaggacagtcgaaggtcagctgacgccctgcttaggctgcaagccatggcaggaatctcggaagaacaaggctcagacacggacacccctatagtgtacaatgacagaaatcttctagactaggtgcgagaggccgagggccagaacaacatccgcctaccatccatcattgttataaaaaacttaggaaccaggtccacacagccgccagcccatcaaccatccactcccacgattggagccaatggcagaagagcaggcacgccatgtcaaaaacggactggaatgcatccgggctctcaaggccgagcccatcggctcactggccatcgaggaagctatggcagcatggtcagaaatatcagacaacccaggacaggagcgagccacctgcagggaagagaaggcaggcagttcgggtctcagcaaaccatgcctctcagcaattggatcaactgaaggcggtgcacctcgcatccgcggtcagggacctggagagagcgatgacgacgctgaaactttgggaatccccccaagaaatctccaggcatcaagcactgggttacagtgttattacgtttatgatcacagcggtgaagcggttaagggaatccaagatgctgactctatcatggttcaatcaggccttgatggtgatagcaccctctcaggaggagacaatgaatctgaaaacagcgatgtggatattggcgaacctgataccgagggatatgctatcactgaccggggatctgctcccatctctatggggttcagggcttctgatgttgaaactgcagaaggaggggagatccacgagctcctgagactccaatccagaggcaacaactttccgaagcttgggaaaactctcaatgttcctccgcccccggaccccggtagggccagcacttccgggacacccattaaaaagggcacagacgcgagattagcctcatttggaacggagatcgcgtctttattgacaggtggtgcaacccaatgtgctcgaaagtcaccctcggaaccatcagggccaggtgcacctgcggggaatgtccccgagtgtgtgagcaatgccgcactgatacaggagtggacacccgaatctggtaccacaatctccccgagatcccagaataatgaagaagggggagactattatgatgatgagctgttctctgatgtccaagatattaaaacagccttggccaaaatacacgaggataatcagaagataatctccaagctagaatcactgctgttattgaagggagaagttgagtcaattaagaagcagatcaacaggcaaaatatcagcatatccaccctggaaggacacctctcaagcatcatgatcgccattcctggacttgggaaggatcccaacgaccccactgcagatgtcgaaatcaatcccgacttgaaacccatcataggcagagattcaggccgagcactggccgaagttctcaagaaacccgttgccagccgacaactccaaggaatgacaaatggacggaccagttccagaggacagctgctgaaggaatttcagctaaagccgatcgggaaaaagatgagctcagccgtcgggtttgttcctgacaccggccctgcatcacgcagtgtaatccgctccattataaaatccagccggctagaggaggatcggaagcgttacctgatgactctccttgatgatatcaaaggagccaatgatcttgccaagttccaccagatgctgatgaagataataatgaagtagctacagctcaacttacctgccaaccccatgccagtcgacccaactagcctaccctccatcattgttataaaaaacttaggaaccaggtccacacagccgccagcccatcaacgcgtacgatgggcatcatattcattcttcttatgctggttacaccgtctatggcggagaaacttcgaatcaaaggtatgagctatacgatgtgcagcggcaagttcaagatcgagaaggaaatggctgaaacccagcacggtacaactgtggtcaaagtcaaatatgagggggctggcgctccctgtaaagtacccattgagattagggacgtcaataaagagaaggtggtaggtcgcatcatctccagtacacctttggccgagaacacgaactccgtcacaaacatagagttggaacccccgttcggagactcatacattgtgatcggggtgggcaactctgcactcacactgcattggttcaagaagggaagcagtatcggccgcagggataagagagacaaactgaaattgaaaggtatgtcctatgccatgtgcacgaatactttcgttctcaagaaagaagtatctgagactcagcacggaaccatcctgatcaaagtcgagtacaaaggagaagacgtgccctgtaagatcccattcagtaccgaggatggacagggcaaggcccataacggcaggctgataaccgccaaccctgtggttacaaagaaggaagagccagtcaatatcgaagctgagccaccgttcggggagagcaacatagtaattggcataggggataatgctttgaagatcaactggtacaagaaaggaagctccattggccgaagagataagcgcgacaaactccagctgaaaggaatgagctactccatgtgtactgggaagttcaagattgtcaaggaaatcgccgaaactcagcatggcactattgtgatccgcgtgcagtatgaaggcgatggtagcccctgcaagataccatttgaaatcaccgatttggagaaacggcacgtcctgggtcggctcattaccgtgaacccaatcgtgaccgagaaggacagtccagttaatatcgaggccgagcctcctttcggcgacagttacatcattgtaggggtggaaccagggcaactgaagctgaactggttcaagaaaggcagcagtataggacggcgggataaacgggacaaactcacactgaaaggcatgtcatacgttatgtgcaccggctcattcaaactggagaaggaagttgcagagacacagcatgggaccgtgctcgtgcaggtcaaatacgagggcaccgacgctccttgcaagattccgttcagtacacaggacgagaaaggcgtgactcagaacggcagattgattacagcgaaccctatcgtgactgacaaggagaagccagttaacatcgagactgagccgcctttcggagaatcatacattatcgtgggagccggcgagaaggcactgaaactcagctggttcaagaagggcagctcaatcggtcggagagacaagcggtctgtcgccctcgcaccgcacgtgggcctgggtctggaaacgaggaccgagacgtggatgagttccgaaggcgcatggaagcaaatccagaaagtggagacgtgggccctcaggcatccgcggagagataaacgagcatcacaggagggaccactgcccgaaattgaggacgaagtgtttagaaagcgaaatctgactattatggacctgcaccccggatctggcaagacccggagatacctgccagccatcgtgagggaggctattaagcggaaactgagaacactgatcctggccccaactcgcgtggtcgcttccgaaatggctgaggccctgaaaggcatgcccatccggtatcagaccacagcagtgaagtctgaacataccggcaaggagattgtggacctgatgtgccacgccactttcaccatgcgactgctgagcccagtgcgggtccccaactacaatatgatcattatggacgaggcccactttactgatcccagctccatcgccgctagaggatatatttccaccagggtgggaatgggcgaggcagcagctatcttcatgacagcaactccccctggcagcgtggaggcatttcctcagtccaacgccgtcatccaggacgaggagcgggacattcctgagcggagctggaattctgggtacgaatggatcacagacgaggatcatgcacactggactgaagccaagatgctgctggacaacattaatactcctgagggaatcattccagctctgttcgagcccgaaagagagaagtctgcagccatcgacggcgagtatagactgaggggagaggcccggaagaccttcgtggaactgatgaggcgcggcgatctgcccgtgtggctgagttacaaggtcgcttcagagggattccagtatagtgaccgacggtggtgctttgatggcgaacgcaacaatcaggtgctggaggagaacatggatgtcgagatttggacaaaggaaggcgagcggaagaaactgcgcccacgatggctggacgctcggacttacagcgatcccctggcactgagagaattcaaagagtttgctgcaggggtggccgtcgagaatcaccatcacgccgctatgctggacgtggatctgcatcctgccagtgcttggaccctgtatgcagtggccactaccatcattaccccaatgatgcgccacacaatcgagaacacaactgccaatatctcactgacagctattgcaaaccaggcagccattctgatgggactggacaaaggctggcccatcagcaagatggatattggcgtgcctctgctggccctggggtgttacagtcaggtgctggacatcattggccagaggatcgagaacattaagcatgagcacaaatcaacctggcattacgacgaagataatccctataagacatgggcctaccacggaagctatgaggtgaaaccttcaggcagcgccagcagcatggtcaacggggtggtcaagctgctgaccaaaccttgggacgtgatcccaatggtcactcagattgccatgaccgataccaccccattcggccagcagcgggtgttcaaggagaaggtggacacccgcacacctaaggctaaacgagggactgcacagatcatggaggtgaccgccaagtggctgtggggattcctgtccaggaacaagaagccaagaatctgtaccagggaagagttcacaagaaaggtccggtcaaacgcctaatgagcgcgcagcgcttagacgtctcgcgatcgatactagtacaacctaaatccattataaaaaacttaggagcaaagtgattgcctcccaaggtccacaatgacagagacctacgacttcgacaagtcggcatgggacatcaaagggtcgatcgctccgatacaacccaccacctacagtgatggcaggctggtgccccaggtcagagtcatagatcctggtctaggcgacaggaaggatgaatgctttatgtacatgtttctgctgggggttgttgaggacagcgattccctagggcctccaatcgggcgagcatttgggttcctgcccttaggtgttggcagatccacagcaaagcccgaaaaactcctcaaagaggccactgagcttgacatagttgttagacgtacagcagggctcaatgaaaaactggtgttctacaacaacaccccactaactctcctcacaccttggagaaaggtcctaacaacagggagtgtcttcaacgcaaaccaagtgtgcaatgcggttaatctgataccgctcgataccccgcagaggttccgtgttgtttatatgagcatcacccgtctttcggataacgggtattacaccgttcctagaagaatgctggaattcagatcggtcaatgcagtggccttcaacctgctggtgacccttaggattgacaaggcgataggccctgggaagatcatcgacaatacagagcaacttcctgaggcaacatttatggtccacatcgggaacttcaggagaaagaagagtgaagtctactctgccgattattgcaaaatgaaaatcgaaaagatgggcctggtttttgcacttggtgggatagggggcaccagtcttcacattagaagcacaggcaaaatgagcaagactctccatgcacaactcgggttcaagaagaccttatgttacccgctgatggatatcaatgaagaccttaatcgattactctggaggagcagatgcaagatagtaagaatccaggcagttttgcagccatcagttcctcaagaattccgcatttacgacgacgtgatcataaatgatgaccaaggactattcaaagttctgtagaccgtagtgcccagcaatgcccgaaaacgacccccctcacaatgacagccagaaggcccggacaaaaaagccccctccgaaagactccacggaccaagcgagaggccagccagcagccgacggcaagcgcgaacaccaggcggccccagcacagaacagccctgacacaaggccaccaccagccaccccaatctgcatcctcctcgtgggacccccgaggaccaacccccaaggctgcccccgatccaaaccaccaaccgcatccccaccacccccgggaaagaaacccccagcaattggaaggcccctccccctcttcctcaacacaagaactccacaaccgaaccgcacaagcgaccgaggtgacccaaccgcaggcatccgactccctagacagatcctctctccccggcaaactaaacaaaacttagggccaaggaacatacacacccaacagaacccagaccccggcccacggcgccgcgcccccaacccccgacaaccagagggagcccccaaccaatcccgccggctcccccggtgcccacaggcagggacaccaacccccgaacagacccagcacccaaccatcgacaatccaagacgggggggcccccccaaaaaaaggcccccaggggccgacagccagcaccgcgaggaagcccacccaccccacacacgaccacggcaaccaaaccagaacccagaccaccctgggccaccagctcccagactcggccatcaccccgcagaaaggaaaggccacaacccgcgcaccccagccccgatccggcggggagccacccaacccgaaccagcacccaagagcgatccccgaaggacccccgaaccgcaaaggacatcagtatcccacagcctctccaagtcccccggtctcctcctcttctcgaagggaccaaaagatcaatccaccacacccgacgacactcaactccccacccctaaaggagacaccgggaatcccagaatcaagactcatccaatgtccatcatgggtctcaaggtgaacgtctctgccatattcatggcagtactgttaactctccaaacacccaccggtcaaatccattggggcaatctctctaagataggggtggtaggaataggaagtgcaagctacaaagttatgactcgttccagccatcaatcattagtcataaaattaatgcccaatataactctcctcaataactgcacgagggtagagattgcagaatacaggagactactgagaacagttttggaaccaattagagatgcacttaatgcaatgacccagaatataagaccggttcagagtgtagcttcaagtaggagacacaagagatttgcgggagtagtcctggcaggtgcggccctaggcgttgccacagctgctcagataacagccggcattgcacttcaccagtccatgctgaactctcaagccatcgacaatctgagagcgagcctggaaactactaatcaggcaattgagacaatcagacaagcagggcaggagatgatattggctgttcagggtgtccaagactacatcaataatgagctgataccgtctatgaaccaactatcttgtgatttaatcggccagaagctcgggctcaaattgctcagatactatacagaaatcctgtcattatttggccccagtttacgggaccccatatctgcggagatatctatccaggctttgagctatgcgcttggaggagacatcaataaggtgttagaaaagctcggatacagtggaggtgatttactgggcatcttagagagcggaggaataaaggcccggataactcacgtcgacacagagtcctacttcattgtcctcagtatagcctatccgacgctgtccgagattaagggggtgattgtccaccggctagagggggtctcgtacaacataggctctcaagagtggtataccactgtgcccaagtatgttgcaacccaagggtaccttatctcgaattttgatgagtcatcgtgtactttcatgccagaggggactgtgtgcagccaaaatgccttgtacccgatgagtcctctgctccaagaatgcctccgggggtacaccaagtcctgtgctcgtacactcgtatccgggtcttttgggaaccggttcattttatcacaagggaacctaatagccaattgtgcatcaatcctttgcaagtgttacacaacaggaacgatcattaatcaagaccctgacaagatcctaacatacattgctgccgatcactgcccggtagtcgaggtgaacggcgtgaccatccaagtcgggagcaggaggtatccagacgctgtgtacttgcacagaattgacctcggtcctcccatatcattggagaggttggacgtagggacaaatctggggaatgcaattgctaagttggaggatgccaaggaattgttggagtcatcggaccagatattgaggagtatgaaaggtttatcgagcactagcatagtctacatcctgattgcagtgtgtcttggagggttgatagggatccccgctttaatatgttgctgcagggggcgttgtaacaaaaagggagaacaagttggtatgtcaagaccaggcctaaagcctgatcttacgggaacatcaaaatcctatgtaaggtcgctctgatcctctacaactcttgaaacacaaatgtcccacaagtctcctcttcgtcatcaagcaaccaccgcacccagcatcaagcccacctgaaattatctccggcttccctctggccgaacaatatcggtagttaatcaaaacttagggtgcaagatcatccacaatgtcaccacaacgagaccggataaatgccttctacaaagataacccccatcccaagggaagtaggatagtcattaacagagaacatcttatgattgatagaccttatgttttgctggctgttctgtttgtcatgtttctgagcttgatcgggttgctagccattgcaggcattagacttcatcgggcagccatctacaccgcagagatccataaaagcctcagcaccaatctagatgtaactaactcaatcgagcatcaggtcaaggacgtgctgacaccactcttcaaaatcatcggtgatgaagtgggcctgaggacacctcagagattcactgacctagtgaaattaatctctgacaagattaaattccttaatccggatagggagtacgacttcagagatctcacttggtgtatcaacccgccagagagaatcaaattggattatgatcaatactgtgcagatgtggctgctgaagagctcatgaatgcattggtgaactcaactctactggagaccagaacaaccaatcagttcctagctgtctcaaagggaaactgctcagggcccactacaatcagaggtcaattctcaaacatgtcgctgtccctgttagacttgtatttaggtcgaggttacaatgtgtcatctatagtcactatgacatcccagggaatgtatgggggaacttacctagtggaaaagcctaatctgagcagcaaaaggtcagagttgtcacaactgagcatgtaccgagtgtttgaagtaggtgttatcagaaatccgggtttgggggctccggtgttccatatgacaaactatcttgagcaaccagtcagtaatgatctcagcaactgtatggtggctttgggggagctcaaactcgcagccctttgtcacggggaagattctatcacaattccctatcagggatcagggaaaggtgtcagcttccagctcgtcaagctaggtgtctggaaatccccaaccgacatgcaatcctgggtccccttatcaacggatgatccagtgatagacaggctttacctctcatctcacagaggtgttatcgctgacaatcaagcaaaatgggctgtcccgacaacacgaacagatgacaagttgcgaatggagacatgcttccaacaggcgtgtaagggtaaaatccaagcactctgcgagaatcccgagtgggcaccattgaaggataacaggattccttcatacggggtcttgtctgttgatctgagtctgacagttgagcttaaaatcaaaattgcttcgggattcgggccattgatcacacacggttcagggatggacctatacaaatccaaccacaacaatgtgtattggctgactatcccgccaatgaagaacctagccttaggtgtaatcaacacattggagtggataccgagattcaaggttagtccctacctcttcactgtcccaattaaggaagcaggcgaagactgccatgccccaacatacctacctgcggaggtggatggtgatgtcaaactcagttccaatctggtgattctacctggtcaagatctccaatatgttttggcaacctacgatacttccagggttgaacatgctgtggtttattacgtttacagcccaagccgctcattttcttacttttatccttttaggttgcctataaagggggtccccatcgaattacaagtggaatgcttcacatgggaccaaaaactctggtgccgtcacttctgtgtgcttgcggactcagaatctggtggacatatcactcactctgggatggtgggcatgggagtcagctgcacagtcacccgggaagatggaaccaatcgcagatagggctgctagtgaaccaatcacatgatgtcacccagacatcaggcatacccactagtgtgaaatagacatcagaattaagaaaaacgtagggtccaagtggttccccgttatggactcgctatctgtcaaccagatcttataccctgaagttcacctagatagcccgatagttaccaataagatagtagccatcctggagtatgctcgagtccctcacgcttacagcctggaggaccctacactgtgtcagaacatcaagcaccgcctaaaaaacggattttccaaccaaatgattataaacaatgtggaagttgggaatgtcatcaagtccaagcttaggagttatccggcccactctcatattccatatccaaattgtaatcaggatttatttaacatagaagacaaagagtcaacgaggaagatccgtgaactcctcaaaaaggggaattcgctgtactccaaagtcagtgataaggttttccaatgcttaagggacactaactcacggcttggcctaggctccgaattgagggaggacatcaaggagaaagttattaacttgggagtttacatgcacagctcccagtggtttgagccctttctgttttggtttacagtcaagactgagatgaggtcagtgattaaatcacaaacccatacttgccataggaggagacacacacctgtattcttcactggtagttcagttgagttgctaatctctcgtgaccttgttgctataatcagtaaagagtctcaacatgtatattacctgacatttgaactggttttgatgtattgtgatgtcatagaggggaggttaatgacagagaccgctatgactattgatgctaggtatacagagcttctaggaagagtcagatacatgtggaaactgatagatggtttcttccctgcactcgggaatccaacttatcaaattgtagccatgctggagcctctttcacttgcttacctgcagctgagggatataacagtagaactcagaggtgctttccttaaccactgctttactgaaatacatgatgttcttgaccaaaacgggttttctgatgaaggtacttatcatgagttaactgaagctctagattacattttcataactgatgacatacatctgacaggggagattttctcatttttcagaagtttcggccaccccagacttgaagcagtaacggctgctgaaaatgttaggaaatacatgaatcagcctaaagtcattgtgtatgagactctgatgaaaggtcatgccatattttgtggaatcataatcaacggctatcgtgacaggcacggaggcagttggccaccgctgaccctccccctgcatgctgcagacacaatccggaatgctcaagcttcaggtgaagggttaacacatgagcagtgcgttgataactggaaatcttttgctggagtgaaatttggctgctttatgcctcttagcctggatagtgatctgacaatgtacctaaaggacaaggcacttgctgctctccaaagggaatgggattcagtttacccgaaagagttcctgcgttacgaccctcccaagggaaccgggtcacggaggcttgtagatgttttccttaatgattcgagctttgacccatatgatgtgataatgtatgttgtaagtggagcttacctccatgaccctgagttcaacctgtcttacagcctgaaagaaaaggagatcaaggaaacaggtagactttttgctaaaatgacttacaaaatgagggcatgccaagtgattgctgaaaatctaatctcaaacgggattggcaaatattttaaggacaatgggatggccaaggatgagcacgatttgactaaggcactccacactctagctgtctcaggagtccccaaagatctcaaagaaagtcacaggggggggccagtcttaaaaacctactcccgaagcccagtccacacaagtaccaggaacgtgagagcagcaaaagggtttatagggttccctcaagtaattcggcaggaccaagacactgatcatccggagaatatggaagcttacgagacagtcagtgcatttatcacgactgatctcaagaagtactgccttaattggagatatgagaccatcagcttgtttgcacagaggctaaatgagatttacggattgccctcatttttccagtggctgcataagaggcttgagacctctgtcctgtatgtaagtgaccctcattgcccccccgaccttgacgcccatatcccgttatataaagtccccaatgatcaaatcttcattaagtaccctatgggaggtatagaagggtattgtcagaagctgtggaccatcagcaccattccctatctatacctggctgcttatgagagcggagtaaggattgcttcgttagtgcaaggggacaatcagaccatagccgtaacaaaaagggtacccagcacatggccctacaaccttaagaaacgggaagctgctagagtaactagagattactttgtaattcttaggcaaaggctacatgatattggccatcacctcaaggcaaatgagacaattgtttcatcacatttttttgtctattcaaaaggaatatattatgatgggctacttgtgtcccaatcactcaagagcatcgcaagatgtgtattctggtcagagactatagttgatgaaacaagggcagcatgcagtaatattgctacaacaatggctaaaagcatcgagagaggttatgaccgttaccttgcatattccctgaacgtcctaaaagtgatacagcaaattctgatctctcttggcttcacaatcaattcaaccatgacccgggatgtagtcatacccctcctcacaaacaacgacctcttaataaggatggcactgttgcccgctcctattggggggatgaattatctgaatatgagcaggctgtttgtcagaaacatcggtgatccagtaacatcatcaattgctgatctcaagagaatgattctcgcctcactaatgcctgaagagaccctccatcaagtaatgacacaacaaccgggggactcttcattcctagactgggctagcgacccttactcagcaaatcttgtatgtgtccagagcatcactagactcctcaagaacataactgcaaggtttgtcctgatccatagtccaaacccaatgttaaaaggattattccatgatgacagtaaagaagaggacgagggactggcggcattcctcatggacaggcatattatagtacctagggcagctcatgaaatcctggatcatagtgtcacaggggcaagagagtctattgcaggcatgctggataccacaaaaggcttgattcgagccagcatgaggaagggggggttaacctctcgagtgataaccagattgtccaattatgactatgaacaattcagagcagggatggtgctattgacaggaagaaagagaaatgtcctcattgacaaagagtcatgttcagtgcagctggcgagagctctaagaagccatatgtgggcgaggctagctcgaggacggcctatttacggccttgaggtccctgatgtactagaatctatgcgaggccaccttattcggcgtcatgagacatgtgtcatctgcgagtgtggatcagtcaactacggatggttttttgtcccctcgggttgccaactggatgatattgacaaggaaacatcatccttgagagtcccatatattggttctaccactgatgagagaacagacatgaagcttgccttcgtaagagccccaagtcgatccttgcgatctgctgttagaatagcaacagtgtactcatgggcttacggtgatgatgatagctcttggaacgaagcctggttgttggctaggcaaagggccaatgtgagcctggaggagctaagggtgatcactcccatctcaacttcgactaatttagcgcataggttgagggatcgtagcactcaagtgaaatactcaggtacatcccttgtccgagtggcgaggtataccacaatctccaacgacaatctctcatttgtcatatcagataagaaggttgatactaactttatataccaacaaggaatgcttctagggttgggtgttttagaaacattgtttcgactcgagaaagataccggatcatctaacacggtattacatcttcacgtcgaaacagattgttgcgtgatcccgatgatagatcatcccaggatacccagctcccgcaagctagagctgagggcagagctatgtaccaacccattgatatatgataatgcacctttaattgacagagatgcaacaaggctatacacccagagccataggaggcaccttgtggaatttgttacatggtccacaccccaactatatcacattttagctaagtccacagcactatctatgattgacctggtaacaaaatttgagaaggaccatatgaatgaaatttcagctctcataggggatgacgatatcaatagtttcataactgagtttctgctcatagagccaagattattcactatctacttgggccagtgtgcggccatcaattgggcatttgatgtacattatcatagaccatcagggaaatatcagatgggtgagctgttgtcatcgttcctttctagaatgagcaaaggagtgtttaaggtgcttgtcaatgctctaagccacccaaagatctacaagaaattctggcattgtggtattatagagcctatccatggtccttcacttgatgctcaaaacttgcacacaactgtgtgcaacatggtttacacatgctatatgacctacctcgacctgttgttgaatgaagagttagaagagttcacatttctcttgtgtgaaagcgacgaggatgtagtaccggacagattcgacaacatccaggcaaaacacttatgtgttctggcagatttgtactgtcaaccagggacctgcccaccaattcgaggtctaagaccggtagagaaatgtgcagttctaaccgaccatatcaaggcagaggctatgttatctccagcaggatcttcgtggaacataaatccaattattgtagaccattactcatgctctctgacttatctccggcgaggatcgatcaaacagataagattgagagttgatccaggattcattttcgacgccctcgctgaggtaaatgtcagtcagccaaagatcggcagcaacaacatctcaaatatgagcatcaaggctttcagacccccacacgatgatgttgcaaaattgctcaaagatatcaacacaagcaagcacaatcttcccatttcagggggcaatctcgccaattatgaaatccatgctttccgcagaatcgggttgaactcatctgcttgctacaaagctgttgagatatcaacattaattaggagatgccttgagccaggggaggacggcttgttcttgggtgagggatcgggttctatgttgatcacttataaagagatacttaaactaaacaagtgcttctataatagtggggtttccgccaattctagatctggtcaaagggaattagcaccctatccctccgaagttggccttgtcgaacacagaatgggagtaggtaatattgtcaaagtgctctttaacgggaggcccgaagtcacgtgggtaggcagtgtagattgcttcaatttcatagttagtaatatccctacctctagtgtggggtttatccattcagatatagagaccttgcctgacaaagatactatagagaagctagaggaattggcagccatcttatcgatggctctgctcctgggcaaaataggatcaatactggtgattaagcttatgcctttcagcggggattttgttcagggatttataagttatgtagggtctcattatagagaagtgaaccttgtataccctagatacagcaacttcatctctactgaatcttatttggttatgacagatctcaaggctaaccggctaatgaatcctgaaaagattaagcagcagataattgaatcatctgtgaggacttcacctggacttataggtcacatcctatccattaagcaactaagctgcatacaagcaattgtgggagacgcagttagtagaggtgatatcaatcctactctgaaaaaacttacacctatagagcaggtgctgatcaattgcgggttggcaattaacggacctaagctgtgcaaagaattgatccaccatgatgttgcctcagggcaagatggattgcttaattctatactcatcctctacagggagttggcaagattcaaagacaaccaaagaagtcaacaagggatgttccacgcttaccccgtattggtaagtagcaggcaacgagaacttatatctaggatcacccgcaaattctgggggcacattcttctttactccgggaacaaaaagttgataaataagtttatccagaatctcaagtccggctatctgatactagacttacaccagaatatcttcgttaagaatctatccaagtcagagaaacagattattatgacggggggtttgaaacgtgagtgggtttttaaggtaacagtcaaggagaccaaagaatggtataagttagtcggatacagtgccctgattaaggactaattggttgaactccggaaccctaatcctgccctaggtggttaggcattatttgcaatatattaaagaaaactttgaaaatacgaagtttctattcccagctttgtctggtggccggcatggtcccagcctcctcgctggcgccggctgggcaacattccgaggggaccgtcccctcggtaatggcgaatgggacgcggccgatccggctgctaacaaagcccgaaaggaagctgagttggctgctgccaccgctgagcaataactagcataaccccttggggcctctaaacgggtcttgaggggttttttgctgaaaggaggaactatatccggatgcggccgcgggccctatggtacccagcttttgttccctttagtgagggttaattccgagcttggcgtaatcatggtcatagctgtttcctgtgtgaaattgttatccgctcacaattccacacaacataggagccggaagcataaagtgtaaagcctggggtgcctaatgagtgaggtaactcacattaattgcgttgcgctcactgcccgctttccagtcgggaaacctgtcgtgccagctgcattaatgaatcggccaacgcgcggggagaggcggtttgcgtattgggcgctcttccgcttcctcgctcactgactcgctgcgctcggtcgttcggctgcggcgagcggtatcagctcactcaaaggcggtaatacggttatccacagaatcaggggataacgcaggaaagaacatgtgagcaaaaggccagcaaaaggccaggaaccgtaaaaaggccgcgttgctggcgtttttccataggctcggcccccctgacgagcatcacaaaaatcgacgctcaagtcagaggtggcgaaacccgacaggactataaagataccaggcgttcccccctggaagctccctcgtgcgctctcctgttccgaccctgccgcttaccggatacctgtccgcctttctcccttcgggaagcgtggcgctttctcaatgctcacgctgtaggtatctcagttcggtgtaggtcgttcgctccaagctgggctgtgtgcacgaaccccccgttcagcccgaccgctgcgccttatccggtaactatcgtcttgagtccaacccggtaagacacgacttatcgccactggcagcagccactggtaacaggattagcagagcgaggtatgtaggcggtgctacagagttcttgaagtggtggcctaactacggctacactagaaggacagtatttggtatctgcgctctgctgaagccagttaccttcggaaaaagagttggtagctcttgatccggcaaacaaaccaccgctggtagcggtggtttttttgtttgcaagcagcagattacgcgcagaaaaaaaggatctcaagaagatcctttgatcttttctacggggtctgacgctcagtggaacgaaaactcacgttaagggattttggtcatgagattatcaaaaaggatcttcacctagatccttttaaattaaaaatgaagttttaaatcaatctaaagtatatatgagtaaacttggtctgacagttaccaatgcttaatcagtgaggcacctatctcagcgatctgtctatttcgttcatccatagttgcctgactgcccgtcgtgtagataactacgatacgggagggcttaccatctggccccagtgctgcaatgataccgcgagacccacgctcaccggctccagatttatcagcaataaaccagccagccggaagggccgagcgcagaagtggtcctgcaactttatccgcctccatccagtctattaattgttgccgggaagctagagtaagtagttcgccagttaatagtttgcgcaacgttgttgccattgctacaggcatcgtggtgtcacgctcgtcgtttggtatggcttcattcagctccggttcccaacgatcaaggcgagttacatgatcccccatgttgtgaaaaaaagcggttagctccttcggtcctccgatcgttgtcagaagtaagttggccgcagtgttatcactcatgcttatggcagcactgcataattctcttactgtcatgccatccgtaagatgcttttctgtgactggtgagtactcaaccaagtcattctgagaatagtgtatgcggcgaccgagttgctcttgcccggcgtcaatacgggataataccgcgccacatagcagaactttaaaagtgctcatcattggaaaacgttcttcggggcgaaaactctcaaggatcttaccgctgttgagatccagttcgatgtaacccactcgtgcacccaactgatcttcagcatcttttactttcaccagcgtttctgggtgagcaaaaacaggaaggcaaaatgccgcaaaaaagggaataagggcgacacggaaatgttgaatactcatactcttcctttttcaatattattgaagcatttatcagggttattgtctcatgagcggatacatatttgaatgtatttagaaaaataaacaaataggggttccgcgcacatttccccgaaaagtgccacctgaaattgtaaacgttaatattttgttaaaattcgcgttaaatttttgttaaatcagctcattttttaaccaataggccgaaatcggcaaaatcccttataaatcaaaagaatagaccgagatagggttgagtgttgttccagtttggaacaagagtccactattaaagaacgtggactccaacgtcaaagggcgaaaaaccgtctatcagggcgatggcccactacgtgaaccatcaccctaatcaagttttttggggtcgaggtgccgtaaagcactaaatcggaaccctaaagggagcccccgatttagagcttgacggggaaagccggcgaacgtggcgagaaaggaagggaagaaagcgaaaggagcgggcgctagggcgctggcaagtgtagcggtcacgctgcgcgtaaccaccacacccgccgcgcttaatgcgccgctacagggcgcgtcccattcgccattcaggctgcgcaactgttgggaagggcgatcggtgcgggcctcttcgctattacgccagccaccgcggtg

SEQ ID NO: 143 - DNA, 22363 bp, Artificial Sequence
  Complete optimised nucleotide sequence of the polynucleotide encoding pTM-MVDVax10
  misc_feature (1)..(8): NotI
  misc_feature (9)..(28): T7 promoter
  misc_feature (29)..(82): Hammerhead ribozyme
  misc_feature (83)..(189): MV Leader and N promoter
  misc_feature (190)..(1767): MV N ORF
  misc_feature (1768)..(1888): MV N-P intergenic
  misc_feature (1889)..(3412): MV P ORF
  misc_feature (3413)..(3531): MV ATU2
  misc_feature (3532)..(5154): DENV1 NS polyepitope
  misc_feature (5155)..(5253): MV P-M intergenic
  misc_feature (5254)..(6261): MV M ORF
  misc_feature (6262)..(7264): MV M-F intergenic
  misc_feature (7265)..(8926): MV F ORF
  misc_feature (8927)..(9086): MV-F-H intergenic
  misc_feature (9087)..(10940): MV H ORF
  misc_feature (10941)..(11067): MV ATU3
  misc_feature (11068)..(12618): DENV tetra EDIII + ectoM
  misc_feature (12619)..(12711): MV H-L intergenic
  misc_feature (12712)..(19263): MV L ORF
  misc_feature (19264)..(19372): MV Trailer
  misc_feature (19373)..(19456): HDV ribozyme
  misc_feature (19457)..(19598): T7 terminator
  misc_feature (19599)..(19606): Not I
  misc_feature (19607)..(122363): pTM plasmid
gcggccgctaatacgactcactatagggccaactttgtttggtctgatgagtccgtgaggacgaaacccggagtcccgggtcaccaaacaaagttgggtaaggatagttcaatcaatgatcatcttctagtgcacttaggattcaagatcctattatcagggacaagagcaggattagggatatccgagatggccacacttttaaggagcttagcattgttcaaaagaaacaaggacaaaccacccattacatcaggatccggtggagccatcagaggaatcaaacacattattatagtaccaatccctggagattcctcaattaccactcgatccagacttctggaccggttggtgaggttaattggaaacccggatgtgagcgggcccaaactaacaggggcactaataggtatattatccttatttgtggagtctccaggtcaattgattcagaggatcaccgatgaccctgacgttagcataaggctgttagaggttgtccagagtgaccagtcacaatctggccttaccttcgcatcaagaggtaccaacatggaggatgaggcggaccaatacttttcacatgatgatccaattagtagtgatcaatccaggttcggatggttcgggaacaaggaaatctcagatattgaagtgcaagaccctgagggattcaacatgattctgggtaccatcctagcccaaatttgggtcttgctcgcaaaggcggttacggccccagacacggcagctgattcggagctaagaaggtggataaagtacacccaacaaagaagggtagttggtgaatttagattggagagaaaatggttggatgtggtgaggaacaggattgccgaggacctctccttacgccgattcatggtcgctctaatcctggatatcaagagaacacccggaaacaaacccaggattgctgaaatgatatgtgacattgatacatatatcgtagaggcaggattagccagttttatcctgactattaagtttgggatagaaactatgtatcctgctcttggactgcatgaatttgctggtgagttatccacacttgagtccttgatgaacctttaccagcaaatgggggaaactgcaccctacatggtaatcctggagaactcaattcagaacaagttcagtgcaggatcataccctctgctctggagctatgccatgggagtaggagtggaacttgaaaactccatgggaggtttgaactttggccgatcttactttgatccagcatattttagattagggcaagagatggtaaggaggtcagctggaaaggtcagttccacattggcatctgaactcggtatcactgccgaggatgcaaggcttgtttcagagattgcaatgcatactactgaggacaagatcagtagagcggttggacccagacaagcccaagtatcatttctacacggtgatcaaagtgagaatgagctaccgagattggggggcaaggaagataggagggtcaaacagagtcgaggagaagccagggagagctacagagaaaccgggcccagcagagcaagtgatgcgagagctgcccatcttccaaccggcacacccctagacattgacactgcaacggagtccagccaagatccgcaggacagtcgaaggtcagctgacgccctgcttaggctgcaagccatggcaggaatctcggaagaacaaggctcagacacggacacccctatagtgtacaatgacagaaatcttctagactaggtgcgagaggccgagggccagaacaacatccgcctaccatccatcattgttataaaaaacttaggaaccaggtccacacagccgccagcccatcaaccatccactcccacgattggagccaatggcagaagagcaggcacgccatgtcaaaaacggactggaatgcatccgggctctcaaggccgagcccatcggctcactggccatcgaggaagctatggcagcatggtcagaaatatcagacaacccaggacaggagcgagccacctgcagggaagagaaggcaggcagttcgggtctcagcaaaccatgcctctcagcaattggatcaactgaaggcggtgcacctcgcatccgcggtcagggacctggagagagcgatgacgacgctgaaactttgggaatccccccaagaaatctccaggcatcaagcactgggttacagtgttattacgtttatgatcacagcggtgaagcggttaagggaatccaagatgctgactctatcatggttcaatcaggccttgatggtgatagcaccctctcaggaggagacaatgaatctgaaaacagcgatgtggatattggcgaacctgataccgagggatatgctatcactgaccggggatctgctcccatctctatggggttcagggcttctgatgttgaaactgcagaaggaggggagatccacgagctcctgagactccaatccagaggcaacaactttccgaagcttgggaaaactctcaatgttcctccgcccccggaccccggtagggccagcacttccgggacacccattaaaaagggcacagacgcgagattagcctcatttggaacggagatcgcgtctttattgacaggtggtgcaacccaatgtgctcgaaagtcaccctcggaaccatcagggccaggtgcacctgcggggaatgtccccgagtgtgtgagcaatgccgcactgatacaggagtggacacccgaatctggtaccacaatctccccgagatcccagaataatgaagaagggggagactattatgatgatgagctgttctctgatgtccaagatattaaaacagccttggccaaaatacacgaggataatcagaagataatctccaagctagaatcactgctgttattgaagggagaagttgagtcaattaagaagcagatcaacaggcaaaatatcagcatatccaccctggaaggacacctctcaagcatcatgatcgccattcctggacttgggaaggatcccaacgaccccactgcagatgtcgaaatcaatcccgacttgaaacccatcataggcagagattcaggccgagcactggccgaagttctcaagaaacccgttgccagccgacaactccaaggaatgacaaatggacggaccagttccagaggacagctgctgaaggaatttcagctaaagccgatcgggaaaaagatgagctcagccgtcgggtttgttcctgacaccggccctgcatcacgcagtgtaatccgctccattataaaatccagccggctagaggaggatcggaagcgttacctgatgactctccttgatgatatcaaaggagccaatgatcttgccaagttccaccagatgctgatgaagataataatgaagtagctacagctcaacttacctgccaaccccatgccagtcgacccaactagcctaccctccatcattgttataaaaaacttaggaaccaggtccacacagccgccagcccatcaacgcgtacgatggcatcacaggagggaccactgcccgaaattgaggacgaagtgtttagaaagcgaaatctgactattatggacctgcaccccggatctggcaagacccggagatacctgccagccatcgtgagggaggctattaagcggaaactgagaacactgatcctggccccaactcgcgtggtcgcttccgaaatggctgaggccctgaaaggcatgcccatccggtatcagaccacagcagtgaagtctgaacataccggcaaggagattgtggacctgatgtgccacgccactttcaccatgcgactgctgagcccagtgcgggtccccaactacaatatgatcattatggacgaggcccactttactgatcccagctccatcgccgctagaggatatatttccaccagggtgggaatgggcgaggcagcagctatcttcatgacagcaactccccctggcagcgtggaggcatttcctcagtccaacgccgtcatccaggacgaggagcgggacattcctgagcggagctggaattctgggtacgaatggatcacagacgaggatcatgcacactggactgaagccaagatgctgctggacaacattaatactcctgagggaatcattccagctctgttcgagcccgaaagagagaagtctgcagccatcgacggcgagtatagactgaggggagaggcccggaagaccttcgtggaactgatgaggcgcggcgatctgcccgtgtggctgagttacaaggtcgcttcagagggattccagtatagtgaccgacggtggtgctttgatggcgaacgcaacaatcaggtgctggaggagaacatggatgtcgagatttggacaaaggaaggcgagcggaagaaactgcgcccacgatggctggacgctcggacttacagcgatcccctggcactgagagaattcaaagagtttgctgcaggggtggccgtcgagaatcaccatcacgccgctatgctggacgtggatctgcatcctgccagtgcttggaccctgtatgcagtggccactaccatcattaccccaatgatgcgccacacaatcgagaacacaactgccaatatctcactgacagctattgcaaaccaggcagccattctgatgggactggacaaaggctggcccatcagcaagatggatattggcgtgcctctgctggccctggggtgttacagtcaggtgctggacatcattggccagaggatcgagaacattaagcatgagcacaaatcaacctggcattacgacgaagataatccctataagacatgggcctaccacggaagctatgaggtgaaaccttcaggcagcgccagcagcatggtcaacggggtggtcaagctgctgaccaaaccttgggacgtgatcccaatggtcactcagattgccatgaccgataccaccccattcggccagcagcgggtgttcaaggagaaggtggacacccgcacacctaaggctaaacgagggactgcacagatcatggaggtgaccgccaagtggctgtggggattcctgtccaggaacaagaagccaagaatctgtaccagggaagagttcacaagaaaggtccggtcaaacgcctaatgagcgcgcagcgcttagacgtctcgcgatcgatactagtacaacctaaatccattataaaaaacttaggagcaaagtgattgcctcccaaggtccacaatgacagagacctacgacttcgacaagtcggcatgggacatcaaagggtcgatcgctccgatacaacccaccacctacagtgatggcaggctggtgccccaggtcagagtcatagatcctggtctaggcgacaggaaggatgaatgctttatgtacatgtttctgctgggggttgttgaggacagcgattccctagggcctccaatcgggcgagcatttgggttcctgcccttaggtgttggcagatccacagcaaagcccgaaaaactcctcaaagaggccactgagcttgacatagttgttagacgtacagcagggctcaatgaaaaactggtgttctacaacaacaccccactaactctcctcacaccttggagaaaggtcctaacaacagggagtgtcttcaacgcaaaccaagtgtgcaatgcggttaatctgataccgctcgataccccgcagaggttccgtgttgtttatatgagcatcacccgtctttcggataacgggtattacaccgttcctagaagaatgctggaattcagatcggtcaatgcagtggccttcaacctgctggtgacccttaggattgacaaggcgataggccctgggaagatcatcgacaatacagagcaacttcctgaggcaacatttatggtccacatcgggaacttcaggagaaagaagagtgaagtctactctgccgattattgcaaaatgaaaatcgaaaagatgggcctggtttttgcacttggtgggatagggggcaccagtcttcacattagaagcacaggcaaaatgagcaagactctccatgcacaactcgggttcaagaagaccttatgttacccgctgatggatatcaatgaagaccttaatcgattactctggaggagcagatgcaagatagtaagaatccaggcagttttgcagccatcagttcctcaagaattccgcatttacgacgacgtgatcataaatgatgaccaaggactattcaaagttctgtagaccgtagtgcccagcaatgcccgaaaacgacccccctcacaatgacagccagaaggcccggacaaaaaagccccctccgaaagactccacggaccaagcgagaggccagccagcagccgacggcaagcgcgaacaccaggcggccccagcacagaacagccctgacacaaggccaccaccagccaccccaatctgcatcctcctcgtgggacccccgaggaccaacccccaaggctgcccccgatccaaaccaccaaccgcatccccaccacccccgggaaagaaacccccagcaattggaaggcccctccccctcttcctcaacacaagaactccacaaccgaaccgcacaagcgaccgaggtgacccaaccgcaggcatccgactccctagacagatcctctctccccggcaaactaaacaaaacttagggccaaggaacatacacacccaacagaacccagaccccggcccacggcgccgcgcccccaacccccgacaaccagagggagcccccaaccaatcccgccggctcccccggtgcccacaggcagggacaccaacccccgaacagacccagcacccaaccatcgacaatccaagacgggggggcccccccaaaaaaaggcccccaggggccgacagccagcaccgcgaggaagcccacccaccccacacacgaccacggcaaccaaaccagaacccagaccaccctgggccaccagctcccagactcggccatcaccccgcagaaaggaaaggccacaacccgcgcaccccagccccgatccggcggggagccacccaacccgaaccagcacccaagagcgatccccgaaggacccccgaaccgcaaaggacatcagtatcccacagcctctccaagtcccccggtctcctcctcttctcgaagggaccaaaagatcaatccaccacacccgacgacactcaactccccacccctaaaggagacaccgggaatcccagaatcaagactcatccaatgtccatcatgggtctcaaggtgaacgtctctgccatattcatggcagtactgttaactctccaaacacccaccggtcaaatccattggggcaatctctctaagataggggtggtaggaataggaagtgcaagctacaaagttatgactcgttccagccatcaatcattagtcataaaattaatgcccaatataactctcctcaataactgcacgagggtagagattgcagaatacaggagactactgagaacagttttggaaccaattagagatgcacttaatgcaatgacccagaatataagaccggttcagagtgtagcttcaagtaggagacacaagagatttgcgggagtagtcctggcaggtgcggccctaggcgttgccacagctgctcagataacagccggcattgcacttcaccagtccatgctgaactctcaagccatcgacaatctgagagcgagcctggaaactactaatcaggcaattgagacaatcagacaagcagggcaggagatgatattggctgttcagggtgtccaagactacatcaataatgagctgataccgtctatgaaccaactatcttgtgatttaatcggccagaagctcgggctcaaattgctcagatactatacagaaatcctgtcattatttggccccagtttacgggaccccatatctgcggagatatctatccaggctttgagctatgcgcttggaggagacatcaataaggtgttagaaaagctcggatacagtggaggtgatttactgggcatcttagagagcggaggaataaaggcccggataactcacgtcgacacagagtcctacttcattgtcctcagtatagcctatccgacgctgtccgagattaagggggtgattgtccaccggctagagggggtctcgtacaacataggctctcaagagtggtataccactgtgcccaagtatgttgcaacccaagggtaccttatctcgaattttgatgagtcatcgtgtactttcatgccagaggggactgtgtgcagccaaaatgccttgtacccgatgagtcctctgctccaagaatgcctccgggggtacaccaagtcctgtgctcgtacactcgtatccgggtcttttgggaaccggttcattttatcacaagggaacctaatagccaattgtgcatcaatcctttgcaagtgttacacaacaggaacgatcattaatcaagaccctgacaagatcctaacatacattgctgccgatcactgcccggtagtcgaggtgaacggcgtgaccatccaagtcgggagcaggaggtatccagacgctgtgtacttgcacagaattgacctcggtcctcccatatcattggagaggttggacgtagggacaaatctggggaatgcaattgctaagttggaggatgccaaggaattgttggagtcatcggaccagatattgaggagtatgaaaggtttatcgagcactagcatagtctacatcctgattgcagtgtgtcttggagggttgatagggatccccgctttaatatgttgctgcagggggcgttgtaacaaaaagggagaacaagttggtatgtcaagaccaggcctaaagcctgatcttacgggaacatcaaaatcctatgtaaggtcgctctgatcctctacaactcttgaaacacaaatgtcccacaagtctcctcttcgtcatcaagcaaccaccgcacccagcatcaagcccacctgaaattatctccggcttccctctggccgaacaatatcggtagttaatcaaaacttagggtgcaagatcatccacaatgtcaccacaacgagaccggataaatgccttctacaaagataacccccatcccaagggaagtaggatagtcattaacagagaacatcttatgattgatagaccttatgttttgctggctgttctgtttgtcatgtttctgagcttgatcgggttgctagccattgcaggcattagacttcatcgggcagccatctacaccgcagagatccataaaagcctcagcaccaatctagatgtaactaactcaatcgagcatcaggtcaaggacgtgctgacaccactcttcaaaatcatcggtgatgaagtgggcctgaggacacctcagagattcactgacctagtgaaattaatctctgacaagattaaattccttaatccggatagggagtacgacttcagagatctcacttggtgtatcaacccgccagagagaatcaaattggattatgatcaatactgtgcagatgtggctgctgaagagctcatgaatgcattggtgaactcaactctactggagaccagaacaaccaatcagttcctagctgtctcaaagggaaactgctcagggcccactacaatcagaggtcaattctcaaacatgtcgctgtccctgttagacttgtatttaggtcgaggttacaatgtgtcatctatagtcactatgacatcccagggaatgtatgggggaacttacctagtggaaaagcctaatctgagcagcaaaaggtcagagttgtcacaactgagcatgtaccgagtgtttgaagtaggtgttatcagaaatccgggtttgggggctccggtgttccatatgacaaactatcttgagcaaccagtcagtaatgatctcagcaactgtatggtggctttgggggagctcaaactcgcagccctttgtcacggggaagattctatcacaattccctatcagggatcagggaaaggtgtcagcttccagctcgtcaagctaggtgtctggaaatccccaaccgacatgcaatcctgggtccccttatcaacggatgatccagtgatagacaggctttacctctcatctcacagaggtgttatcgctgacaatcaagcaaaatgggctgtcccgacaacacgaacagatgacaagttgcgaatggagacatgcttccaacaggcgtgtaagggtaaaatccaagcactctgcgagaatcccgagtgggcaccattgaaggataacaggattccttcatacggggtcttgtctgttgatctgagtctgacagttgagcttaaaatcaaaattgcttcgggattcgggccattgatcacacacggttcagggatggacctatacaaatccaaccacaacaatgtgtattggctgactatcccgccaatgaagaacctagccttaggtgtaatcaacacattggagtggataccgagattcaaggttagtccctacctcttcactgtcccaattaaggaagcaggcgaagactgccatgccccaacatacctacctgcggaggtggatggtgatgtcaaactcagttccaatctggtgattctacctggtcaagatctccaatatgttttggcaacctacgatacttccagggttgaacatgctgtggtttattacgtttacagcccaagccgctcattttcttacttttatccttttaggttgcctataaagggggtccccatcgaattacaagtggaatgcttcacatgggaccaaaaactctggtgccgtcacttctgtgtgcttgcggactcagaatctggtggacatatcactcactctgggatggtgggcatgggagtcagctgcacagtcacccgggaagatggaaccaatcgcagatagggctgctagtgaaccaatcacatgatgtcacccagacatcaggcatacccactagtctaccctccatcattgttataaaaaacttaggaaccaggtccacacagccgccagcccatcaacgcgtacgatgggcatcatattcattcttcttatgctggttacaccgtctatggcggagaaacttcgaatcaaaggtatgagctatacgatgtgcagcggcaagttcaagatcgagaaggaaatggctgaaacccagcacggtacaactgtggtcaaagtcaaatatgagggggctggcgctccctgtaaagtacccattgagattagggacgtcaataaagagaaggtggtaggtcgcatcatctccagtacacctttggccgagaacacgaactccgtcacaaacatagagttggaacccccgttcggagactcatacattgtgatcggggtgggcaactctgcactcacactgcattggttcaagaagggaagcagtatcggccgcagggataagagagacaaactgaaattgaaaggtatgtcctatgccatgtgcacgaatactttcgttctcaagaaagaagtatctgagactcagcacggaaccatcctgatcaaagtcgagtacaaaggagaagacgtgccctgtaagatcccattcagtaccgaggatggacagggcaaggcccataacggcaggctgataaccgccaaccctgtggttacaaagaaggaagagccagtcaatatcgaagctgagccaccgttcggggagagcaacatagtaattggcataggggataatgctttgaagatcaactggtacaagaaaggaagctccattggccgaagagataagcgcgacaaactccagctgaaaggaatgagctactccatgtgtactgggaagttcaagattgtcaaggaaatcgccgaaactcagcatggcactattgtgatccgcgtgcagtatgaaggcgatggtagcccctgcaagataccatttgaaatcaccgatttggagaaacggcacgtcctgggtcggctcattaccgtgaacccaatcgtgaccgagaaggacagtccagttaatatcgaggccgagcctcctttcggcgacagttacatcattgtaggggtggaaccagggcaactgaagctgaactggttcaagaaaggcagcagtataggacggcgggataaacgggacaaactcacactgaaaggcatgtcatacgttatgtgcaccggctcattcaaactggagaaggaagttgcagagacacagcatgggaccgtgctcgtgcaggtcaaatacgagggcaccgacgctccttgcaagattccgttcagtacacaggacgagaaaggcgtgactcagaacggcagattgattacagcgaaccctatcgtgactgacaaggagaagccagttaacatcgagactgagccgcctttcggagaatcatacattatcgtgggagccggcgagaaggcactgaaactcagctggttcaagaagggcagctcaatcggtcggagagacaagcggtctgtcgccctcgcaccgcacgtgggcctgggtctggaaacgaggaccgagacgtggatgagttccgaaggcgcatggaagcaaatccagaaagtggagacgtgggccctcaggcatccgtaatgagcgcgcagcgcttagacgtctcgcgatcgatgctagtgtgaaatagacatcagaattaagaaaaacgtagggtccaagtggttccccgttatggactcgctatctgtcaaccagatcttataccctgaagttcacctagatagcccgatagttaccaataagatagtagccatcctggagtatgctcgagtccctcacgcttacagcctggaggaccctacactgtgtcagaacatcaagcaccgcctaaaaaacggattttccaaccaaatgattataaacaatgtggaagttgggaatgtcatcaagtccaagcttaggagttatccggcccactctcatattccatatccaaattgtaatcaggatttatttaacatagaagacaaagagtcaacgaggaagatccgtgaactcctcaaaaaggggaattcgctgtactccaaagtcagtgataaggttttccaatgcttaagggacactaactcacggcttggcctaggctccgaattgagggaggacatcaaggagaaagttattaacttgggagtttacatgcacagctcccagtggtttgagccctttctgttttggtttacagtcaagactgagatgaggtcagtgattaaatcacaaacccatacttgccataggaggagacacacacctgtattcttcactggtagttcagttgagttgctaatctctcgtgaccttgttgctataatcagtaaagagtctcaacatgtatattacctgacatttgaactggttttgatgtattgtgatgtcatagaggggaggttaatgacagagaccgctatgactattgatgctaggtatacagagcttctaggaagagtcagatacatgtggaaactgatagatggtttcttccctgcactcgggaatccaacttatcaaattgtagccatgctggagcctctttcacttgcttacctgcagctgagggatataacagtagaactcagaggtgctttccttaaccactgctttactgaaatacatgatgttcttgaccaaaacgggttttctgatgaaggtacttatcatgagttaactgaagctctagattacattttcataactgatgacatacatctgacaggggagattttctcatttttcagaagtttcggccaccccagacttgaagcagtaacggctgctgaaaatgttaggaaatacatgaatcagcctaaagtcattgtgtatgagactctgatgaaaggtcatgccatattttgtggaatcataatcaacggctatcgtgacaggcacggaggcagttggccaccgctgaccctccccctgcatgctgcagacacaatccggaatgctcaagcttcaggtgaagggttaacacatgagcagtgcgttgataactggaaatcttttgctggagtgaaatttggctgctttatgcctcttagcctggatagtgatctgacaatgtacctaaaggacaaggcacttgctgctctccaaagggaatgggattcagtttacccgaaagagttcctgcgttacgaccctcccaagggaaccgggtcacggaggcttgtagatgttttccttaatgattcgagctttgacccatatgatgtgataatgtatgttgtaagtggagcttacctccatgaccctgagttcaacctgtcttacagcctgaaagaaaaggagatcaaggaaacaggtagactttttgctaaaatgacttacaaaatgagggcatgccaagtgattgctgaaaatctaatctcaaacgggattggcaaatattttaaggacaatgggatggccaaggatgagcacgatttgactaaggcactccacactctagctgtctcaggagtccccaaagatctcaaagaaagtcacaggggggggccagtcttaaaaacctactcccgaagcccagtccacacaagtaccaggaacgtgagagcagcaaaagggtttatagggttccctcaagtaattcggcaggaccaagacactgatcatccggagaatatggaagcttacgagacagtcagtgcatttatcacgactgatctcaagaagtactgccttaattggagatatgagaccatcagcttgtttgcacagaggctaaatgagatttacggattgccctcatttttccagtggctgcataagaggcttgagacctctgtcctgtatgtaagtgaccctcattgcccccccgaccttgacgcccatatcccgttatataaagtccccaatgatcaaatcttcattaagtaccctatgggaggtatagaagggtattgtcagaagctgtggaccatcagcaccattccctatctatacctggctgcttatgagagcggagtaaggattgcttcgttagtgcaaggggacaatcagaccatagccgtaacaaaaagggtacccagcacatggccctacaaccttaagaaacgggaagctgctagagtaactagagattactttgtaattcttaggcaaaggctacatgatattggccatcacctcaaggcaaatgagacaattgtttcatcacatttttttgtctattcaaaaggaatatattatgatgggctacttgtgtcccaatcactcaagagcatcgcaagatgtgtattctggtcagagactatagttgatgaaacaagggcagcatgcagtaatattgctacaacaatggctaaaagcatcgagagaggttatgaccgttaccttgcatattccctgaacgtcctaaaagtgatacagcaaattctgatctctcttggcttcacaatcaattcaaccatgacccgggatgtagtcatacccctcctcacaaacaacgacctcttaataaggatggcactgttgcccgctcctattggggggatgaattatctgaatatgagcaggctgtttgtcagaaacatcggtgatccagtaacatcatcaattgctgatctcaagagaatgattctcgcctcactaatgcctgaagagaccctccatcaagtaatgacacaacaaccgggggactcttcattcctagactgggctagcgacccttactcagcaaatcttgtatgtgtccagagcatcactagactcctcaagaacataactgcaaggtttgtcctgatccatagtccaaacccaatgttaaaaggattattccatgatgacagtaaagaagaggacgagggactggcggcattcctcatggacaggcatattatagtacctagggcagctcatgaaatcctggatcatagtgtcacaggggcaagagagtctattgcaggcatgctggataccacaaaaggcttgattcgagccagcatgaggaagggggggttaacctctcgagtgataaccagattgtccaattatgactatgaacaattcagagcagggatggtgctattgacaggaagaaagagaaatgtcctcattgacaaagagtcatgttcagtgcagctggcgagagctctaagaagccatatgtgggcgaggctagctcgaggacggcctatttacggccttgaggtccctgatgtactagaatctatgcgaggccaccttattcggcgtcatgagacatgtgtcatctgcgagtgtggatcagtcaactacggatggttttttgtcccctcgggttgccaactggatgatattgacaaggaaacatcatccttgagagtcccatatattggttctaccactgatgagagaacagacatgaagcttgccttcgtaagagccccaagtcgatccttgcgatctgctgttagaatagcaacagtgtactcatgggcttacggtgatgatgatagctcttggaacgaagcctggttgttggctaggcaaagggccaatgtgagcctggaggagctaagggtgatcactcccatctcaacttcgactaatttagcgcataggttgagggatcgtagcactcaagtgaaatactcaggtacatcccttgtccgagtggcgaggtataccacaatctccaacgacaatctctcatttgtcatatcagataagaaggttgatactaactttatataccaacaaggaatgcttctagggttgggtgttttagaaacattgtttcgactcgagaaagataccggatcatctaacacggtattacatcttcacgtcgaaacagattgttgcgtgatcccgatgatagatcatcccaggatacccagctcccgcaagctagagctgagggcagagctatgtaccaacccattgatatatgataatgcacctttaattgacagagatgcaacaaggctatacacccagagccataggaggcaccttgtggaatttgttacatggtccacaccccaactatatcacattttagctaagtccacagcactatctatgattgacctggtaacaaaatttgagaaggaccatatgaatgaaatttcagctctcataggggatgacgatatcaatagtttcataactgagtttctgctcatagagccaagattattcactatctacttgggccagtgtgcggccatcaattgggcatttgatgtacattatcatagaccatcagggaaatatcagatgggtgagctgttgtcatcgttcctttctagaatgagcaaaggagtgtttaaggtgcttgtcaatgctctaagccacccaaagatctacaagaaattctggcattgtggtattatagagcctatccatggtccttcacttgatgctcaaaacttgcacacaactgtgtgcaacatggtttacacatgctatatgacctacctcgacctgttgttgaatgaagagttagaagagttcacatttctcttgtgtgaaagcgacgaggatgtagtaccggacagattcgacaacatccaggcaaaacacttatgtgttctggcagatttgtactgtcaaccagggacctgcccaccaattcgaggtctaagaccggtagagaaatgtgcagttctaaccgaccatatcaaggcagaggctatgttatctccagcaggatcttcgtggaacataaatccaattattgtagaccattactcatgctctctgacttatctccggcgaggatcgatcaaacagataagattgagagttgatccaggattcattttcgacgccctcgctgaggtaaatgtcagtcagccaaagatcggcagcaacaacatctcaaatatgagcatcaaggctttcagacccccacacgatgatgttgcaaaattgctcaaagatatcaacacaagcaagcacaatcttcccatttcagggggcaatctcgccaattatgaaatccatgctttccgcagaatcgggttgaactcatctgcttgctacaaagctgttgagatatcaacattaattaggagatgccttgagccaggggaggacggcttgttcttgggtgagggatcgggttctatgttgatcacttataaagagatacttaaactaaacaagtgcttctataatagtggggtttccgccaattctagatctggtcaaagggaattagcaccctatccctccgaagttggccttgtcgaacacagaatgggagtaggtaatattgtcaaagtgctctttaacgggaggcccgaagtcacgtgggtaggcagtgtagattgcttcaatttcatagttagtaatatccctacctctagtgtggggtttatccattcagatatagagaccttgcctgacaaagatactatagagaagctagaggaattggcagccatcttatcgatggctctgctcctgggcaaaataggatcaatactggtgattaagcttatgcctttcagcggggattttgttcagggatttataagttatgtagggtctcattatagagaagtgaaccttgtataccctagatacagcaacttcatctctactgaatcttatttggttatgacagatctcaaggctaaccggctaatgaatcctgaaaagattaagcagcagataattgaatcatctgtgaggacttcacctggacttataggtcacatcctatccattaagcaactaagctgcatacaagcaattgtgggagacgcagttagtagaggtgatatcaatcctactctgaaaaaacttacacctatagagcaggtgctgatcaattgcgggttggcaattaacggacctaagctgtgcaaagaattgatccaccatgatgttgcctcagggcaagatggattgcttaattctatactcatcctctacagggagttggcaagattcaaagacaaccaaagaagtcaacaagggatgttccacgcttaccccgtattggtaagtagcaggcaacgagaacttatatctaggatcacccgcaaattctgggggcacattcttctttactccgggaacaaaaagttgataaataagtttatccagaatctcaagtccggctatctgatactagacttacaccagaatatcttcgttaagaatctatccaagtcagagaaacagattattatgacggggggtttgaaacgtgagtgggtttttaaggtaacagtcaaggagaccaaagaatggtataagttagtcggatacagtgccctgattaaggactaattggttgaactccggaaccctaatcctgccctaggtggttaggcattatttgcaatatattaaagaaaactttgaaaatacgaagtttctattcccagctttgtctggtggccggcatggtcccagcctcctcgctggcgccggctgggcaacattccgaggggaccgtcccctcggtaatggcgaatgggacgcggccgatccggctgctaacaaagcccgaaaggaagctgagttggctgctgccaccgctgagcaataactagcataaccccttggggcctctaaacgggtcttgaggggttttttgctgaaaggaggaactatatccggatgcggccgcgggccctatggtacccagcttttgttccctttagtgagggttaattccgagcttggcgtaatcatggtcatagctgtttcctgtgtgaaattgttatccgctcacaattccacacaacataggagccggaagcataaagtgtaaagcctggggtgcctaatgagtgaggtaactcacattaattgcgttgcgctcactgcccgctttccagtcgggaaacctgtcgtgccagctgcattaatgaatcggccaacgcgcggggagaggcggtttgcgtattgggcgctcttccgcttcctcgctcactgactcgctgcgctcggtcgttcggctgcggcgagcggtatcagctcactcaaaggcggtaatacggttatccacagaatcaggggataacgcaggaaagaacatgtgagcaaaaggccagcaaaaggccaggaaccgtaaaaaggccgcgttgctggcgtttttccataggctcggcccccctgacgagcatcacaaaaatcgacgctcaagtcagaggtggcgaaacccgacaggactataaagataccaggcgttcccccctggaagctccctcgtgcgctctcctgttccgaccctgccgcttaccggatacctgtccgcctttctcccttcgggaagcgtggcgctttctcaatgctcacgctgtaggtatctcagttcggtgtaggtcgttcgctccaagctgggctgtgtgcacgaaccccccgttcagcccgaccgctgcgccttatccggtaactatcgtcttgagtccaacccggtaagacacgacttatcgccactggcagcagccactggtaacaggattagcagagcgaggtatgtaggcggtgctacagagttcttgaagtggtggcctaactacggctacactagaaggacagtatttggtatctgcgctctgctgaagccagttaccttcggaaaaagagttggtagctcttgatccggcaaacaaaccaccgctggtagcggtggtttttttgtttgcaagcagcagattacgcgcagaaaaaaaggatctcaagaagatcctttgatcttttctacggggtctgacgctcagtggaacgaaaactcacgttaagggattttggtcatgagattatcaaaaaggatcttcacctagatccttttaaattaaaaatgaagttttaaatcaatctaaagtatatatgagtaaacttggtctgacagttaccaatgcttaatcagtgaggcacctatctcagcgatctgtctatttcgttcatccatagttgcctgactgcccgtcgtgtagataactacgatacgggagggcttaccatctggccccagtgctgcaatgataccgcgagacccacgctcaccggctccagatttatcagcaataaaccagccagccggaagggccgagcgcagaagtggtcctgcaactttatccgcctccatccagtctattaattgttgccgggaagctagagtaagtagttcgccagttaatagtttgcgcaacgttgttgccattgctacaggcatcgtggtgtcacgctcgtcgtttggtatggcttcattcagctccggttcccaacgatcaaggcgagttacatgatcccccatgttgtgaaaaaaagcggttagctccttcggtcctccgatcgttgtcagaagtaagttggccgcagtgttatcactcatgcttatggcagcactgcataattctcttactgtcatgccatccgtaagatgcttttctgtgactggtgagtactcaaccaagtcattctgagaatagtgtatgcggcgaccgagttgctcttgcccggcgtcaatacgggataataccgcgccacatagcagaactttaaaagtgctcatcattggaaaacgttcttcggggcgaaaactctcaaggatcttaccgctgttgagatccagttcgatgtaacccactcgtgcacccaactgatcttcagcatcttttactttcaccagcgtttctgggtgagcaaaaacaggaaggcaaaatgccgcaaaaaagggaataagggcgacacggaaatgttgaatactcatactcttcctttttcaatattattgaagcatttatcagggttattgtctcatgagcggatacatatttgaatgtatttagaaaaataaacaaataggggttccgcgcacatttccccgaaaagtgccacctgaaattgtaaacgttaatattttgttaaaattcgcgttaaatttttgttaaatcagctcattttttaaccaataggccgaaatcggcaaaatcccttataaatcaaaagaatagaccgagatagggttgagtgttgttccagtttggaacaagagtccactattaaagaacgtggactccaacgtcaaagggcgaaaaaccgtctatcagggcgatggcccactacgtgaaccatcaccctaatcaagttttttggggtcgaggtgccgtaaagcactaaatcggaaccctaaagggagcccccgatttagagcttgacggggaaagccggcgaacgtggcgagaaaggaagggaagaaagcgaaaggagcgggcgctagggcgctggcaagtgtagcggtcacgctgcgcgtaaccaccacacccgccgcgcttaatgcgccgctacagggcgcgtcccattcgccattcaggctgcgcaactgttgggaagggcgatcggtgcgggcctcttcgctattacgccagccaccgcggtg

SEQ ID NO: 144 - DNA, 1554 bp, Artificial Sequence
  Nucleotide sequence of the polynucleotide encoding DENV tetra EDIII-ectoM
atgggcatcatattcattcttcttatgctggttacaccgtctatggcggagaaacttcgaatcaaaggtatgagctatacgatgtgcagcggcaagttcaagatcgagaaggaaatggctgaaacccagcacggtacaactgtggtcaaagtcaaatatgagggggctggcgctccctgtaaagtacccattgagattagggacgtcaataaagagaaggtggtaggtcgcatcatctccagtacacctttggccgagaacacgaactccgtcacaaacatagagttggaacccccgttcggagactcatacattgtgatcggggtgggcaactctgcactcacactgcattggttcaagaagggaagcagtatcggccgcagggataagagagacaaactgaaattgaaaggtatgtcctatgccatgtgcacgaatactttcgttctcaagaaagaagtatctgagactcagcacggaaccatcctgatcaaagtcgagtacaaaggagaagacgtgccctgtaagatcccattcagtaccgaggatggacagggcaaggcccataacggcaggctgataaccgccaaccctgtggttacaaagaaggaagagccagtcaatatcgaagctgagccaccgttcggggagagcaacatagtaattggcataggggataatgctttgaagatcaactggtacaagaaaggaagctccattggccgaagagataagcgcgacaaactccagctgaaaggaatgagctactccatgtgtactgggaagttcaagattgtcaaggaaatcgccgaaactcagcatggcactattgtgatccgcgtgcagtatgaaggcgatggtagcccctgcaagataccatttgaaatcaccgatttggagaaacggcacgtcctgggtcggctcattaccgtgaacccaatcgtgaccgagaaggacagtccagttaatatcgaggccgagcctcctttcggcgacagttacatcattgtaggggtggaaccagggcaactgaagctgaactggttcaagaaaggcagcagtataggacggcgggataaacgggacaaactcacactgaaaggcatgtcatacgttatgtgcaccggctcattcaaactggagaaggaagttgcagagacacagcatgggaccgtgctcgtgcaggtcaaatacgagggcaccgacgctccttgcaagattccgttcagtacacaggacgagaaaggcgtgactcagaacggcagattgattacagcgaaccctatcgtgactgacaaggagaagccagttaacatcgagactgagccgcctttcggagaatcatacattatcgtgggagccggcgagaaggcactgaaactcagctggttcaagaagggcagctcaatcggtcggagagacaagcggtctgtcgccctcgcaccgcacgtgggcctgggtctggaaacgaggaccgagacgtggatgagttccgaaggcgcatggaagcaaatccagaaagtggagacgtgggccctcaggcatccgtaatga

SEQ ID NO: 145 - protein, 516 aa, Artificial Sequence
  Amino acid sequence of DENV tetra EDIII-ectoM
MGIIFILLMLVTPSMAEKLRIKGMSYTMCSGKFKIEKEMAETQHGTTVVKVKYEGAGAPCKVPIEIRDVNKEKVVGRIISSTPLAENTNSVTNIELEPPFGDSYIVIGVGNSALTLHWFKKGSSIGRRDKRDKLKLKGMSYAMCTNTFVLKKEVSETQHGTILIKVEYKGEDVPCKIPFSTEDGQGKAHNGRLITANPVVTKKEEPVNIEAEPPFGESNIVIGIGDNALKINWYKKGSSIGRRDKRDKLQLKGMSYSMCTGKFKIVKEIAETQHGTIVIRVQYEGDGSPCKIPFEITDLEKRHVLGRLITVNPIVTEKDSPVNIEAEPPFGDSYIIVGVEPGQLKLNWFKKGSSIGRRDKRDKLTLKGMSYVMCTGSFKLEKEVAETQHGTVLVQVKYEGTDAPCKIPFSTQDEKGVTQNGRLITANPIVTDKEKPVNIETEPPFGESYIIVGAGEKALKLSWFKKGSSIGRRDKRSVALAPHVGLGLETRTETWMSSEGAWKQIQKVETWALRHP

SEQ ID NO: 146 - protein, 537 aa, Artificial Sequence
  Amino acid sequence of the chimeric polyepitope of DENV2
KSIEDNPEIEDDIFRKKRLTIMDLHPGAGKTKRYLPAIVREAIKRGLRTLILAPTRVVAAEMEEALRGLPIRYQTPAIRAEHTGREIVDLMCHATFTMRLLSPVRVPNYNLIIMDEAHFTDPASIAARGYISTRVEMGEAAGIFMTATPPGSRDPFPQSNAPIMDEEREIPERSWNSGHEWVTDEDCAHWKEAKMLLDNINTPEGIIPSMFEPEREKVDAIDGEYRLRGEARKTFVDLMRRGDLPVWLAYKVAAEGINYADRRWCFDGIKNNQILEENVEVEIWTKEGERKKLKPRWLDARIYSDPLALKEFKEFAAGITTQESESNILDIDLRPASAWTLYAVATTFVTPMLRHSIENSSVNVSLTAIANQATVLMGLGKGWPLSKMDIGVPLLAIGCYSQVLDIIGKRIEKIKQEHETSWHYDQDHPYKTWAYHGSYETKQTGSASSMVNGVVRLLTKPWDVVPMVTQMAMTDTTPFGQQRVFKEKVDTRTQEPKEGTKKLMKITAEWLWKELGKKKTPRMCTREEFTRKVRSNA

SEQ ID NO: 147 - protein, 538 aa, Artificial Sequence
  Amino acid sequence of the chimeric polyepitope of DENV3
AEPDGPTPELEEEMFKKRNLTIMDLHPGSGKTRKYLPAIVREAIKRRLRTLILAPTRVVAAEMEEALKGLPIRYQTTATKSEHTGREIVDLMCHATFTMRLLSPVRVPNYNLIIMDEAHFTDPASIAARGYISTRVGMGEAAAIFMTATPPGTADAFPQSNAPIQDEERDIPERSWNSGNEWITDEDHAHWTEAKMLLDNINTPEGIIPALFEPEREKSAAIDGEYRLKGESRKTFVELMRRGDLPVWLAHKVASEGIKYTDRKWCFDGQRNNQILEENMDVEIWTKEGEKKKLRPRWLDARTYSDPLALKEFKDFAAGEPGVVSPTSYLDVDLHPASAWTLYAVATTVITPMLRHTIENSTANVSLAAIANQAVVLMGLDKGWPISKMDLGVPLLALGCYSQVMDVIGERIKRIKEEHNSTWHYDDENPYKTWAYHGSYEVKATGSASSMINGVVKLLTKPWDVVPMVTQMAMTDTTPFGQQRVFKEKVDTRTPRSMPGTRRVMGITAEWLWRTLGRNKKPRLCTREEFTKKVRTNA

SEQ ID NO: 148 - protein, 534 aa, Artificial Sequence
  Amino acid sequence of the chimeric polyepitope of DENV4
RIGEPDYEVDEDIFRKKRLTIMDLHPGAGKTKRILPSIVREALKRRLRTLILAPTRVVAAEMEEALRGLPIRYQTPAVKSEHTGREIVDLMCHATFTTRLLSSTRVPNYNLIVMDEAHFTDPSSVAARGYISTRVEMGEAAAIFMTATPPGATDPFPQSNSPIEDIEREIPERSWNTGFDWITDEDHAHWTEAKMLLDNIYTPEGIIPTLFGPEREKTQAIDGEFRLRGEQRKTFVELMRRGDLPVWLSYKVASAGISYKDREWCFTGERNNQILEENMEVEIWTREGEKKKLRPRWLDARVYADPMALKDFKEFASGVKTETTILDVDLRPASAWTLYAVATTILTPMLRHTIENTSANLSLAAIANQAAVLMGLGKGWPLHRMDLGVPLLAMGCYSQVMTIIGRRLQRLQEEHKETWHYDQENPYRTWAYHGSYEAPSTGSASSMVNGVVKLLTKPWDVIPMVTQLAMTDTTPFGQQRVFKEKVDTRTPQPKPGTRMVMTTTANWLWALLGKKKNPRLCTREEFISKVRSNA

SEQ ID NO: 149 - DNA, 22243 bp, Artificial Sequence
  Complete optimised nucleotide sequence of the polynucleotide encoding pTM-MVDVax11
  misc_feature (1)..(8): NotI
  misc_feature (9)..(28): T7 promoter
  misc_feature (29)..(82): Hammerhead ribozyme
  misc_feature (83)..(189): MV Leader and N promoter
  misc_feature (190)..(1767): MV N ORF
  misc_feature (1768)..(1888): MV N-P intergenic
  misc_feature (1889)..(3412): MV P ORF
  misc_feature (3413)..(3531): MV ATU2
  misc_feature (3532)..(6699): DENV1 NS polyepitope/DENV tetra EDIII/ectoM
  misc_feature (6700)..(6813): MV P-M intergenic
  misc_feature (6814)..(7803): MV M ORF
  misc_feature (7804)..(8806): MV M-F intergenic
  misc_feature (8807)..(10468): MV F ORF
  misc_feature (10469)..(10628): MV-F-H intergenic
  misc_feature (10629)..(12482): MV H ORF
  misc_feature (12483)..(12591): MV H-L intergenic
  misc_feature (12592)..(19143): MV L ORF
  misc_feature (19144)..(19252): MV Trailer
  misc_feature (19253)..(19336): HDV ribozyme
  misc_feature (19337)..(19478): T7 terminator
  misc_feature (19479)..(19486): Not I
  misc_feature (19487)..(22243): Not I
gcggccgctaatacgactcactatagggccaactttgtttggtctgatgagtccgtgaggacgaaacccggagtcccgggtcaccaaacaaagttgggtaaggatagttcaatcaatgatcatcttctagtgcacttaggattcaagatcctattatcagggacaagagcaggattagggatatccgagatggccacacttttaaggagcttagcattgttcaaaagaaacaaggacaaaccacccattacatcaggatccggtggagccatcagaggaatcaaacacattattatagtaccaatccctggagattcctcaattaccactcgatccagacttctggaccggttggtgaggttaattggaaacccggatgtgagcgggcccaaactaacaggggcactaataggtatattatccttatttgtggagtctccaggtcaattgattcagaggatcaccgatgaccctgacgttagcataaggctgttagaggttgtccagagtgaccagtcacaatctggccttaccttcgcatcaagaggtaccaacatggaggatgaggcggaccaatacttttcacatgatgatccaattagtagtgatcaatccaggttcggatggttcgggaacaaggaaatctcagatattgaagtgcaagaccctgagggattcaacatgattctgggtaccatcctagcccaaatttgggtcttgctcgcaaaggcggttacggccccagacacggcagctgattcggagctaagaaggtggataaagtacacccaacaaagaagggtagttggtgaatttagattggagagaaaatggttggatgtggtgaggaacaggattgccgaggacctctccttacgccgattcatggtcgctctaatcctggatatcaagagaacacccggaaacaaacccaggattgctgaaatgatatgtgacattgatacatatatcgtagaggcaggattagccagttttatcctgactattaagtttgggatagaaactatgtatcctgctcttggactgcatgaatttgctggtgagttatccacacttgagtccttgatgaacctttaccagcaaatgggggaaactgcaccctacatggtaatcctggagaactcaattcagaacaagttcagtgcaggatcataccctctgctctggagctatgccatgggagtaggagtggaacttgaaaactccatgggaggtttgaactttggccgatcttactttgatccagcatattttagattagggcaagagatggtaaggaggtcagctggaaaggtcagttccacattggcatctgaactcggtatcactgccgaggatgcaaggcttgtttcagagattgcaatgcatactactgaggacaagatcagtagagcggttggacccagacaagcccaagtatcatttctacacggtgatcaaagtgagaatgagctaccgagattggggggcaaggaagataggagggtcaaacagagtcgaggagaagccagggagagctacagagaaaccgggcccagcagagcaagtgatgcgagagctgcccatcttccaaccggcacacccctagacattgacactgcaacggagtccagccaagatccgcaggacagtcgaaggtcagctgacgccctgcttaggctgcaagccatggcaggaatctcggaagaacaaggctcagacacggacacccctatagtgtacaatgacagaaatcttctagactaggtgcgagaggccgagggccagaacaacatccgcctaccatccatcattgttataaaaaacttaggaaccaggtccacacagccgccagcccatcaaccatccactcccacgattggagccaatggcagaagagcaggcacgccatgtcaaaaacggactggaatgcatccgggctctcaaggccgagcccatcggctcactggccatcgaggaagctatggcagcatggtcagaaatatcagacaacccaggacaggagcgagccacctgcagggaagagaaggcaggcagttcgggtctcagcaaaccatgcctctcagcaattggatcaactgaaggcggtgcacctcgcatccgcggtcagggacctggagagagcgatgacgacgctgaaactttgggaatccccccaagaaatctccaggcatcaagcactgggttacagtgttattacgtttatgatcacagcggtgaagcggttaagggaatccaagatgctgactctatcatggttcaatcaggccttgatggtgatagcaccctctcaggaggagacaatgaatctgaaaacagcgatgtggatattggcgaacctgataccgagggatatgctatcactgaccggggatctgctcccatctctatggggttcagggcttctgatgttgaaactgcagaaggaggggagatccacgagctcctgagactccaatccagaggcaacaactttccgaagcttgggaaaactctcaatgttcctccgcccccggaccccggtagggccagcacttccgggacacccattaaaaagggcacagacgcgagattagcctcatttggaacggagatcgcgtctttattgacaggtggtgcaacccaatgtgctcgaaagtcaccctcggaaccatcagggccaggtgcacctgcggggaatgtccccgagtgtgtgagcaatgccgcactgatacaggagtggacacccgaatctggtaccacaatctccccgagatcccagaataatgaagaagggggagactattatgatgatgagctgttctctgatgtccaagatattaaaacagccttggccaaaatacacgaggataatcagaagataatctccaagctagaatcactgctgttattgaagggagaagttgagtcaattaagaagcagatcaacaggcaaaatatcagcatatccaccctggaaggacacctctcaagcatcatgatcgccattcctggacttgggaaggatcccaacgaccccactgcagatgtcgaaatcaatcccgacttgaaacccatcataggcagagattcaggccgagcactggccgaagttctcaagaaacccgttgccagccgacaactccaaggaatgacaaatggacggaccagttccagaggacagctgctgaaggaatttcagctaaagccgatcgggaaaaagatgagctcagccgtcgggtttgttcctgacaccggccctgcatcacgcagtgtaatccgctccattataaaatccagccggctagaggaggatcggaagcgttacctgatgactctccttgatgatatcaaaggagccaatgatcttgccaagttccaccagatgctgatgaagataataatgaagtagctacagctcaacttacctgccaaccccatgccagtcgacccaactagcctaccctccatcattgttataaaaaacttaggaaccaggtccacacagccgccagcccatcaacgcgtacgatggcatcacaggagggaccactgcccgaaattgaggacgaagtgtttagaaagcgaaatctgactattatggacctgcaccccggatctggcaagacccggagatacctgccagccatcgtgagggaggctattaagcggaaactgagaacactgatcctggccccaactcgcgtggtcgcttccgaaatggctgaggccctgaaaggcatgcccatccggtatcagaccacagcagtgaagtctgaacataccggcaaggagattgtggacctgatgtgccacgccactttcaccatgcgactgctgagcccagtgcgggtccccaactacaatatgatcattatggacgaggcccactttactgatcccagctccatcgccgctagaggatatatttccaccagggtgggaatgggcgaggcagcagctatcttcatgacagcaactccccctggcagcgtggaggcatttcctcagtccaacgccgtcatccaggacgaggagcgggacattcctgagcggagctggaattctgggtacgaatggatcacagacgaggatcatgcacactggactgaagccaagatgctgctggacaacattaatactcctgagggaatcattccagctctgttcgagcccgaaagagagaagtctgcagccatcgacggcgagtatagactgaggggagaggcccggaagaccttcgtggaactgatgaggcgcggcgatctgcccgtgtggctgagttacaaggtcgcttcagagggattccagtatagtgaccgacggtggtgctttgatggcgaacgcaacaatcaggtgctggaggagaacatggatgtcgagatttggacaaaggaaggcgagcggaagaaactgcgcccacgatggctggacgctcggacttacagcgatcccctggcactgagagaattcaaagagtttgctgcaggggtggccgtcgagaatcaccatcacgccgctatgctggacgtggatctgcatcctgccagtgcttggaccctgtatgcagtggccactaccatcattaccccaatgatgcgccacacaatcgagaacacaactgccaatatctcactgacagctattgcaaaccaggcagccattctgatgggactggacaaaggctggcccatcagcaagatggatattggcgtgcctctgctggccctggggtgttacagtcaggtgctggacatcattggccagaggatcgagaacattaagcatgagcacaaatcaacctggcattacgacgaagataatccctataagacatgggcctaccacggaagctatgaggtgaaaccttcaggcagcgccagcagcatggtcaacggggtggtcaagctgctgaccaaaccttgggacgtgatcccaatggtcactcagattgccatgaccgataccaccccattcggccagcagcgggtgttcaaggagaaggtggacacccgcacacctaaggctaaacgagggactgcacagatcatggaggtgaccgccaagtggctgtggggattcctgtccaggaacaagaagccaagaatctgtaccagggaagagttcacaagaaaggtccggtcaaacgccggcatcatattcattcttcttatgctggttacaccgtctatggcggagaaacttcgaatcaaaggtatgagctatacgatgtgcagcggcaagttcaagatcgagaaggaaatggctgaaacccagcacggtacaactgtggtcaaagtcaaatatgagggggctggcgctccctgtaaagtacccattgagattagggacgtcaataaagagaaggtggtaggtcgcatcatctccagtacacctttggccgagaacacgaactccgtcacaaacatagagttggaacccccgttcggagactcatacattgtgatcggggtgggcaactctgcactcacactgcattggttcaagaagggaagcagtatcggccgcagggataagagagacaaactgaaattgaaaggtatgtcctatgccatgtgcacgaatactttcgttctcaagaaagaagtatctgagactcagcacggaaccatcctgatcaaagtcgagtacaaaggagaagacgtgccctgtaagatcccattcagtaccgaggatggacagggcaaggcccataacggcaggctgataaccgccaaccctgtggttacaaagaaggaagagccagtcaatatcgaagctgagccaccgttcggggagagcaacatagtaattggcataggggataatgctttgaagatcaactggtacaagaaaggaagctccattggccgaagagataagcgcgacaaactccagctgaaaggaatgagctactccatgtgtactgggaagttcaagattgtcaaggaaatcgccgaaactcagcatggcactattgtgatccgcgtgcagtatgaaggcgatggtagcccctgcaagataccatttgaaatcaccgatttggagaaacggcacgtcctgggtcggctcattaccgtgaacccaatcgtgaccgagaaggacagtccagttaatatcgaggccgagcctcctttcggcgacagttacatcattgtaggggtggaaccagggcaactgaagctgaactggttcaagaaaggcagcagtataggacggcgggataaacgggacaaactcacactgaaaggcatgtcatacgttatgtgcaccggctcattcaaactggagaaggaagttgcagagacacagcatgggaccgtgctcgtgcaggtcaaatacgagggcaccgacgctccttgcaagattccgttcagtacacaggacgagaaaggcgtgactcagaacggcagattgattacagcgaaccctatcgtgactgacaaggagaagccagttaacatcgagactgagccgcctttcggagaatcatacattatcgtgggagccggcgagaaggcactgaaactcagctggttcaagaagggcagctcaatcggtcggagagacaagcggtctgtcgccctcgcaccgcacgtgggcctgggtctggaaacgaggaccgagacgtggatgagttccgaaggcgcatggaagcaaatccagaaagtggagacgtgggccctcaggcatccgtaagcgcgcagcgcttagacgtctcgcgatcgatactagtacaacctaaatccattataaaaaacttaggagcaaagtgattgcctcccaaggtccacaatgacagagacctacgacttcgacaagtcggcatgggacatcaaagggtcgatcgctccgatacaacccaccacctacagtgatggcaggctggtgccccaggtcagagtcatagatcctggtctaggcgacaggaaggatgaatgctttatgtacatgtttctgctgggggttgttgaggacagcgattccctagggcctccaatcgggcgagcatttgggttcctgcccttaggtgttggcagatccacagcaaagcccgaaaaactcctcaaagaggccactgagcttgacatagttgttagacgtacagcagggctcaatgaaaaactggtgttctacaacaacaccccactaactctcctcacaccttggagaaaggtcctaacaacagggagtgtcttcaacgcaaaccaagtgtgcaatgcggttaatctgataccgctcgataccccgcagaggttccgtgttgtttatatgagcatcacccgtctttcggataacgggtattacaccgttcctagaagaatgctggaattcagatcggtcaatgcagtggccttcaacctgctggtgacccttaggattgacaaggcgataggccctgggaagatcatcgacaatacagagcaacttcctgaggcaacatttatggtccacatcgggaacttcaggagaaagaagagtgaagtctactctgccgattattgcaaaatgaaaatcgaaaagatgggcctggtttttgcacttggtgggatagggggcaccagtcttcacattagaagcacaggcaaaatgagcaagactctccatgcacaactcgggttcaagaagaccttatgttacccgctgatggatatcaatgaagaccttaatcgattactctggaggagcagatgcaagatagtaagaatccaggcagttttgcagccatcagttcctcaagaattccgcatttacgacgacgtgatcataaatgatgaccaaggactattcaaagttctgtagaccgtagtgcccagcaatgcccgaaaacgacccccctcacaatgacagccagaaggcccggacaaaaaagccccctccgaaagactccacggaccaagcgagaggccagccagcagccgacggcaagcgcgaacaccaggcggccccagcacagaacagccctgacacaaggccaccaccagccaccccaatctgcatcctcctcgtgggacccccgaggaccaacccccaaggctgcccccgatccaaaccaccaaccgcatccccaccacccccgggaaagaaacccccagcaattggaaggcccctccccctcttcctcaacacaagaactccacaaccgaaccgcacaagcgaccgaggtgacccaaccgcaggcatccgactccctagacagatcctctctccccggcaaactaaacaaaacttagggccaaggaacatacacacccaacagaacccagaccccggcccacggcgccgcgcccccaacccccgacaaccagagggagcccccaaccaatcccgccggctcccccggtgcccacaggcagggacaccaacccccgaacagacccagcacccaaccatcgacaatccaagacgggggggcccccccaaaaaaaggcccccaggggccgacagccagcaccgcgaggaagcccacccaccccacacacgaccacggcaaccaaaccagaacccagaccaccctgggccaccagctcccagactcggccatcaccccgcagaaaggaaaggccacaacccgcgcaccccagccccgatccggcggggagccacccaacccgaaccagcacccaagagcgatccccgaaggacccccgaaccgcaaaggacatcagtatcccacagcctctccaagtcccccggtctcctcctcttctcgaagggaccaaaagatcaatccaccacacccgacgacactcaactccccacccctaaaggagacaccgggaatcccagaatcaagactcatccaatgtccatcatgggtctcaaggtgaacgtctctgccatattcatggcagtactgttaactctccaaacacccaccggtcaaatccattggggcaatctctctaagataggggtggtaggaataggaagtgcaagctacaaagttatgactcgttccagccatcaatcattagtcataaaattaatgcccaatataactctcctcaataactgcacgagggtagagattgcagaatacaggagactactgagaacagttttggaaccaattagagatgcacttaatgcaatgacccagaatataagaccggttcagagtgtagcttcaagtaggagacacaagagatttgcgggagtagtcctggcaggtgcggccctaggcgttgccacagctgctcagataacagccggcattgcacttcaccagtccatgctgaactctcaagccatcgacaatctgagagcgagcctggaaactactaatcaggcaattgagacaatcagacaagcagggcaggagatgatattggctgttcagggtgtccaagactacatcaataatgagctgataccgtctatgaaccaactatcttgtgatttaatcggccagaagctcgggctcaaattgctcagatactatacagaaatcctgtcattatttggccccagtttacgggaccccatatctgcggagatatctatccaggctttgagctatgcgcttggaggagacatcaataaggtgttagaaaagctcggatacagtggaggtgatttactgggcatcttagagagcggaggaataaaggcccggataactcacgtcgacacagagtcctacttcattgtcctcagtatagcctatccgacgctgtccgagattaagggggtgattgtccaccggctagagggggtctcgtacaacataggctctcaagagtggtataccactgtgcccaagtatgttgcaacccaagggtaccttatctcgaattttgatgagtcatcgtgtactttcatgccagaggggactgtgtgcagccaaaatgccttgtacccgatgagtcctctgctccaagaatgcctccgggggtacaccaagtcctgtgctcgtacactcgtatccgggtcttttgggaaccggttcattttatcacaagggaacctaatagccaattgtgcatcaatcctttgcaagtgttacacaacaggaacgatcattaatcaagaccctgacaagatcctaacatacattgctgccgatcactgcccggtagtcgaggtgaacggcgtgaccatccaagtcgggagcaggaggtatccagacgctgtgtacttgcacagaattgacctcggtcctcccatatcattggagaggttggacgtagggacaaatctggggaatgcaattgctaagttggaggatgccaaggaattgttggagtcatcggaccagatattgaggagtatgaaaggtttatcgagcactagcatagtctacatcctgattgcagtgtgtcttggagggttgatagggatccccgctttaatatgttgctgcagggggcgttgtaacaaaaagggagaacaagttggtatgtcaagaccaggcctaaagcctgatcttacgggaacatcaaaatcctatgtaaggtcgctctgatcctctacaactcttgaaacacaaatgtcccacaagtctcctcttcgtcatcaagcaaccaccgcacccagcatcaagcccacctgaaattatctccggcttccctctggccgaacaatatcggtagttaatcaaaacttagggtgcaagatcatccacaatgtcaccacaacgagaccggataaatgccttctacaaagataacccccatcccaagggaagtaggatagtcattaacagagaacatcttatgattgatagaccttatgttttgctggctgttctgtttgtcatgtttctgagcttgatcgggttgctagccattgcaggcattagacttcatcgggcagccatctacaccgcagagatccataaaagcctcagcaccaatctagatgtaactaactcaatcgagcatcaggtcaaggacgtgctgacaccactcttcaaaatcatcggtgatgaagtgggcctgaggacacctcagagattcactgacctagtgaaattaatctctgacaagattaaattccttaatccggatagggagtacgacttcagagatctcacttggtgtatcaacccgccagagagaatcaaattggattatgatcaatactgtgcagatgtggctgctgaagagctcatgaatgcattggtgaactcaactctactggagaccagaacaaccaatcagttcctagctgtctcaaagggaaactgctcagggcccactacaatcagaggtcaattctcaaacatgtcgctgtccctgttagacttgtatttaggtcgaggttacaatgtgtcatctatagtcactatgacatcccagggaatgtatgggggaacttacctagtggaaaagcctaatctgagcagcaaaaggtcagagttgtcacaactgagcatgtaccgagtgtttgaagtaggtgttatcagaaatccgggtttgggggctccggtgttccatatgacaaactatcttgagcaaccagtcagtaatgatctcagcaactgtatggtggctttgggggagctcaaactcgcagccctttgtcacggggaagattctatcacaattccctatcagggatcagggaaaggtgtcagcttccagctcgtcaagctaggtgtctggaaatccccaaccgacatgcaatcctgggtccccttatcaacggatgatccagtgatagacaggctttacctctcatctcacagaggtgttatcgctgacaatcaagcaaaatgggctgtcccgacaacacgaacagatgacaagttgcgaatggagacatgcttccaacaggcgtgtaagggtaaaatccaagcactctgcgagaatcccgagtgggcaccattgaaggataacaggattccttcatacggggtcttgtctgttgatctgagtctgacagttgagcttaaaatcaaaattgcttcgggattcgggccattgatcacacacggttcagggatggacctatacaaatccaaccacaacaatgtgtattggctgactatcccgccaatgaagaacctagccttaggtgtaatcaacacattggagtggataccgagattcaaggttagtccctacctcttcactgtcccaattaaggaagcaggcgaagactgccatgccccaacatacctacctgcggaggtggatggtgatgtcaaactcagttccaatctggtgattctacctggtcaagatctccaatatgttttggcaacctacgatacttccagggttgaacatgctgtggtttattacgtttacagcccaagccgctcattttcttacttttatccttttaggttgcctataaagggggtccccatcgaattacaagtggaatgcttcacatgggaccaaaaactctggtgccgtcacttctgtgtgcttgcggactcagaatctggtggacatatcactcactctgggatggtgggcatgggagtcagctgcacagtcacccgggaagatggaaccaatcgcagatagggctgctagtgaaccaatcacatgatgtcacccagacatcaggcatacccactagtgtgaaatagacatcagaattaagaaaaacgtagggtccaagtggttccccgttatggactcgctatctgtcaaccagatcttataccctgaagttcacctagatagcccgatagttaccaataagatagtagccatcctggagtatgctcgagtccctcacgcttacagcctggaggaccctacactgtgtcagaacatcaagcaccgcctaaaaaacggattttccaaccaaatgattataaacaatgtggaagttgggaatgtcatcaagtccaagcttaggagttatccggcccactctcatattccatatccaaattgtaatcaggatttatttaacatagaagacaaagagtcaacgaggaagatccgtgaactcctcaaaaaggggaattcgctgtactccaaagtcagtgataaggttttccaatgcttaagggacactaactcacggcttggcctaggctccgaattgagggaggacatcaaggagaaagttattaacttgggagtttacatgcacagctcccagtggtttgagccctttctgttttggtttacagtcaagactgagatgaggtcagtgattaaatcacaaacccatacttgccataggaggagacacacacctgtattcttcactggtagttcagttgagttgctaatctctcgtgaccttgttgctataatcagtaaagagtctcaacatgtatattacctgacatttgaactggttttgatgtattgtgatgtcatagaggggaggttaatgacagagaccgctatgactattgatgctaggtatacagagcttctaggaagagtcagatacatgtggaaactgatagatggtttcttccctgcactcgggaatccaacttatcaaattgtagccatgctggagcctctttcacttgcttacctgcagctgagggatataacagtagaactcagaggtgctttccttaaccactgctttactgaaatacatgatgttcttgaccaaaacgggttttctgatgaaggtacttatcatgagttaactgaagctctagattacattttcataactgatgacatacatctgacaggggagattttctcatttttcagaagtttcggccaccccagacttgaagcagtaacggctgctgaaaatgttaggaaatacatgaatcagcctaaagtcattgtgtatgagactctgatgaaaggtcatgccatattttgtggaatcataatcaacggctatcgtgacaggcacggaggcagttggccaccgctgaccctccccctgcatgctgcagacacaatccggaatgctcaagcttcaggtgaagggttaacacatgagcagtgcgttgataactggaaatcttttgctggagtgaaatttggctgctttatgcctcttagcctggatagtgatctgacaatgtacctaaaggacaaggcacttgctgctctccaaagggaatgggattcagtttacccgaaagagttcctgcgttacgaccctcccaagggaaccgggtcacggaggcttgtagatgttttccttaatgattcgagctttgacccatatgatgtgataatgtatgttgtaagtggagcttacctccatgaccctgagttcaacctgtcttacagcctgaaagaaaaggagatcaaggaaacaggtagactttttgctaaaatgacttacaaaatgagggcatgccaagtgattgctgaaaatctaatctcaaacgggattggcaaatattttaaggacaatgggatggccaaggatgagcacgatttgactaaggcactccacactctagctgtctcaggagtccccaaagatctcaaagaaagtcacaggggggggccagtcttaaaaacctactcccgaagcccagtccacacaagtaccaggaacgtgagagcagcaaaagggtttatagggttccctcaagtaattcggcaggaccaagacactgatcatccggagaatatggaagcttacgagacagtcagtgcatttatcacgactgatctcaagaagtactgccttaattggagatatgagaccatcagcttgtttgcacagaggctaaatgagatttacggattgccctcatttttccagtggctgcataagaggcttgagacctctgtcctgtatgtaagtgaccctcattgcccccccgaccttgacgcccatatcccgttatataaagtccccaatgatcaaatcttcattaagtaccctatgggaggtatagaagggtattgtcagaagctgtggaccatcagcaccattccctatctatacctggctgcttatgagagcggagtaaggattgcttcgttagtgcaaggggacaatcagaccatagccgtaacaaaaagggtacccagcacatggccctacaaccttaagaaacgggaagctgctagagtaactagagattactttgtaattcttaggcaaaggctacatgatattggccatcacctcaaggcaaatgagacaattgtttcatcacatttttttgtctattcaaaaggaatatattatgatgggctacttgtgtcccaatcactcaagagcatcgcaagatgtgtattctggtcagagactatagttgatgaaacaagggcagcatgcagtaatattgctacaacaatggctaaaagcatcgagagaggttatgaccgttaccttgcatattccctgaacgtcctaaaagtgatacagcaaattctgatctctcttggcttcacaatcaattcaaccatgacccgggatgtagtcatacccctcctcacaaacaacgacctcttaataaggatggcactgttgcccgctcctattggggggatgaattatctgaatatgagcaggctgtttgtcagaaacatcggtgatccagtaacatcatcaattgctgatctcaagagaatgattctcgcctcactaatgcctgaagagaccctccatcaagtaatgacacaacaaccgggggactcttcattcctagactgggctagcgacccttactcagcaaatcttgtatgtgtccagagcatcactagactcctcaagaacataactgcaaggtttgtcctgatccatagtccaaacccaatgttaaaaggattattccatgatgacagtaaagaagaggacgagggactggcggcattcctcatggacaggcatattatagtacctagggcagctcatgaaatcctggatcatagtgtcacaggggcaagagagtctattgcaggcatgctggataccacaaaaggcttgattcgagccagcatgaggaagggggggttaacctctcgagtgataaccagattgtccaattatgactatgaacaattcagagcagggatggtgctattgacaggaagaaagagaaatgtcctcattgacaaagagtcatgttcagtgcagctggcgagagctctaagaagccatatgtgggcgaggctagctcgaggacggcctatttacggccttgaggtccctgatgtactagaatctatgcgaggccaccttattcggcgtcatgagacatgtgtcatctgcgagtgtggatcagtcaactacggatggttttttgtcccctcgggttgccaactggatgatattgacaaggaaacatcatccttgagagtcccatatattggttctaccactgatgagagaacagacatgaagcttgccttcgtaagagccccaagtcgatccttgcgatctgctgttagaatagcaacagtgtactcatgggcttacggtgatgatgatagctcttggaacgaagcctggttgttggctaggcaaagggccaatgtgagcctggaggagctaagggtgatcactcccatctcaacttcgactaatttagcgcataggttgagggatcgtagcactcaagtgaaatactcaggtacatcccttgtccgagtggcgaggtataccacaatctccaacgacaatctctcatttgtcatatcagataagaaggttgatactaactttatataccaacaaggaatgcttctagggttgggtgttttagaaacattgtttcgactcgagaaagataccggatcatctaacacggtattacatcttcacgtcgaaacagattgttgcgtgatcccgatgatagatcatcccaggatacccagctcccgcaagctagagctgagggcagagctatgtaccaacccattgatatatgataatgcacctttaattgacagagatgcaacaaggctatacacccagagccataggaggcaccttgtggaatttgttacatggtccacaccccaactatatcacattttagctaagtccacagcactatctatgattgacctggtaacaaaatttgagaaggaccatatgaatgaaatttcagctctcataggggatgacgatatcaatagtttcataactgagtttctgctcatagagccaagattattcactatctacttgggccagtgtgcggccatcaattgggcatttgatgtacattatcatagaccatcagggaaatatcagatgggtgagctgttgtcatcgttcctttctagaatgagcaaaggagtgtttaaggtgcttgtcaatgctctaagccacccaaagatctacaagaaattctggcattgtggtattatagagcctatccatggtccttcacttgatgctcaaaacttgcacacaactgtgtgcaacatggtttacacatgctatatgacctacctcgacctgttgttgaatgaagagttagaagagttcacatttctcttgtgtgaaagcgacgaggatgtagtaccggacagattcgacaacatccaggcaaaacacttatgtgttctggcagatttgtactgtcaaccagggacctgcccaccaattcgaggtctaagaccggtagagaaatgtgcagttctaaccgaccatatcaaggcagaggctatgttatctccagcaggatcttcgtggaacataaatccaattattgtagaccattactcatgctctctgacttatctccggcgaggatcgatcaaacagataagattgagagttgatccaggattcattttcgacgccctcgctgaggtaaatgtcagtcagccaaagatcggcagcaacaacatctcaaatatgagcatcaaggctttcagacccccacacgatgatgttgcaaaattgctcaaagatatcaacacaagcaagcacaatcttcccatttcagggggcaatctcgccaattatgaaatccatgctttccgcagaatcgggttgaactcatctgcttgctacaaagctgttgagatatcaacattaattaggagatgccttgagccaggggaggacggcttgttcttgggtgagggatcgggttctatgttgatcacttataaagagatacttaaactaaacaagtgcttctataatagtggggtttccgccaattctagatctggtcaaagggaattagcaccctatccctccgaagttggccttgtcgaacacagaatgggagtaggtaatattgtcaaagtgctctttaacgggaggcccgaagtcacgtgggtaggcagtgtagattgcttcaatttcatagttagtaatatccctacctctagtgtggggtttatccattcagatatagagaccttgcctgacaaagatactatagagaagctagaggaattggcagccatcttatcgatggctctgctcctgggcaaaataggatcaatactggtgattaagcttatgcctttcagcggggattttgttcagggatttataagttatgtagggtctcattatagagaagtgaaccttgtataccctagatacagcaacttcatctctactgaatcttatttggttatgacagatctcaaggctaaccggctaatgaatcctgaaaagattaagcagcagataattgaatcatctgtgaggacttcacctggacttataggtcacatcctatccattaagcaactaagctgcatacaagcaattgtgggagacgcagttagtagaggtgatatcaatcctactctgaaaaaacttacacctatagagcaggtgctgatcaattgcgggttggcaattaacggacctaagctgtgcaaagaattgatccaccatgatgttgcctcagggcaagatggattgcttaattctatactcatcctctacagggagttggcaagattcaaagacaaccaaagaagtcaacaagggatgttccacgcttaccccgtattggtaagtagcaggcaacgagaacttatatctaggatcacccgcaaattctgggggcacattcttctttactccgggaacaaaaagttgataaataagtttatccagaatctcaagtccggctatctgatactagacttacaccagaatatcttcgttaagaatctatccaagtcagagaaacagattattatgacggggggtttgaaacgtgagtgggtttttaaggtaacagtcaaggagaccaaagaatggtataagttagtcggatacagtgccctgattaaggactaattggttgaactccggaaccctaatcctgccctaggtggttaggcattatttgcaatatattaaagaaaactttgaaaatacgaagtttctattcccagctttgtctggtggccggcatggtcccagcctcctcgctggcgccggctgggcaacattccgaggggaccgtcccctcggtaatggcgaatgggacgcggccgatccggctgctaacaaagcccgaaaggaagctgagttggctgctgccaccgctgagcaataactagcataaccccttggggcctctaaacgggtcttgaggggttttttgctgaaaggaggaactatatccggatgcggccgcgggccctatggtacccagcttttgttccctttagtgagggttaattccgagcttggcgtaatcatggtcatagctgtttcctgtgtgaaattgttatccgctcacaattccacacaacataggagccggaagcataaagtgtaaagcctggggtgcctaatgagtgaggtaactcacattaattgcgttgcgctcactgcccgctttccagtcgggaaacctgtcgtgccagctgcattaatgaatcggccaacgcgcggggagaggcggtttgcgtattgggcgctcttccgcttcctcgctcactgactcgctgcgctcggtcgttcggctgcggcgagcggtatcagctcactcaaaggcggtaatacggttatccacagaatcaggggataacgcaggaaagaacatgtgagcaaaaggccagcaaaaggccaggaaccgtaaaaaggccgcgttgctggcgtttttccataggctcggcccccctgacgagcatcacaaaaatcgacgctcaagtcagaggtggcgaaacccgacaggactataaagataccaggcgttcccccctggaagctccctcgtgcgctctcctgttccgaccctgccgcttaccggatacctgtccgcctttctcccttcgggaagcgtggcgctttctcaatgctcacgctgtaggtatctcagttcggtgtaggtcgttcgctccaagctgggctgtgtgcacgaaccccccgttcagcccgaccgctgcgccttatccggtaactatcgtcttgagtccaacccggtaagacacgacttatcgccactggcagcagccactggtaacaggattagcagagcgaggtatgtaggcggtgctacagagttcttgaagtggtggcctaactacggctacactagaaggacagtatttggtatctgcgctctgctgaagccagttaccttcggaaaaagagttggtagctcttgatccggcaaacaaaccaccgctggtagcggtggtttttttgtttgcaagcagcagattacgcgcagaaaaaaaggatctcaagaagatcctttgatcttttctacggggtctgacgctcagtggaacgaaaactcacgttaagggattttggtcatgagattatcaaaaaggatcttcacctagatccttttaaattaaaaatgaagttttaaatcaatctaaagtatatatgagtaaacttggtctgacagttaccaatgcttaatcagtgaggcacctatctcagcgatctgtctatttcgttcatccatagttgcctgactgcccgtcgtgtagataactacgatacgggagggcttaccatctggccccagtgctgcaatgataccgcgagacccacgctcaccggctccagatttatcagcaataaaccagccagccggaagggccgagcgcagaagtggtcctgcaactttatccgcctccatccagtctattaattgttgccgggaagctagagtaagtagttcgccagttaatagtttgcgcaacgttgttgccattgctacaggcatcgtggtgtcacgctcgtcgtttggtatggcttcattcagctccggttcccaacgatcaaggcgagttacatgatcccccatgttgtgaaaaaaagcggttagctccttcggtcctccgatcgttgtcagaagtaagttggccgcagtgttatcactcatgcttatggcagcactgcataattctcttactgtcatgccatccgtaagatgcttttctgtgactggtgagtactcaaccaagtcattctgagaatagtgtatgcggcgaccgagttgctcttgcccggcgtcaatacgggataataccgcgccacatagcagaactttaaaagtgctcatcattggaaaacgttcttcggggcgaaaactctcaaggatcttaccgctgttgagatccagttcgatgtaacccactcgtgcacccaactgatcttcagcatcttttactttcaccagcgtttctgggtgagcaaaaacaggaaggcaaaatgccgcaaaaaagggaataagggcgacacggaaatgttgaatactcatactcttcctttttcaatattattgaagcatttatcagggttattgtctcatgagcggatacatatttgaatgtatttagaaaaataaacaaataggggttccgcgcacatttccccgaaaagtgccacctgaaattgtaaacgttaatattttgttaaaattcgcgttaaatttttgttaaatcagctcattttttaaccaataggccgaaatcggcaaaatcccttataaatcaaaagaatagaccgagatagggttgagtgttgttccagtttggaacaagagtccactattaaagaacgtggactccaacgtcaaagggcgaaaaaccgtctatcagggcgatggcccactacgtgaaccatcaccctaatcaagttttttggggtcgaggtgccgtaaagcactaaatcggaaccctaaagggagcccccgatttagagcttgacggggaaagccggcgaacgtggcgagaaaggaagggaagaaagcgaaaggagcgggcgctagggcgctggcaagtgtagcggtcacgctgcgcgtaaccaccacacccgccgcgcttaatgcgccgctacagggcgcgtcccattcgccattcaggctgcgcaactgttgggaagggcgatcggtgcgggcctcttcgctattacgccagccaccgcggtg

SEQ ID NO: 150 - protein, 9 aa, Artificial Sequence
  Synthetic peptide HBSP A2-2
TLCIPHVAV

SEQ ID NO: 151 - protein, 9 aa, Artificial Sequence
  Synthetic peptide Sv B7-3
SPFLPLLPI

SEQ ID NO: 152 - protein, 5 aa, Artificial Sequence
  Synthetic furin sites
RRDKR